European Patent Application EP 4 394 034 A1, published July 3, 2024. Title: Engineered acyltransferases having altered substrate specificity. Applicant: kez.biosolutions GmbH. The sequence listing filed with the application follows.

SEQUENCE LISTING (82 sequences)

SEQ ID NO: 1 - protein, 2504 aa, Mus musculus
MEEVVIAGMSGKLPESENLQEFWANLIGGVDMVTDDDRRWKAGLYGLPKRSGKLKDLSKFDASFFGVHPKQAHTMDPQLRLLLEVSYEAIVDGGINPASLRGTNTGVWVGVSGSEASEALSRDPETLLGYSMVGCQRAMMANRLSFFFDFKGPSIALDTACSSSLLALQNAYQAIRSGECPAALVGGINLLLKPNTSVQFMKLGMLSPDGTCRSFDDSGSGYCRSEAVVAVLLTKKSLARRVYATILNAGTNTDGSKEQGVTFPSGEVQEQLICSLYQPAGLAPESLEYIEAHGTGTKVGDPQELNGITRSLCAFRQAPLLIGSTKSNMGHPEPASGLAALTKVLLSLEHGVWAPNLHFHNPNPEIPALLDGRLQVVDRPLPVRGGNVGINSFGFGGSNVHVILQPNTRQAPAPTAHAALPHLLHASGRTLEAVQDLLEQGRQHSQDLAFVSMLNDIAATPTAAMPFRGYTVLGVEGRVQEVQQVSTNKRPLWFICSGMGTQWRGMGLSLMRLDSFRESILRSDEAVKPLGVKVSDLLLSTDERTFDDIVHAFVSLTAIQIALIDLLTSVGLKPDGIIGHSLGEVACGYADGCLSQREAVLAAYWRGQCIKDAHLPPGSMAAVGLSWEECKQRCPAGVVPACHNSEDTVTISGPQAAVNEFVEQLKQEGVFAKEVRTGGLAFHSYFMEGIAPTLLQALKKVIREPRPRSARWLSTSIPEAQWQSSLARTSSAEYNVNNLVSPVLFQEALWHIPEHAVVLEIAPHALLQAVLKRGVKSSCTIIPLMKRDHKDNLEFFLTNLGKVHLTGINVNPNALFPPVEFPAPRGTPLISPHIKWDHSQTWDVPVAEDFPNGSSSSSATVYSIDASPESPDHYLVDHCIDGRVIFPGTGYLCLVWKTLARSLGLSLEETPVVFENVSFHQATILPKTGTVALEVRLLEASHAFEVSDTGNLIVSGKVYLWEDPNSKLFDHPEVPTPPESASVSRLTQGEVYKELRLRGYDYGPQFQGICEATLEGEQGKLLWKDNWVTFMDTMLQVSILGSSQQSLQLPTRVTAIYIDPATHRQKVYRLKEDTQVADVTTSRCLGITVSGGIHISRLQTTATSRRQQEQLVPTLEKFVFTPHMEAECLSESTALQKELQLCKGLARALQTKATQQGLKAAMLGQEDPPQHGLPRLLAAACQLQLNGNLQLELGEALAQERLLLPEDPLISGLLNSQALKACVDTALENLSTLKMKVAEVLAGEGHLYSRIPALLNTQPMLQLEYTATDRHPQALKDVQTKLQQHDVAQGQWNPSDPAPSSLGALDLLVCNCALATLGDPALALDNMVAALKEGGFLLVHTVLKGHALGETLACLPSEVQPAPSLLSQEEWESLFSRKALHLVGLKRSFYGTALFLCRRAIPQEKPIFLSVEDTSFQWVDSLKSTLATSSSQPVWLTAMDCPTSGVVGLVNCLRKEPGGHRIRCILLSNLSNTSHAPKLDPGSPELQQVLKHDLVMNVYRDGAWGAFRHFQLEQDKPKEQTAHAFVNVLTRGDLASIRWVSSPLKHTQPSSSGAQLCTVYYASLNFRDIMLATGKLSPDAIPGKWASRDCMLGMEFSGRDRCGRRVMGLVPAEGLATSVLLSSDFLWDVPSSWTLEEAASVPVVYTTAYYSLVVRGRIQRGETVLIHSGSGGVGQAAISIALSLGCRVFTTVGSAEKRAYLQARFPQLDDTSFANSRDTSFEQHVLLHTGGKGVDLVLNSLAEEKLQASVRCLAQHGRFLEIGKFDLSNNHPLGMAIFLKNVTFHGILLDALFEEANDSWREVAALLKAGIRDGVVKPLKCTVFPKAQVEDAFRYMAQGKHIGKVLVQVREEEPEAVLPGAQPTLISAISKTFCPAHKSYIITGGLGGFGLELARWLVLRGAQRLVLTSRSGIRTGYQAKHIREWRRQGIQVLVSTSNVSSLEGARALIAEATKLGPVGGVFNLAMVLRDAMLENQTPELFQDVNKPKYNGTLNLDRATREACPELDYFVAFSSVSCGRGNAGQTNYGFANSTMERICEQRRHDGLPGLAVQWGAIGDVGIVLEAMGTNDTVIGGTLPQRISSCMEVLDLFLNQPHAVLSSFVLAEKKAVAHGDGDTQRDLVKAVAHILGIRDLAGINLDSTLADLGLDSLMGVEVRQILEREHDLVLPMREVRQLTLRKLQEMSSKTDSATDTTAPKSRSDTSLKQNQLNLSTLLVNPEGPTLTQLNSVQSSERPLFLVHPIEGSTTVFHSLAAKLSVPTYGLQCTQAAPLDSIPNLAAYYIDCIKQVQPEGPYRIAGYSFGACVAFEMCSQLQAQQGPAPTHNNLFLFDGSHTYVLAYTQSYRAKMTPGCEAEAEAEALCFFIKQFLDVEHSKVLEALLPLKSLEDRVAASVDLITKSHHSLDRRELSFAAVSFYHKLRAADQYKPKAKYHGNVTLLRAKTGGTYGEDLGADYNLSQVCDGKVSVHIIEGDHRTLLEGSGLESIINIIHSSLAEPRVSVREG

SEQ ID NO: 2 - protein, 2505 aa, Rattus norvegicus
MEEVVIAGMSGKLPESENLQEFWANLIGGVDMVTDDDRRWKAGLYGLPKRSGKLKDLSKFDASFFGVHPKQAHTMDPQLRLLLEVSYEAIVDGGINPASLRGTNTGVWVGVSGSEASEALSRDPETLLGYSMVGCQRAMMANRLSFFFDFKGPSIALDTACSSSLLALQNAYQAIRSGECPAAIVGGINLLLKPNTSVQFMKLGMLSPDGTCRSFDDSGNGYCRAEAVVAVLLTKKSLARRVYATILNAGTNTDGCKEQGVTFPSGEAQEQLIRSLYQPGGVAPESLEYIEAHGTGTKVGDPQELNGITRSLCAFRQSPLLIGSTKSNMGHPEPASGLAALTKVLLSLENGVWAPNLHFHNPNPEIPALLDGRLQVVDRPLPVRGGIVGINSFGFGGANVHVILQPNTQQAPAPAPHAALPHLLHASGRTMEAVQGLLEQGRQHSQDLAFVSMLNDIAATPTAAMPFRGYTVLGVEGHVQEVQQVPASQRPLWFICSGMGTQWRGMGLSLMRLDSFRESILRSDEALKPLGVKVSDLLLSTDEHTFDDIVHSFVSLTAIQIALIDLLTSMGLKPDGIIGHSLGEVACGYADGCLSQREAVLAAYWRGQCIKDANLPAGSMAAVGLSWEECKQRCPPGVVPACHNSEDTVTISGPQAAVNEFVEQLKQEGVFAKEVRTGGLAFHSYFMEGIAPTLLQALKKVIREPRPRSARWLSTSIPEAQWQSSLARTSSAEYNVNNLVSPVLFQEALWHVPEHAVVLEIAPHALLQAVLKRGVKPSCTIIPLMKRDHKDNLEFFLTNLGKVHLTGIDINPNALFPPVEFPVPRGTPLISPHIKWDHSQTWDIPVAEDFPNGSSSSSATVYNIDASSESSDHYLVDHCIDGRVLFPGTGYLYLVWKTLARSLSLSLEETPVVFENVTFHQATILPRTGTVPLEVRLLEASHAFEVSDSGNLIVSGKVYQWEDPDSKLFDHPEVPIPAESESVSRLTQGEVYKELRLRGYDYGPHFQGVYEATLEGEQGKLLWKDNWVTFMDTMLQISILGFSKQSLQLPTRVTAIYIDPATHLQKVYMLEGDTQVADVTTSRCLGVTVSGGVYISRLQTTATSRRQQEQLVPTLEKFVFTPHVEPECLSESAILQKELQLCKGLAKALQTKATQQGLKMTVPGLEDLPQHGLPRLLAAACQLQLNGNLQLELGEVLARERLLLPEDPLISGLLNSQALKACIDTALENLSTLKMKVVEVLAGEGHLYSHISALLNTQPMLQLEYTATDRHPQALKDVQTKLQQHDVAQGQWDPSGPAPTNLGALDLVVCNCALATLGDPALALDNMVAALKDGGFLLMHTVLKGHALGETLACLPSEVQPGPSFLSQEEWESLFSRKALHLVGLKKSFYGTALFLCRRLSPQDKPIFLPVEDTSFQWVDSLKSILATSSSQPVWLTAMNCPTSGVVGLVNCLRKEPGGHRIRCILLSNLSSTSHVPKLDPGSSELQKVLESDLVMNVYRDGAWGAFRHFQLEQDKPEEQTAHAFVNVLTRGDLASIRWVSSPLKHMQPPSSSGAQLCTVYYASLNFRDIMLATGKLSPDAIPGKWASRDCMLGMEFSGRDKCGRRVMGLVPAEGLATSVLLSPDFLWDVPSSWTLEEAASVPVVYTTAYYSLVVRGRIQHGETVLIHSGSGGVGQAAISIALSLGCRVFTTVGSAEKRAYLQARFPQLDDTSFANSRDTSFEQHVLLHTGGKGVDLVLNSLAEEKLQASVRCLAQHGRFLEIGKFDLSNNHPLGMAIFLKNVTFHGILLDALFEGANDSWREVAELLKAGIRDGVVKPLKCTVFPKAQVEDAFRYMAQGKHIGKVLVQVREEEPEAMLPGAQPTLISAISKTFCPEHKSYIITGGLGGFGLELARWLVLRGAQRLVLTSRSGIRTGYQAKHVREWRRQGIHVLVSTSNVSSLEGARALIAEATKLGPVGGVFNLAMVLRDAMLENQTPELFQDVNKPKYNGTLNLDRATREACPELDYFVAFSSVSCGRGNAGQSNYGFANSTMERICEQRRHDGLPGLAVQWGAIGDVGIILEAMGTNDTVVGGTLPQRISSCMEVLDLFLNQPHAVLSSFVLAEKKAVAHGDGEAQRDLVKAVAHILGIRDLAGINLDSSLADLGLDSLMGVEVRQILEREHDLVLPIREVRQLTLRKLQEMSSKAGSDTELAAPKSKNDTSLKQAQLNLSILLVNPEGPTLTRLNSVQSSERPLFLVHPIEGSITVFHSLAAKLSVPTYGLQCTQAAPLDSIPNLAAYYIDCIKQVQPEGPYRVAGYSFGACVAFEMCSQLQAQQGPAPAHNNLFLFDGSHTYVLAYTQSYRAKLTPGCEAEAEAEAICFFIKQFVDAEHSKVLEALLPLKSLEDRVAAAVDLITRSHQSLDRRDLSFAAVSFYYKLRAADQYKPKAKYHGNVILLRAKTGGTYGEDLGADYNLSQVCDGKVSVHIIEGDHRTLLEGRGLESIINIIHSSLAEPRVSVREG

SEQ ID NO: 3 - protein, 2503 aa, Cricetulus griseus
MEEVVIAGMSGKLPESENLQEFWANLIGGVDMVTDDDRRWKAGLYGLPKRSGKLKDLSKFDASFFGVHPKQAHTMDPQLRLLLEVSYEAIVDGGINPASLRGTNTGVWVGVSGSEASEALSRDPETLLGYSMVGCQRAMMANRLSFFFDFKGPSIALDSACSSSLLALQSAYQAIRNGECPAALVGGINVLLKPNTSVQFMKLGMLSPEGTCKSFDDSGNGYCRSEAVVAVLLTKKSLARRVYATILNAGTNTDGCKEQGVTFPSGEAQEQLIQSLYRPAGLAPESLEYIEAHGTGTKVGDPQELNGIVRSLCASRQGPLLIGSTKSNMGHPEPASGLAALTKVLLSLENGVWAPNLHFHNPNPEIPALLDGRLQVVDRPLPVRGGNVGINSFGFGGANVHVILQPNTQQAPAPAPHAALPHLLHASGRTAEAVQGLLEQGRKHSQDMAFVSMLNDIAATPTAAMPFRGYTVLGVEGDVQEVQQVPASKRPLWFICSGMGTQWRGMGLSLMRLDSFRESILRSDEAVKPLGIKVSDLLLSTDESTFDDIVHAFVGLTAIQIALIDLLTSVGLKPDGIIGHSLGEVACGYADGCLSQREAVLAAYWRGQCIKDAHLPPGSMAAVGLSWEECKQRCPSGVVPACHNSEDTVTISGPQAAVSEFVEQLKQEGVFAKEVRTGGLAFHSYFMEGIAPMLLQALKKVIREPRPRSARWLSTSIPEAQWQSSLARTSSAEYNVNNLVSPVLFQEALWHVPEHAVLLEIAPHALLQAVLKRGVKSSCTIIPLMKRDHKDNLEFFLTNLGKVHLTGIDVNPNALFPPVDFPAPRGTPLISPHIKWDHSQTWDVPAAEDFPNGSCSSSATVYSIDASPESPDHYLVDHCIDGRVLFPATGYLYLVWKTLARNLSLSLEETPVVFEDVTIHQATILPKTGTVPLEVRLLEASRAFEVSENGNLIVSGKVYQWEDPDSKLFDHPHVLNPPESTPVSRLTQTEVYKELRLRGYDYGPHFQGIVEASLEGEQGKLLWKGNWVTFLDTMLQVSILGVSQQSLRLPVRVTAIHIDPATHLQKVYTLEGENQVADVTTSLCLDSTVSGGVRISRLHTTAAPRRQQEQLVPTLEKFIFTPHVEDGCLSENTTLQRELQLCKDLAQALQTKATQQGLKMTVPGLEGPPQHGLSRLLAAACQLQLNGNLQLELGEALAQERVLLPEDPLISGLLNSQALKACVDTALENLPSLKMKVVEVLSGEGRLYSRIPSLLNTQPMLQLEYTATDLHPEALKDVQAKLQQHDIAQGQWNPEDPAPSNLGALDLVVCSCAVATLGNPALALSNMVAALKEGGFLLMHTVLRGHSLGETLACLPSAVQPGPSLSQEEWESLFSKKGLHLVGLKKSFYGTALFLCRRATLQDNPLFLPVEDTSYQWVDSLKRILAESSSQPVWLTATDCPTSGVVGLVNCLRKEPGGHRIRCILLSNLSTSSHTPKMGPGSSELQKVLKNDLVMNVYRDGAWGAFRHFLLEQDKPEEQTAHAFVNVLTRGDLASIRWVCSPLKHAQPTSPGTQLCTVYYASLNFRDIMLATGKLPPDAIPGKWASRDCMLGMEFSGRDKCGRRVMGLVPAEGLATSVLLSPDFLWEVPSSWTLEEAASVPVVYTTAYYSLVVRGRVQRGETVLIHSGSGGVGQAAISIALSLGCRVFTTVGSAEKRAYLQARFPQLDDTSFANSRDTSFEQHVLLHTGGKGVNLVLNSLAEEKLQASVRCLAQHGRFLEIGKFDLSNNHPLGMAIFLKNVTFHGILLDALFEEANDSWREVAALLQAGIRDGVVKPLKCTVFPKDQVEDAFRFMAQGKHIGKVLVQVREEEPEAVLPGAQPTLIPAISKTFCPAHKSYIITGGLGGFGLELARWLVLRGAQRLVLTSRSGIRTGYQAKQVQEWRRQGIHVLVSTSNASSLEGARALITEATKLGPVGGVFNLAMVLRDAMLENQTPELFQDVNKPKYNGTLNLDRTTREACPELDYFVAFSSVSCGRGNAGQTNYGFANSAMERICEQRRHDGLPGLAVQWGAIGDVGIVLEAMGTNDTVIGGTLPQRIASCMEVLDLFLNQPYAVLSSFVLAEKKAVAQGDGEAQRDLVKAVAHILGIRDLAGVNLDSSLADLGLDSLMGVEVRQILEHEHDLVLPMREVRQLTLRKLEELSSKAGSASETTAPKSKNDTALKQTQLNLSTLLVNPEGPTLTRLNSVQSSERPLFLVHPIEGSTTVFHSLAAKLSVPTYGLQCTQAAPLDSIPDLAAYYIDCIKQVQPEGPYRVAGYSFGACVAFEMCSQLQAQQGPTPTHNSLFLFDGSHTYVLAYTQSYRARMTPGCEAEAEAEAICYFIKQFTDAEHNKVLEALLSLKSLEDRVTAAVDLITKSHHSLDRRELSFAALSFYQKLRAADQYKPKAKYHGNVTLLRAKTGGTYGEDLGADYNLSQVCDGKVSVHIIEGDHRTLLEGSGLESIINIIHSSLAEPRVSVREG

SEQ ID NO: 4 - protein, 2511 aa, Homo sapiens
MEEVVIAGMSGKLPESENLQEFWDNLIGGVDMVTDDDRRWKAGLYGLPRRSGKLKDLSRFDASFFGVHPKQAHTMDPQLRLLLEVTYEAIVDGGINPDSLRGTHTGVWVGVSGSETSEALSRDPETLVGYSMVGCQRAMMANRLSFFFDFRGPSIALDTACSSSLMALQNAYQAIHSGQCPAAIVGGINVLLKPNTSVQFLRLGMLSPEGTCKAFDTAGNGYCRSEGVVAVLLTKKSLARRVYATILNAGTNTDGFKEQGVTFPSGDIQEQLIRSLYQSAGVAPESFEYIEAHGTGTKVGDPQELNGITRALCATRQEPLLIGSTKSNMGHPEPASGLAALAKVLLSLEHGLWAPNLHFHSPNPEIPALLDGRLQVVDQPLPVRGGNVGINSFGFGGSNVHIILRPNTQPPPAPAPHATLPRLLRASGRTPEAVQKLLEQGLRHSQDLAFLSMLNDIAAVPATAMPFRGYAVLGGERGGPEVQQVPAGERPLWFICSGMGTQWRGMGLSLMRLDRFRDSILRSDEAVKPFGLKVSQLLLSTDESTFDDIVHSFVSLTAIQIGLIDLLSCMGLRPDGIVGHSLGEVACGYADGCLSQEEAVLAAYWRGQCIKEAHLPPGAMAAVGLSWEECKQRCPPGVVPACHNSKDTVTISGPQAPVFEFVEQLRKEGVFAKEVRTGGMAFHSYFMEAIAPPLLQELKKVIREPKPRSARWLSTSIPEAQWHSSLARTSSAEYNVNNLVSPVLFQEALWHVPEHAVVLEIAPHALLQAVLKRGLKPSCTIIPLMKKDHRDNLEFFLAGIGRLHLSGIDANPNALFPPVEFPAPRGTPLISPLIKWDHSLAWDVPAAEDFPNGSGSPSAAIYNIDTSSESPDHYLVDHTLDGRVLFPATGYLSIVWKTLARALGLGVEQLPVVFEDVVLHQATILPKTGTVSLEVRLLEASRAFEVSENGNLVVSGKVYQWDDPDPRLFDHPESPTPNPTEPLFLAQAEVYKELRLRGYDYGPHFQGILEASLEGDSGRLLWKDNWVSFMDTMLQMSILGSAKHGLYLPTRVTAIHIDPATHRQKLYTLQDKAQVADVVVSRWLRVTVAGGVHISGLHTESAPRRQQEQQVPILEKFCFTPHTEEGCLSERAALQEELQLCKGLVQALQTKVTQQGLKMVVPGLDGAQIPRDPSQQELPRLLSAACRLQLNGNLQLELAQVLAQERPKLPEDPLLSGLLDSPALKACLDTAVENMPSLKMKVVEVLAGHGHLYSRIPGLLSPHPLLQLSYTATDRHPQALEAAQAELQQHDVAQGQWDPADPAPSALGSADLLVCNCAVAALGDPASALSNMVAALREGGFLLLHTLLRGHPLGDIVAFLTSTEPQYGQGILSQDAWESLFSRVSLRLVGLKKSFYGSTLFLCRRPTPQDSPIFLPVDDTSFRWVESLKGILADEDSSRPVWLKAINCATSGVVGLVNCLRREPGGNRLRCVLLSNLSSTSHVPEVDPGSAELQKVLQGDLVMNVYRDGAWGAFRHFLLEEDKPEEPTAHAFVSTLTRGDLSSIRWVCSSLRHAQPTCPGAQLCTVYYASLNFRDIMLATGKLSPDAIPGKWTSQDSLLGMEFSGRDASGKRVMGLVPAKGLATSVLLSPDFLWDVPSNWTLEEAASVPVVYSTAYYALVVRGRVRPGETLLIHSGSGGVGQAAIAIALSLGCRVFTTVGSAEKRAYLQARFPQLDSTSFANSRDTSFEQHVLWHTGGKGVDLVLNSLAEEKLQASVRCLATHGRFLEIGKFDLSQNHPLGMAIFLKNVTFHGVLLDAFFNESSADWREVWALVQAGIRDGVVRPLKCTVFHGAQVEDAFRYMAQGKHIGKVVVQVLAEEPEAVLKGAKPKLMSAISKTFCPAHKSYIIAGGLGGFGLELAQWLIQRGVQKLVLTSRSGIRTGYQAKQVRRWRRQGVQVQVSTSNISSLEGARGLIAEAAQLGPVGGVFNLAVVLRDGLLENQTPEFFQDVCKPKYSGTLNLDRVTREACPELDYFVVFSSVSCGRGNAGQSNYGFANSAMERICEKRRHEGLPGLAVQWGAIGDVGILVETMSTNDTIVSGTLPQRMASCLEVLDLFLNQPHMVLSSFVLAEKAAAYRDRDSQRDLVEAVAHILGIRDLAAVNLDSSLADLGLDSLMSVEVRQTLERELNLVLSVREVRQLTLRKLQELSSKADEASELACPTPKEDGLAQQQTQLNLRSLLVNPEGPTLMRLNSVQSSERPLFLVHPIEGSTTVFHSLASRLSIPTYGLQCTRAAPLDSIHSLAAYYIDCIRQVQPEGPYRVAGYSYGACVAFEMCSQLQAQQSPAPTHNSLFLFDGSPTYVLAYTQSYRAKLTPGCEAEAETEAICFFVQQFTDMEHNRVLEALLPLKGLEERVAAAVDLIIKSHQGLDRQELSFAARSFYYKLRAAEQYTPKAKYHGNVMLLRAKTGGAYGEDLGADYNLSQVCDGKVSVHVIEGDHRTLLEGSGLESIISIIHSSLAEPRVSVREG

SEQ ID NO: 5 - protein, 2510 aa, Macaca mulatta
MEEVVIAGMSGKLPESENLQEFWDNLIGGVDMVTDDDRRWKAGLYGLPRRSGKLKDLSRFDASFFGVHPKQAHTMDPQLRLLLEVTYEAIVDAGINPASLRGTHTGVWVGVSGSEASEALSRDPETLVGYSMVGCQRAMMANRLSFFFDFKGPSIALDTACSSSMVALQSAYQAISSGQCPAAIVGGINVLLKPNTSVQFLRLGMLSPEGTCKAFDAEGNGYCRSEGVVAVLLTKKSLARRVYATILNAGTNTDGCKEQGVTFPSGEAQEQLIRSLYQSAGVAPESFEYIEAHGTGTKVGDPQELNGIARALCATRQEPLLVGSTKSNMGHPEPVSGLAALAKVLLSLEHGLWAPNLHFHSPHPEIPALLDGRLQVVAQPLPVRGGNVGINSFGFGGSNVHVILRPHTQPPPAPAPHASLPRLLRASGRTPEAVQELLEQGLQHSQELAFLSMLNDIAAIPTTAMPFRGYAVLGGEHSGPEVQQVPAGERPLWFICSGMGTQWRGMGLSLMRLDRFRDSILRSDEAVKPFGLKVSQLLLSMDESTFDDIVHAFVSLTAIQIGLIDLLSCMGLRPDGIIGHSLGEVACGYADGCLSQEEAVLAAYWRGQCIKEAHLPPGAMAAVGLSWEECKQRCPPGVVPACHNSKDTVTISGPQASVFEFMEQLRKEGVFAKEVRTGGMAFHSYFMEAIAPPLLQALKKVIREPKPRSARWLSTSIPEAQWHSSLARTSSAEYNVNNLVSPVLFQEALCHVPEHAVVLEVAPHALLQAVLKRGLKPGCTIIPLMKKDHRDNLEFFLTGIGRLHLSGIDANPNALFPPVEFPAPRGTPLISPLIKWDHSLAWDVPAAEDFPNGSGSPSAAVYNIDTSSESPDHYLVDHTIDGRVIFPATGYLCIVWKTLARALGLAVEQLPVVFEDVVLHQATILPKTGTVSLEVRLLEASRAFEVSQNGNLIVSGKVYQWEDPDPRLFNHPESPTPNPEEPLFLTQAEVYKELRLRGYDYGPHFHGILEASLEGESGRLLWKDNWVSFLDAMLQISILGLAKRSLPLPTRITAIHIDPATHRQKLYTLQDDAQVADVVVSRWLSITVAGGVHMSRVHTESAPRRQQDQQVPILEKFCFTPHVEEGCLSERAALQKELQLCKGLAQALQTKVTQQGLRMVVPGLDGAQVPQDPLQQGLPQLLSAACRLQLNGNLQLELAQVLAQKRPELSEDPLLSGLLDSPALRACLDTAVENMPSRKMKVVEVLAGHGHLYSRIPGLLGAQPLLQLSYTATDRHPQALEAAEAQLQQHDIAQGQWDPADPAPSTLGSTDLLVCNCAVAALGDPASALSNMVATLREGGFLLLHTLLRGHPLGETVAFLTSAEPQYGQGILSQDAWESLFSSVSLRLVGLKKSFYGSALFLCRRPAPQDSPIFLPVDDTSFRWVESLKGILADEDSSRPVWLKAVNCATSGVVGLVNCLRQEPGGHRLRCVLLSNLSSTSRVPEVDPGSAELQKVLQGDLVMNVYRDGAWGAFRHFLLEEDKPEEPTAHAFVTTLTRGDLSSIRWVCSSLRHAQPSRPGAQLCTVYYASLNFRDIMLATGKLSPEAIPGKWASQDNLLGMEFSGRDPSGKRVMGLVPAEGLATSVLLSPDFLWDVPSNWTLEEAASVPVVYCTAYYSLVVRGRVRPGETVLIHSGSGGVGQAAIAIALSLGCRVFTTVGSSEKRAYLQARFPQLDSTSFANSRDTSFEQHVLRHTGGKGVDLVLNSLAEEKLQASVRCLAQHGRFLEIGKFDLSQNHPLGMAIFLKNVTFHGILLDALLDGSAEWQEVAALLQAGIRDGVVQPLKCTVFPGAQVEDAFRYMAQGKHIGKVLVQVLAEEPEAVLKGAKPTLMSAISKTFCPAYKSYIIAGGLGGLGLELAQWLIQRGAQKLVLTSRSGVRTGYQAKQVRQWRRQGVQVLVSTSNISSLEGARGLIAEAAQLGPVGGIFNLTMVLRDAMLENQTPEFFQDVCKPKYSGTLNLDRVTREACPELDYFVVFSSVSSGRGNAGQSNYGFANSAMERICEKRRHEGLPGLAVQWGAIGDVGILADTVNIHATVIGGTLPQRVASCLEVLDLFLNQPHMVLSSFVLAEKAAAYRDRDGEQDLVKAVAHILGIRDLAAINLDSSLADLGLDSLMSVEVRQTLERELNLVLSMREVRQLTLRRLQELSLKADAANDLASPTPKEDGPAQQQTQLNLRSLLVNPEGPTLMRLNSVQSSERPLFLVHPIEGSTTVFHSLASRLSIPTYGLQCTRAAPLDSIHSLAAYYIDCIRQVQPEGPYRVAGYSYGACVAFEMCSQLQAQQNPAPTHNSLFLFDGSHTYVLAYTQSYRAKLTPGCEAEAETEAICFFVQQFTDMEHNRVLEALLPLKGLEERVAAAVDLIIKSHQGLDRQELSFAALSFYYKLRAAEQYTPKAKYHGNVMLLRAKTGGAYGEDLGADYNLSQVCDGKVSVHVIEGDHRTLLEGSGLESIVSIIHSSLAEPRVSVREG

SEQ ID NO: 6 - protein, 2513 aa, Bos taurus
MEEVVITGMSGKLPESENLEEFWANLIGGVDMVTDDDRRWKAGLYGLPRRSGKLKDLSRFDASFFGVHPKQAHNMDPQLRLLLEVTYEAIVDAGINPASIRGTNTGVWVGVSGSEASEALSRDPETLVGYSMVGCQRAMLANRLSFFFDFKGPSITLDTACSSSLLALQRAYQAIQRGECAMAIVGGVNIRLKPNTSVQFMKLGMLSPEGTCKFFDASGNGYCRAKAVMAILLTKKSLARRVYATILNAGTNTDGCKEKGVTFPSGEAQEQLISSLYKPAGLDPETLEYVEAHGTGTKVGDPQELNGIVQALCGTRQSPLRIGSTKSNMGHPEPASGLAALAKVLLSLEHGLWAPNLHFHNPNPKIPALQDGRLQVVDRPLPVLGGNVGINSFGFGGSNVHVILQPNSQPLPPPAPHAALPRLLRASGRTLEGVQGLLELGLQHSQNLAFVSMLNDIATPSPAAMPFRGYAVLGSQGGSQKVQQVLAGKRPLWFICSGMGTQWRGMGLSLMRLSRFRDSILRSDEAVKPLGLQVSQLLLSTDEAIFDDMVISFVSLTAIQIALIDLLTSMGLQPDGIIGHSLGEVACGYADGCISQEEAILSAYWRGQCIKEANIPPGAMAAVGLTWEECKQRCPPGIVPACHNCIDTVTISGPQASMLEFVQQLKQEGVFAKEVRTGGMAFHSYFMDAIAPMLLQQLKKVIREPQPRSPRWLSTSIPETQWQESLARTFSAEYNVNNLVSPVLFQEALWRVPEDAVVLEIAPHALLQAVLKRGLKSSCTIIPLMKKDHRDNLEFFLSNVGQLYLTGIDVNPNGLFPPVEFPAPRGTPLISPHIKWDHSQTWDVPTAEDFPSGSSSSSATIYKIDINPESPDHYLVDHCIDGRIIFPGTGYLCLVWKTLARALDQNMEHTPVVFEDVTLHQAVILPKTGIVLLKVRLLEASCTFEVSENGNLIASGKVYQWEDPNPKLFDNRYGPDPATPVDPTTAIHLSRGDVYKELQLQGFNYGPYFQGILEASSEGNTGQLLWKDNWVTFMDTMLQMSILAPSKRSLRLPTRITAIYIHPATHQQKLYTLQDKTQVADVVINRCLDTTVAGGIYISRIHTSVAPRHQQEQLVPILEKFCFTPHVETGCLAGNLALQEELQLCVGLAQALQTRVAQQGIKMVVPGLDGAQAPQEAPQQGLPRLLATACQLQLNGNLQMEMGQILAQERALLCDDPLLSGLLNSPALKACVTLALENMTSLKMKVVLAGDGQLYSRIPTLLNTQPLLELDYTATDRHPQALEAAQAKLQQLDITQGQWDPSDPAPSNLGGANLVVCNYALASLGDPATAVGNMVAALKEGGFLLLHTLLRGHPLGETVTFLTCPEPQQGQRHLLSQDEWERLFAGASLHLVALKKSFYGSVLFLCRRLAPLDSPIFLPVEDTSFQWVDSLKNILADSSSRAVWLMAVGCTTSGVVGLVNCLRKEPDGHRIRCVLVSNLNSTSPIPETDPKSLELQKVLQSDLVMNVYRDGAWGAFRHFPLEQDKPEEQTEHAFINVLTRGDLSSIRWVCSPLRHSQPTAPGFQLCTIYYASLNFKRNHAGHGQAVPRRHPRNWASRNCLLGMEFSGRDASGKRVMGLVPAEGLATSTLVPQSFLWDVPSNWTLEEAASVPVVYSTAYYALMVRGRMQPGETVLIHSGSGGVGQAAIAIALSLGCRVFPLVGSAEKRAYLQSRFPQLNETSFANSRDTSFEQHVLWHTAGKGADLVLNSLAEEKLQASVRCLAQHGRFLEIGKFDLSKNHPLGMAIFLKNVTFHGILLDSLFEENNTMWQEVSTLLKAGIRKGVVQPLKRTVFPRTQAEDAFRYMAQGKHIGKVVIQVREEEQEAVLHGTKPTQMVALCKTFCPAHKSYIITGGLGGFGLELAHWLVERGAQKLVLTSRSGIRTGYQARQVHEWRRQGVQVLVSTSDVSTLDGTRSLITEAAQLGPVGGIFNLAVVLRDAMLDNQTPEFFQDVNKPKYNGTLNLDRVTREACPELDYFEVFSSVSCGRGNAGQTNYGFANSTMERICEKRRHDGLPGLAVQWGAIADVGLLMELKGTKDKAIGGTLPQRITSCMEVLDLFLNQPHPVLSSFVLAEKATSRGPSGSHQDLVKAVTHILGIRDLATVNLDSSLSDLGLDSLMGVEVRQMLEREHNLLLSMREIRQLTIHKLQEISAQAGTADELTDSTPKFGSPAQSHTQLNLSTLLVNPEGPTLTRLNSVQSSERPLFLVHPIEGSTTVFHSLATKLSIPTYGLQCTGAAPLDSIQSLATYYIECIRQVQPEGNYRIAGYSYGACVAFEMCSQLQAQQNAGPTNNSLFLFDGSHTFVMAYTQSYRAKLNPGCEAEAEAEAMCFFMQQFTEAEHSRVLEALLPLGDLEARVAATVELIVQSHAGLDRHALSFAARSFYHKLRAAEEYTPRATYHGNVTLLRAKMGSAYQEGLGADYNLSQVCDGKVSVHIIEGDHRTLLEGSGLESILSIIHSSLAEPRVSVREG

SEQ ID NO: 7 - protein, 2514 aa, Capra hircus
MEEVVIAGMSGKLPESENLEEFWANLIGGVDMVTDDDRRWKAGLYGLPRRSGKLKDLSRFDASFFGVHPKQAHNMDPQLRLLLEVAYEAIVDAGINPASIRGTNTGVWVGVSGSEAAEALSRDPETLVGYSMVGCQRAMMANRLSFFFDFKGPSIALDTACSSSLLALQRAYQAIQRGECAMAIVGGINILLKPNTSLQFMKLGMLSPEGTRKSFDASGDGYCRAEAVMAVFLTKKSLARRVYATILNAGTNTDGCKKQGVTYPSGEAQEQLISSLYKPAGLDPETLEYIEAHGTGTKVGDPEELNGITQALCGTRQGPLLIGSTKSNMGHPEPASGLAALAKVLLSLEHGLWAPNLHYHNPNPKIPALQDGRLQVVDRPLPVLGGIVGINSFGFGGSNVHVILQPNSQPPPPPGPHAALPRLLRASGRTLEGVQGLLELGLQHSQNLAFVSMLNDIAAPSPAAMPFRGYAVLGSQEGSQEVQQVPTSKRPLWFICSGMGTQWRGMGLSLMRLSSFRDSILRSDEAVKPLGLRVSQLLLSADDIFDDIIVSFVSLTAFQIALIDLLTSMGLRPDGIIGHSLGEVACAYADGCISQEEAILSAYWRGQCIKEANIPPGAMAAVGLTWEECKQRCPPGIVPACHNSIDTVTISGPQASMLEFVKQLKQEGVFAKEVQTGGMAFHSYFMDAIAPTLLQQLKKVIREPQLRSPRWLSTSIPESQWHESLARTFSAEYNVNNLVSPVLFQEALWHVPENAVVLEIAPHALLQAILKRGLQPSCTIIPLMKKDHRDNLEFFLSNVGQLYLTGIDVNPNGLFPPVEFPAPRGTPLISPHIKWDHSQTWDVPAAEDFPNGSSSSSATVYKIDISPESPDHYLVDHCIDGRVLFPATGYLCLVWKTLARALDQNTEHTPVVFEDVMLHQATLLPKTGTVLLEVRLLEASCTFEVSEKGSLIVSGKVYQWEDPDPKLFDNRYGTEPATPVDPTTAIHLRCGDVYKELQLQGFNYGPNFQGILETSSEGNMGQLLWKDNWVTFMDTMLQMSILAPGQRSLRLPTRITAIYIHPATHQQKLYTLQDGTQVADVVMNRCLDTTVAGGVYISRIHTSVAPRHQQEQPVPILEKFCFTPHVESGCLAGNLALQEELQLCVGLAQALQTKVAQQGIKMVVPGLDGTQASQEAPQQGLPQLLATACQLQLNGNLQMGMGQILAQERALLCDDPLLSGLLNSPALKACVDTALENMTSLKMKVVEVLAGDGQLYSRIPALLNTQPLLELDYIATDRHPQALEAAQAKLQQLNITQGQWDPSDPAPSNLGGANLVVCNCALASLGDPATAVGNMVAALKEGGFLLLHTLLRGHPLGETVTFLTCPEPQQGQRHLLSQDEWESLFAGTSLHLVALKKSFYGSVLFLCRRLAPRDSPIFLPVEDTSFQWVDSLKNILADSSSRPVWFMAVGCTTSGVVGLVNCLRKEPDGHRIRCVLVSNLNSTSPIPEIAPKSLELQKVLQSDLVMNVYRDGAWGAFRHFLLEQDKPEEQTEHAFINVLTRGDLSSIRWVCSPLRHSQSTGPGVQLCTIYYASLNFRDIMLATGKLSPDAIPGNWASRNCMLGMEFSGRDASGKRVMGLVPAEGLATSTLVPQSFLWDVPSNWTLEEAASVPVVYSTAYYALIVRGRMQPGETVLIHSGSGGVGQAAIAIALSLGCCVFTTVGSAEKRAYLQSRFPQLNETSFANSRDTSFEQHVLWHTAGKGVDLVLNSLAEEKLQASARCLAQHGRFLEIGKFDLSNNHPLGMAIFLKNVTFHGILLDALFEENSTMWQEVSSLLKAGIREGVVQPLKRTVFPRTQVEDAFRYMAQGKHIGKVVIQVREEEQKAVLHGTKPTQMAALCKTFCPAHKSYVITGGLGGFGLELAHWLVERGAQKLVLTSRSGIRTGYQARQVREWRRQGVQVLVSTRDVSSLDGTQRLITEAAQLGPVGGVFNLAVVLRDAMLDNQTPEFFQDVNKPKYNGTLNLDRVTREACPELDYFVVFSSVSCGRGNAGQTNYGFANSTMERICEKRRHDGLPGLAVQWGAIADVGILVELKGTNDKAIGGTLPQRITSCLEVPDFFLNQPHPVLSSFALAEKAASRGPSGSQQDLVKAVAHILGIRDLATVNPDSSLSDLGLDSLMGVEVRQMLERERSLTLSMREIRQLTIRKLQEISAQAGTADELTNSTHKLSSPAQSQTQLNLSTLLVNPEGPTLTRLNSVQSSERPLFLVHPIEGSTTVFHSLAAKLSIPTYGLQCTRAAPLDSIQSLAAYYIECIRQVQPEGPYRIAGYSYGACVAFEMCSQLQAQQSAGPTNNSLFLFDGSHTFVMAYTQSYRAKMNPGCEAEAEAEAMCFFMRQFMEAEHSRVLEALLPLGDLEARVAATVELIVQRHAGLDRHALSFAARSFYHKLRAAEQYTPRATYHGNVTLLRAKMGGAYGEGLGADYNLSQVCDGKVSVHIIEGDHRTLLEGSGLESILSIIHSSLAEPRVSVREG

SEQ ID NO: 8 - protein, 2489 aa, Equus caballus
MEEVVIAGMSGRLPESENMQEFWANLIGGVDMVTDDDRRWKAGLYGLPRRSGKLKDLSKFDASFFGVHPKQAHTMDPQLRLLLEVTYEAIVDGGINPALLRGTHTGVWVGVSGSEASEALSRDPETLLGYSMVGCQRAMMANRLSFFFDLKGPSITLDTACSSSLLALHNAYQAIRSGECPAAIVGGINVLLKPNTSVQFMKLGMLSPEGACKSFDEAGNGYCRSEAVVAVLLTKKSLARRVYATILNSGTNTDGSKEQGVTFPSGDAQEQLMSSLYKPAGVAPESLEYLEAHGTGTRVGDPQELKGVVRALCATRQDPLLIGSTKSNMGHPEPASGLAALAKVLLSLEHGLWAPNLHFHSPNPEIPALRDGRLQVVDRPLPIRGGNVGINSFGFGGSNVHVILQPNSRLPLVPTPHVALPCLLRASGRTSEAVLGLLEQGRQHSQDLAFVSMLNDIAATPPSAMPFRGYAVLGGEGDAQEVQQVSTGQRPLWFICSGMGAQWRGMGLSLMRLGTFRDSILRSDKAVKPLGLQVSDLLLSADEATFDDTVPGFVSLTAIQIALIDLLTSMGLRPDGIIGHSLGEVACGYADGCVSQEEAILAAYWRGQCIKEANIPPGAMAAVGLSWEECKQRCPPGVVPACHNSKDTVTISGPQAAVSEFVEQLKQEGVFAKEVRTGGLAFHSYFMDSISHTLLQALKKVIREPRPRSVRWLSTSIPEAQWQSSLARTFSAEYNVNNLVSPVLFQEALCHVPEHAVVLEIAPHALLQAVLKRGLKPSCTIVPLMKKDHRDNLEFFLSNVGRLHLMGIDVNPNGLFPPVEFPAPRGTPLISPHIKWDHSQTWYVPSAKDFPSGSSCSSSTVYNIDASPESPDHYLVDHCIDGRTLFPATGYLCLVWRTLAHALGENLEQMPVVFEDVTLYQATILPKTGTMPLEVRLLEASHTFEVSENGTLIVSGKVYQWDNPNPKLFDNRDSLDPADPTDPTATFHLAQGDVYKELRLRGYDYGPHFQGILKANLEGNTGQLLWKDNWVTFLDTMLQMSILGSAQRSLRLPTRIAAIHIDPATHQQKVYTLQGEAQVADLVVDSCLSSTVAGGAIISRLHTSLAPRRQQEQLAPTLEKFCFTPHVEGGCLAGSATLQEELQLCKGLAQALQVKVAQQGLKMVVPGLDGAQVPRESPQQGLPRLLAAACQLQLNGNLQLELGQVLAQESPLLCDDPLLSGLLDSPALKACVDTALENVASLRMKVVEVLAGDGHLYSRIPALLTTQPMLQLDYTATDRHAQALKAAQAKLQQHHVAQGQWDPMDPAPSSLGATDLLVCNCAVATLGDPATALGNMAAVLKEGGFLLLHTLLRGYPLGEMVAFLTCPEPQRGRQGLLSQDEWESLFAGASLRLVALKKSFYGSVLFLCRRPAPQDSPIFLPVEDMSFRWVDSLKNILADLSSRPVWLTAVSCSTSGVIGMANCLRKEPGGHRIRCILVSNLSNTSPVPKMDPSSSELQKVLQGDLVMNVYRDGAWGTFRHFPLEQDQPEEQTEHAFINVLTRGDLSSIRWVCSPLRHAQHPGPGLQLCTVYYASLNFRDIMLATGKLSPDAIPGKWAARDCMLGMEFSGRDASGKRVMGLVPAEGLATSVLLSQDFLWDVPSCWTLEEAASVPVVYTTAYYSLVVRGRVRRGETVLIHSGSGGVGQAAIAIALSLGCRVFTTVGSAEKRAYLQARFPQLNDTSFANSRDTSFEQHVLRHTAGKGVDLVLNSLAEEKLQASVRCLAQHGRFLEIGKFDLSNNHPLGMAVFLKNVTFHGILLDALFDETSSDWQEVVALVRAGIQDGVVQPLKCTVFPKTQVEDAFRYMAQGKHIGKVVVQVREEEPEAVLQEVKPTRMVALSKTFFPAHKSYVVVGGLGGFGLELAQWLVLRGAQKLVLTSRSGIRTGYQAKQVREWRRQGVQVLVSTCNASSLDGARGLIAEAAQLGPVGGVFNLAMVLRDAMLENQTPELFQDVNKPKYNGTLNLDRVTRETCPELDYFVAFSSVSCGRGNAGQTNYGFANSTMERICEKRRHDGLPGLAVQWGAIGDVGIILEAMGANDTVIGGTLPQRIASCLEVLDLFLNQPHPVLSSFVLAEKKAAAHSDSSSQQDLVKAVAHILGIQDLATINLDSSLVDLGLDSLMGVEVRQTLEREHDMVLSMRDIQQLTLRKLQELSSQTCMADELAAPTPKEDGLTRQQAQLNLSTLLVNPEAPTLTRLNSVQSSERPLFLVHPIEGSITVFHSLATKLSIPTYGLQCTKAAPLDSIQSLAAYYIECIRQVQPEGPYRIAGYSYGACVAFEMCSQLQAQQSSAPAHNSLFLFDGSHAYVLAYTQSYRAKLTPGCEAEAETEAMCFFIQQFTDAEHSRVLEALLPLKGLEERVVAAVDLIVQNHAGLDRRVLSFAARSFYYKLRAAEQYMPRATYHGNVTLLRAKTGSAYSEDLGADYNLSQKHDSNCCVDFEISCQLSV

SEQ ID NO: 9 - protein, 2655 aa, Felis catus
MALPAALCEALSQEHPSSRLQRLQGLLGSRYEAAGPWGGWSPQARAPEVPGQCQRPEGPVLPVKSEGWLDQCGLPHTPEASVLASPGRRSWPPGSGSHRSQTRRWCCGVRKPGERLQPGGLAAGSDQRQAPTLLPLHRAAMEEVVIAGMSGKLPESENMEEFWANLIGGVDMVTDDDRRWKAGLYGLPKRTGKLKDLSKFDASFFGVHPKQAHTMDPQLRLLLEVTYEAILDGGINPATLRGTHTGVWVGVSGSEASEALSRDPETLVGYSMVGCQRAMMANRLSFFFDFKGPSIALDTACSSSLLALQNAYQAIRRGECPAAIVGGLNLLLKPNTSVQFMKLGMLSPDGICKAFDESGDGYCRAEAVVAVLLTKKSLARRVYATILNAGTNTDGCKEQGVTFPSGEVQEQLIRSLYEPAGLSPESLEYIEAHGTGTKVGDPQELNGIARALCPSRQEPLLIGSTKSNMGHPEPASGLAALAKVLLSLEHGLWAPNLHFRSPNTQIPALQDGRLQVVQQPLPVRGGNVCINSFGFGGSNVHVILRPNMRPPLAPTRHASLPRLLRASGRTPEAVHCLLEQGRRHSQDLAFVSMLNDIAAISPTAMPFRGYTVLGGKGGSQEVQLVAAGKRPLWFICSGMGAQWCGMGLSLMRLGSFRDSILRSDEAVKPLGLQVSELLLSTDEATFDDIIHAFVSLTAIQIALIDLLNSMGLRPDGIIGHSLGEVACGYADGCLSQEEAILAAYWRGQCIKETNIPPGTMAAVGLSWEECKQRCPPGVVPACHNSEDTVTISGPQAEVAAFVAELKREGVFAKEVRTGGMAFHSYFMDSIAPTLLQALKKVIREPRPRSARWLSTSIPEAQWQGSLARTFSAEYNVNNLVSPVLFQEALWHVPGDAVVLEIAPHALLQAVLKRGLKSSCTIVPLMKKDQRDNLEFFLSNVGKLHLLGFDVNPNGLLPPVEFPVPRGTPLISPHIKWDHSQTWDVPTAKDFPSGSSGSSASTVCNISISPESPDHYLADHCIDGRVLFPATGYLCLVWKTLARTLSQNMEQVPVAFEDVTLHQATVLPKTGTVPLEVRLLQASRTFEVSENGNLIVSGKVYQWEDPDTKLFDSRDGLDATDPMATFHLSQRDVYKELRLRGYDYGPHFQGILEANLEGNAGRLLWKNNWVTFLDAMLQTSILGLAQRSLRLPTRITSVRIDPATHQRRVYSLQGEAQAVNVLVNRCLNSTVAGGVLVSGLHASMAPRRQQEQFAPILEKFCFTPHTEEGLLAGDAALQEGLQLCRGLAQALQTKVAQQGLKMVVSGLDGAQAPQEPPKQGLPRLLAAACQLQLNGGLQLELGQLLAQQRPLLQDDPLLSGLLASPALKACVDTALENMPSLKMKVVEVLAGDGRLYSHIPALLNTQPMLQLEYTATDRHPQALEAVQAKLQQHGIAQGQWDPADHAPGSLGSADLLLCNCAVASLGDPAVAVGNMGAALKEGGFLLLHALLKGHPLGETVAFLTCPEPQRGQQSLLSQDQWESLFAGASLHLVALKKSFYGSVLFLCRRPVLWDSPVFLPVEDPSFQWVNSLKNILADSSQQPVWLTATSCPDSGVVGLVNCLRREPGGHRIRCVLVSNLSSTSSTPSLDPGSSELQKVLRGDLVMNVYRDGAWGAFRHFPLERGLPEEQTEHAFVNVLTRGDLSSIRWVCSPLRHTQLTGPGTHLCAVYYASLNFRDIMLATGKLSPDAIPGKWARHDCLLGMEFSGRDASGKRVMGLVPAEGLATSVLLSQDFLWEVPSSWTLEEAASVPVVYTTAYYSLVVRGRVQPGETVLIHSGSGGVGQAAIAIALSLGCRVFTTVGSAEKRAYLQARFPQLDDTSFANSRDTSFEQHVLRHTAGKGVDLVLNSLAEEKLQASVRCLAQHGRFLEIGKFDLSNNHLLGMAVFLKNVTFHGVLLDSLMDEGGNSWQEVAALLKAGIRDGVVQPLKCTVFPKDRVEDAFRYMAQGKHIGKVVVQVRREEPEAVLRETGPTLMAAVSKTYCPAHKSYVITGGLGGLGLELAQWLVLRGARKLVLTSRSGIRTGYQAKQVREWRRQGIQVLVSTSNASSLDGAQSLIDEATQLGPVGGVFNLAVVLRDAMLENQTPELFEDVVRPKYSGTVNLDRVTRAACPELDYFVAFSSVSCGRGNAGQTNYGFANSTMERVCEKRQHDGLPGLAIQWGAVGDVGIVLESMGSNDVVIGGTLPQRIASCLEVLDVFLNQPHPVLSSFVLAEKKATAHNDSSSRQDPMEAVAHILGIRDLATVNLDSSLADLGLDSLMGVEVRQMLEREHDLVMSMRDIRQLTLRKLQELSSKAGTANELAAPTPKEDTPAGQQAQLNLSTLLVNPEGPTLTRLNSVQSSERPLFLVHPIEGSITVFRSLASKLSIPTYGLQCTRAAPLDSIQSLAAYYIECIRQVQPEGPYRIAGYSYGACVAFEMCSQLQAAQQGPTPAHNSLFLFDGSHTYVLAYTQSYRAKLTPGCEAEAEAEAMCFFVQQFTDMEHNRVLEALLPLKSLEERVAATVDLITRSHAGLDPRELSFAARSFYHKLRAAEQYIPRATYHGNVTLLRTKTGSVYSEGLGADYNLSQVCDGKVSVHVIEGDHRTLLEGSGLETILSIIHSSLAEPRVSVREG

SEQ ID NO: 10 - protein, 2512 aa, Sus scrofa
MEEVVIAGMSGKLPESENLEEFWANLIGGVDMVTADDRRWKAGLYGLPRRMGKLKDLSRFDASFFGVHSKQANTMDPQLRMLLEVTYEAIVDGGINPASLRGTSTGVWVGVSSSDASEALSRDPETLVGYSMIGCQRAMMANRLSFFFDFKGPSITIDTACSSSLLALQSAYQAIRGGECSAAVVGGLNVLLKPNSSLQFMKLGMLSQDGTCRSFDAEGTGYCRAEAVVAVLLTKKSLARRVYATILNAGTNTDGSKEQGVTFPSGDVQEQLIRSLYAPAGPDPESLEYIEAHGTGTKVGDPQELNGIVNALCATRREPLLIGSTKSNMGHPEPASGVAALIKVLLSLEHGVWAPNLHYHTPNPEIPALQDGRLQVVDRPLPIRGGNVGINSFGFGGSNVHVILQPNSRPAPPPAQHAALPRLLQASGRTLEAVQTLLEQGLRHSRDLAFVGMLNEIAAVSPVAMPFRGYAVLGGEAGSQEVQQVPGSKRPVWFICSGMGAQWQGMGLSLMRLDRFRDSILRSDQALKPLGLRVSDLLLSTDEAVLDDIVSSFVSLTSIQIALIDLLTSLGLQPDGIIGHSLGEVACGYADGCLTQEEAVLSSYWRGYCIKEANVLPGAMAAVGLSWEECKQRCPPGIVPACHNSKDTVTISGPQAAMSEFLQQLKREDVFVKEVRTGGIAFHSYFMESIAPTLLRQLRKVILDPKPRSKRWLSTSIPEAQWQGSLARTFSAEYSVNNLVSPVLFQEALQHVPAHAVVVEIAPHALLQAVLKRSLESSCTIIPLMKKDHRDNLEFFLSNVGRLHLAGVSVNPNGLFPPVEFPAPRGTPLISPHXKWDHSQAWDVPSAADFPSGSSCSSVAVYKFDVSPESPDHYLVDHCIDGRVLFPGTGYLWLTWKTLARALSQNLEETPVVFEDVTLHQATILPKTGTVSLEVRLLEASHAFEVSDSNGSLIASGKVYQWESPDPKLFDTRAAVDPADSTAEFRLSQGDVYKDLRLRGYDYGPFFQLVLESDLEGNRGRLQWNDSWVSFLDAMLHMSILAPGQLGLYLPTRFTSIRIDPVTHRQKLYTLQDTTQAADVVVDRNLNTVVAGGALFLGAHSSVAPRRPQEHLKPILEKFCFTPHVESGCLAGNTALQEELQLCRGLAQALQTKVAQQGLKMVVPGLDGAQAPREAPQQSLPRLLAAACQLQLNGNLQLELGQVLAQERPLLCDDPLLSGLLDAPALKACVDTALENMASPKMKVVEVLAGDGQLYSRIPALLNTQPVMDLDYTATDRNPQALEAAQAKLEQLHVTQGQWDPANPAPGSLGKADLLVCNCALATLGDPAVAVGNMAATLKEGGFLLLHTLLAGHPLGEMVGFLTSPEQGGRHLLSQDQWESLFAGASLHLVALKRSFYGSVLFLCRQQTPQDSPVFLSVEDTSFRWVDSLKDILADASSRPVWLMAVGCSTSGVVGMVNCLRKEPGGHRIRCVLVSNLSSTSPAPEMHPSSSELQKVLQGDLVMNVYRDGAWGAFRHFPLEQDRPEKQTEHAFVNVLSRGDLSSIRWVCSPLHYALPASCQDRLCSVYYTSLNFRDVMLATGKLSPDSIPGKWLTRDCMLGMEFSGRDASGRRVMGMVPAEGLATSVLLLQHATWEVPSTWTLEEAASVPIVYTTAYYSLVVRGRMQPGESVLIHSGSGGVGQAAIAIALSRGCRVFTTVGSAEKRAYLQARFPQLDETCFANSRDTSFEQHVLRHTAGKGVDLVLNSLAEEKLQASVRCLAQHGRFLEIGKFDLSNNHALGMAVFLKNVTFHGILLDSLFEEGGATWQEVSELLKAGIQEGVVQPLKCTVFPRTKVEAAFRYMAQGKHIGKVVIQVREEEQGPAPRGLPPIALTGLSKTFCPPHKSYVITGGLGGFGLQLAQWLRLRGAQKLVLTSRSGIRTGYQARQVREWRRQGVQVLVSTSNASSLDGARSLITEATQLGPVGGVFNLAMVLRDAVLENQTPEFFQDVSKPKYSGTANLDRVTREACPELDYFVIFSSVSCGRGNAGQANYGFANSAMERICEKRRHDGLPGLAVQWGAIGDVGVVLETMGTNDTVIGGTLPQRIASCLEVLDLFLSQPHPVLSSFVLAEKKAAAPRDGSSQKDLVKAVAHILGIRDVASINPDSTLVDLGLDSLMGVEVRQILEREHDLVLSMREVRQLSLRKLQELSSKTSTDADPATPTSHEDSPVRQQATLNLSTLLVNPEGPTLTRLNSVQSAERPLFLVHPIEGSITVFHGLAAKLSIPTYGLQCTGAAPLDSIQSLASYYIECIRQVQPEGPYRIAGYSYGACVAFEMCSQLQAQQSATPGNHSLFLFDGSHTFVLAYTQSVRAKMTPGCEAEAEAKAMYFFVQQFTDMEQGKVLEALIPLQGLEARVAATVDLITQSHAGLDRHALSFAARSFYQKLRAAENYWPQATYHGNVTLLRAKTGGAYGEDLGADYNLSQVCDGKVSVHVIEGDHRTLLEGSGLESILSIIHSCLAEPRVSVREG

SEQ ID NO: 11 - protein, 2507 aa, Cuculus canorus
MEEVVIAGMAGKLPESANLQEFWENLMNGVDMVTEDDRRWKPGIYGLPRRNGKLKDLTKFDASFFGVHPKQAETMDPQLRMLLEVSYEAILDAGINPATLRGTDTGVWIGTGGSEAGEALSQDPEELSGYSMTGCQRAMLANRLSYFYDIKGPSVTIDTACSSSLVAMENAFKAIRAGQCHTALVGGCSLLLKPNTSVQFMKLGLLSPNGVCKSFDASGDGYCRSEAIVVLFLTKRSLAKRIYATIVNAGINADGFKEQGVMFPSGEMQQKLASSLLKESGIRPEEVEYVETHGTGTKIGDPQELNGITNVLCRCERAPLLIGSVKSNMGHSEPASGVAALAKVTGGLRRKNGRGQQCVNIPALHDGSMQVVCKPTPVKGGFVSINSFGFGGANANVILKPNMKKQQPVETSNVPRLIQFCGRTQEAVEVLIEESKKHAECIPFISLLSDISGIPASSMPYRGYTILGSESDIREVQQVQSTGRPLWYICSGMGTQWKGMGLSLMKLDLFRQSVLRSDEALKHTGLKVSELLLNEDENTFDDTVHAFVGLAAIQIAQIDILKAAGLEPDGIVGHSVGELACGYADNSLSHEEAILAAYWRGRCVKDAKLPPGGMAAVGLSWEECKQICPPNVVPACHNSEDTVTVSGPLGAVSEFVAKLKKDGVFAKEVRTSGVAFHSHYMASIAPVLLSALKKVIPHPKPRSPRWISTSIPESQWQSDLARYSSAEYHVNNLVNPVLFHEGLSHVPGNALVVEIAPHALLQAILKRSLKPTCIILPLMKKEHKNNLEFFLTQLGKFHMSGVNFNGNNLFPRVEYPVPVETPLISPHIKWDHSQEWYVPQAKDFPSGSKGTSSASVYNIDISPESPDHYLVDHCIDGRVLFPATGYLVLAWRTLARSLGMTIEKMPVTFEDVTIHQATILPKKGAVQLEVRLMPVSHCFEVSGNGNLAVSGKIFVLENDAAKKLDNQPVDCGTQVDVSSKVNLLKEDIYQELHLRGYNYGPNFQGVLEWNSEGTKSKVLWNGNWVTFLDTLLHVVILVESGRSLRLPTRIRTMSIDPVLHQERVCQYKDDVKAIDVVTDRCLASVRAGGVQFSGLHASVAPRRQQERIPPTLEKFCFVPYTEKNCLSSSVHLHDYLKQCKDLIQNLVNKVVVHGIKLVIPGLETADPDAEPLSVQKGLQHILAEMRKLEPNGNLHSELQQIVTREKMHLRDDPLLNGLLDSSELKTCLDVAVENVSSRRMKIIEVLAGSGQLFSRVKSVLTTQPLLQPDYIATDRSLEALSAAETELQDAGVVFSQWDPSSPPAGNLTDADLVVYNCSSVTENTPEIFSNLAAAVKEEGFVLIHTLLRGETVGEFVSFLTSPDLQQKHQFLSEAQWDSLFNSASLNLVAMKKSFFGSVIFLCRRRAPAKTPIFLPVDENDFKWVESLKGILAEQSEQPVWLTATSCGISGILGMVNCLRLEAEGHRIRCLFVSNLKPSSVVPPTSPSCPEMQNIVQKDLVMNVYRDGTWGSFRHLPLQQAQPQELTEYAYVNVLTRGDLSSLRWIASPLRHFQRTNPDVQLCKVYYSSLNFRDIMLATGKLPPDAIPGNWALQQCMLGMEFSGRDMSGRRVMGLLPAKGLATVVDCDKKFLWEVPKNWTLEEAASVPVVYATAYYALVVRGGMKKGESVLIHSGSGGVGQAAIAIALSMGCRVFATVGSTEKREYLQARFPQLDANSFASSRNTSFEQHIMRVTKGKGVNLVLNSLAEEKLQASLRCLAQHGRFLEIGKFDLSNNSQLGMALFLKNVAFHGILLDALFEDGNQDWNIVSELLMKGIKDGVVKPLRSTVFNKEEVEAAFRFMAQGKHIGKVMIKVQEEEKEYPLRRSEPVRISAISRTACPPTKSYILVGGLGGFGLELAQWLVERGAQKLVLTSRSGIRTGYQAKRVEEWKALGVQVLISTRDAATLEGAQQLIEEALRLGPIGGIFNLAVVLRDSMIENQTPELYLEVNKPKYSGTLHLDQVSRKKCPDLDYFVVFSSVSCGRGNAGQSNYGFANSTMERICEQRQHDGLPGLAIQWGAIGDVGVLVKTIGNKDVVVGGTVPQPISSCLEVLDVFLHQPHPVMSSFVLAEKVSVKSDGGSQRDLVEAVGNILGIRDMSTLNPDTSLADLGLDSLMGVEVRQTLERDYDIIMNMREIRLLTINKLRELSSMSGRTEEMKPSQMMKAGFPELPKLNLNNLLVNPEGPTITRLNDVQSTERPLFLIHPIEGSITFFHTLASRLHIPCYGFQCTKAAPLDSIQTLASYYIDCMKQIQPEGPYRIAGYSFGACVAFEMCSQLQAQQNASHTLNNLFLFDGSHSFVAAYTQSYRATLDEGDLAAVETEALSVFVQQFTGMEYNKLLEILLPLEDLAARVNATVDLITQVHTDINREELSFAATSYFYKLKAADQYVPASKYHGNVTLMRVKARSEYEEGLGTDYRLSEVCDGKISVHMVDGDHNTLLEDGVESIVGIIHSSLAEPRVSVREG

SEQ ID NO: 12 - protein, 2511 aa, Calypte anna
MEDVVIAGIAGKLPESENLQEFWENLLNGVDMVTEDDRRWKPGIYGLPRRNGKLKDISKFDASFFGVHPKQAHTMDPQLRLLLEVSYEAILDAGIDPATLRGTDTGVWVGASGSEAAEALSQDPEELLGYSMTGCQRGMFANRISYFYDLTGPSLTIDTACSSSLIALENAYKAIRHGQCSAALVGGVNLLLKPNTSVQFMKLGMLSPEGACKAFDASGNGYCRSEAVVIVLLTKRSMAKRIYATIVNAGTNTDGFKEQGVTFPSGEMQQQLISSLYRESGISPEEVEYVEAHGTGTKAGDPQELNSIVNVFCKCEREPLKIGSTKSNMGHPEPAAGLAALAKVTGGLRRKIGQGRKHNSVGLVCFDIPGLQDGSLEVICKPTPVKGGLVSINSFGFGGANAHVILRPNENRRQPPETCNIPRLVQVCGRTQEAVEVLIQESRKHGGCSPFVSLLSDISAMPVSSMPYRGYTLVGTESDIQEIQQVQASGRPLWYICSGMGTQWKGMGLSLMKLDLFRQSILRSDQALKNTGLKVSDLLLQADDNTFDETVHAFVGLAAIQIAQIDMLKAAGLQPDGILGHSVGELACGYADNCLSHEEAILAAYWRGRCVKEAKLPPGGMAAVGLTWEECKQQCPPNVVPACHNSEDTVTISGPLATVSEFVAKLKKAGVFAKEVRSAGVAFHSHYMASIAPVLLSALKKVIPHPKPRSARWISTSIPESQWQSDLAKYSSAEYHVNNLVSPVLFHEGLKHIPENAVVVEIAPHALLQAILKRTLKPTCTILPLMKKDHKNNLEFFLTQAGKIHLTGINVLGNNLFPPVEYPVPVGTPLISPYIKWDHSQGWDVPKAEDFPSGSKGSASASIYNIDVSPDSPDHYLVGHCIDGRVLYPATGYLVLAWRTLARSLGMVMEQTAVKFEDVTIHQATILPKNGSVQLEVRLMPASHSFEVSGNGNLAVSGKISLLENTALKPADFHTRAGMGLKPGLLKEDIYQELHLRGYNYGPTFQGVLECNSEASAAKVLWNGNWVTFLDTLLHVIILSDTGRSLRLPTRIRSVCVDPVLHQEMVCQYQDNVEVCDAVVDLCLDRLQAGGVQLDGLHASVAPRRQQERMTPTLEKFCFVPYTESDCLSSNAHLHDCLDHCKVLIQKMQAKLAVHGVKLVIPGLDTGSTAAKSSPIQKGLQHILTEICRLELNGNLRSELEQIVTREKMHFHDDPLLSGLLDSSELKSCLDVAVENMTSHRMKIIEALAGSGRLFSRVKSILNTQPLLQVDYIATDRVLETLSASETELQDAGVSSSQWDPSSLPSGNLTNADLVVYNCATNVLGNTTEILSNLAAAVKEGGFVLLHTLLKGETLGEIVSFLSSPDLQQKHKFLHETQWEDLFSKASLNLVAMKKSFFGSVIFLCRRQVPAKTPIFLPVDETHYKWVESLKEILADSSEQPVWLTATSCGNSGILGMVNCLRLESEGHRIRCVFISNLNPSSAVPPTSHSSLEMQKIVQGDLVMNVYRDGKWGSFRHLPLQQAQPQELTEYAYVNVLTRGDLSSLRWIVSPLQHFQANNPDIQLCKVYYASLNFRDIMLATGKLSPDAIPGNWVLQQCMLGMEFSGRDMAGRRVMGLLPAKGLATVVDCEKKFLWEVPKNWTLEEAASVPVVYATAYYALVVRGRMKKGESVLVHSGSGGVGQAAIAIALSMGCRVFTTVGSAEKREYLQARFPQLDANSFASSRDTAFEQHVLRVTNGKGVNLVLNSLAEEKLQASLRCLARHGRFLEIGKFDLSNNSQLGMALFLKNVAFHGILLDAIFEGGNQEWDIVSELLTKGIKDGVVKPLKSTVFKKEEVEAAFRFMAQGKHIGKVMIQIQEEEKEYSVRRSEPVKISAISRTSCPPSKSYIITGGLGGFGLELAQWLVERGAQKLILTSRSGIRTGYQARRVREWKALGIQVLVSTSDIGTLEGAQRLIEEALQLGPVGGIFNLAVVLRDAMIENQTPELFVEVNKPKYSGTLHLDWVTRKKCPDLDYFVVFSSVSCGRGNAGQSNYGFANSTMERICEQRHHDGLPGLAIQWGAIGDVGILLKTMGNKEVVVGGTIPQQISSCLEVLDTFLNQPHPVTSSFVLAEKVSVKAEGGSQRDLVEAVAHILGVRDVSSLNADSSLADLGLDSLMGVEVRQTLERDYDIVMTMREIRLLTINKLRELSSKSGTTEELKPSQVMKTGAGEPPKLDLNNLLVNPEGPTITRINDVQSTERPLFLVHPIEGSTAVFKTLASKLHMPCYGFQCTKVAPLDSIQSLATYYINCMKQIQPEGPYRIAGYSFGACVAFEMCSQLQAQHKGSHALNSLFLFDGSHSFVAAYTQRYRAKLSQGNEAALETEALCAFVQQFTGIEYNKLLEILLPLKDLEARVNAAADLITQVHTHINREALCFAATSFYHKLKAADKYIPESKYHGNVTLVRAKSHNEYEEGLGGDYRLSEVCDGKVSVHVVEGDHRTMLEGNGAESIIGIIHSSLAEPRVSVREG

SEQ ID NO: 13 - protein, 2513 aa, Anas platyrhynchos
MEDVVIAGIAGKLPESENLQEFWENLLNGVDMVTEDDRRWKPGMYGLPKRNGKLKDISKFDASFFGVHPKQAHTMDPQLRLLLEVSYEAILDGGINPATLRGTDTGVWVGASGSEAAEAFSQDPEQLLGYSMTGCQRAMFANRISYFFDFKGPSLTIDTACSSSLMALENAYKAIRNGQCSAAVVGGVNLLLKPHTSVQFMKLGMLSPDGACKAFDASGNGYCRSEAVVVVLLTKKSMAKRIYATIVNAGSNTDGFKEQGVTFPSGDMQRQLVSSLHRECGIKPGDIEYVETHGTGTKVGDPQEVNGIADVFCQCEREPLLIGSTKSNMGHPEPASGLAALAKVVLSLEHGLWAPNLHFSDPNPDIPALLNGSLKVVCEPTPTKGGLVSINSFGFGGANVHVILKPNEKKHQPPETCNLPRLVQVCGRTQEAVETLIQESKKQRGCGPFLRLLTDISAIPVSLMPYRGYTLVGTESDIGEVQQVQVSGRPLWYICSGMGTQWKGMGLSLMKLDVFRQSIMRSDEALKNTGLKVSDLLLQADDNTFDETVNAFVGVAAVQIAQIDMLKAAGLQPDGILGHSVGEVACGYADNSLSHEEAILAAYWRGRCVKEAKLPPGGMAAVGLTWEECKQRCPPNVVPACHNSEDTVTISGPLDSVNEFVAKLKKDGVFAKEVRSAGVAFHSYYMASIAPALLSALRKVIPHPKPRSARWISTSIPESQWQSDLARNSSAEYYVNNLVSPVLFHEGLKHIPENAVVVEIAPHALLQAILRRSLKPSCTILPLMKKDQKNNLEFFLTQAGKIHLTGINVLGNNMFPSVEYPVPVGTPLISPYIKWDHSQDWDVPKAEDFPSGSKGSASASVYNIDVSPDSPDHYLVGHCIDGRILYPATGYLVLAWRSLAGSLGMAMEQTAVMFEDVTIHQATILPKKGSVQLEVRIMPASHCFEVSGNGNLAVSGKINLLENDALKNFRNQLAAFQTHLDTSSKSGLLKEDVYQELHLRGYNYGPTFQGVLECNSEGSAGKVLWNGNWVTFLDTLLHMIVLAETGRSLRLPTRIRSVYIDPVLHPEHVCQYQDNVEALDVVVDHCLNSLKAGGVQINGLHASVAPRRQQERIPPTLEKYCFIPYIESNCLSSSAQLHAYLEHCKGLIKNLQAKVAVHGVKLIIHGLETAGAAAGSSPMQKGLQHILAEICHLELNGNLHSELEQIVTQEKMHFQDDPLLNGLLDSSELKACLDVALENMTSHRMKIVEALAGNGHLFSRVTSILNTQPLLHLDYIATDCTLEALSANETELQDAGISFSQWDPSNPPSGNLSNADLVVYNCSTNVLGNTTKIVSNLAAAVKEGGFVLLHTLLQGETLGEIVSFLTSPDLQQKHSFLSQAQWEGLFSKASLNMIAMKRSFFGSVIFLCRRQSPAKTPIFLPIDETHYKWVESLKEILADQSEQPVWLTATSCGNSGILGMVNCLRLEAEGHRVRCVFVSNLNPSSAVPSISLSSLEMQEIVQRDLVMNVYRDGKWGSFRHLPLQQGQPQELTEYAYVNALTRGDLSSLHWIVSPLQHFYTTNPDVQLCKVYYASLNFRDIMLATGKLSPDAIPGNWASQQCMLGMEFSGRDMAGRRVMGLVSAKGLATVVDCNKRFLWEVPKNWTLEEAASVPVVYATAYYALVVRGGMKKGESILIHSGSGGVGQAAIAIALSMGCRVFTTVGSAEKRQYLQARFPQLDANSFASSRNTTFEQHVLRVTNGKGVNLVLNSLAEEKLQASLRCLAQHGRFLEIGKFDLSNNSQLGMALFLKNVSFHGILLDSIFGESNEEWEVVSKLLTKGIENGVVKPLRSTVFNKDEVEAAFRFMAQGKHIGKVMIKVQEEEKQYPLRRSEPVKLSAISRTSCPPTKSYIITGGLGGFGLELAQWLIERGAQKLVLTSRSGIRTGYQAKCVREWKALGIQVLVSTSDIGTLEGTQLLIEEALRLGPVGGIFNLAVVLRDAMIENQTPELFWEVNKAKYSGTLHLDWVTRKKCPDLDYFVVFSSVSCGRGNAGQSNYGFANSAMERICEQRHHDGLPGLAIQWGAIGDVGILKTVGNTDVVIGGTIPQQISSCLEVLDTFLNQSHPVVSSFVLAEKVSVKSEGSNQRDLVEAVAHIIGVRDVSSLNADSTLADLGLDSLMGVEVRQTLERDYDIIMTMREIRLLTINKLRELSSKSGTAEELKPSQLLKTGPGEPPKLDLNNLLVNPEGPTITRLNDVQSTERPLFLVHPIEGSIAVFYTLASRLHMPCYGLQCTKAAPLDSIQSLASYYIDCMKQIQPEGPYRIAGYSFGACVAFEMCSQLQGQQNASHALNSLFLFDGSHSFVAAYTQSYRAKLAQGNEAALETEALCAFVQQFTGIEYNKLLEILLPLKDLEARVNAAADLITQIHKNINREALSFAAASFYHKLKAADKYIPESKYHGNVTLMRAKTHNEYEEGLGGDYRLSEVCDGKVSVHVIEGDHRTLLEGDGVESIIGIIHSSLAEPRVSVREG

SEQ ID NO: 14 - protein, 2512 aa, Gallus gallus
MEDVVIAGIAGKLPESENLQEFWENLLNGVDMVTEDDRRWKPGIYGLPKRNGKLKDIKKFDASFFGVHPKQAHTMDPQLRLLLEVSYEAILDGGINPTALRGTDTGVWVGASGSEALEALSQDPEELLGYSMTGCQRAMLANRISYFYDFTGPSLTIDTACSSSLMALENAYKAIRHGQCSAALVGGVNILLKPNTSVQFMKLGMLSPDGACKAFDVSGNGYCRSEAVVVVLLTKKSMAKRVYATIVNAGSNTDGFKEQGVTFPSGEMQQQLVGSLYRECGIKPGDVEYVEAHGTGTKVGDPQEVNGIVNVFCQCEREPLLIGSTKSNMGHPEPASGLAALAKVILSLEHGLWAPNLHFNDPNPDIPALHDGSLKVVCKPTPVKGGLVSINSFGFGGSNAHVILRPNEKKCQPQETCNLPRLVQVCGRTQEAVEILIEESRKHGGCSPFLSLLSDISAVPVSSMPYRGYTLVGTESDITEIQQVQASGRPLWYICSGMGTQWKGMGLSLMKLDLFRQSILRSDEALKSTGLKVSDLLLNADENTFDDTVHAFVGLAAIQIAQIDVLKAAGLQPDGILGHSVGELACGYADNSLSHEEAVLAAYWRGRCVKEAKLPPGGMAAVGLTWEECKQRCPPNVVPACHNSEDTVTVSGPLDSVSEFVTKLKKDGVFAKEVRRAGVAFHSYYMASIAPALLSALKKVIPHPKPRSARWISTSIPESQWQSDLARNSSAEYHVNNLVNPVLFHEGLKHIPENAVVVEIAPHALLQAILRRTLKPTCTILPLMKKDHKNNLEFFLTQTGKIHLTGINVLGNNLFPPVEYPVPVGTPLISPYIKWDHSQDWDVPKAEDFPSGSKGSASASVYNIDVSPDSPDHYLVGHCIDGRVLYPATGYLVLAWRTLARSLGMVMEQTAVMFEEVTIHQATILPKKGSTQLEVRIMPASHSFEVSGNGNLAVSGKISLLENDALKNFHNQLADFQSQANVTAKSGLLMEDVYQELHLRGYNYGPTFQGVLECNSEGSAGKILWNGNWVTFLDTLLHLIVLAETGRSLRLPTRIRSVYIDPVLHQEQVYQYQDNVEAFDVVVDRCLDSLKAGGVQINGLHASVAPRRQQERISPTLEKFSFVPYIESDCLSSSTQLHAYLEHCKGLIQKLQAKMALHGVKLVIHGLETKGAAAGSPPAQKGLQHILTEICRLELNGNPHSELEQIVTQEKMHLQDDPLLNGLLDSSELKTCLDVAKENTTSHRMKIVEALAGSGRLFSRVQSILNTQPLLQLDYIATDCTPETLSDNETELHDAGISFSQWDPSSLPSGNLTNADLAVCNCSTSVLGNTAEIISNLAAAVKEGGFVLLHTLLKEETLGEIVSFLTSPDLQQKHSFLSQAQWEELFSKASLNLVAMKRSFFGSVIFLCRRQSPAKAPILLPVDDTHYKWVDSLKEILADSSEQPLWLTATNCGNSGILGMVNCLRLEAEGHRIRCVFVSNLSPSSTVPATSLSSLEMQKIIERDLVMNVYRDGKWGSFRHLPLQQAQPQELTECAYVNVLTRGDLSSLRWIVSPLRHFQTTNPNVQLCKVYYASLNFWDIMLATGKLSPDAIPGNWTLQQCMLGMEFSGRDLAGRRVMGLLPAKGLATVVDCDKRFLWEVPENWTLEEAASVPVVYATAYYALVVRGGMKKGESVLIHSGSGGVGQAAIAIALSMGCRVFATVGSAEKREYLQARFPQLDANSFASSRNTTFQQHILRVTNGKGVSLVLNSLAEEKLQASLRCLAQHGRFLEIGKFDLSNNSQLGMALFLKNVAFHGILLDSIFEEGNQEWEVVSELLTKGIKDGVVKPLRTTVFGKEEVEAAFRFMAQGKHIGKVMIKIQEEEKQYPLRSEPVKLSAISRTSCPPTKSYIITGGLGGFGLELAQWLIERGAQKLVLTSRSGIRTGYQAKCVREWKALGIQVLVSTSDVGTLEGTQLLIEEALKLGPVGGIFNLAVVLKDAMIENQTPELFWEVNKPKYSGTLHLDWVTRKKCPDLDYFVVFSSVSCGRGNAGQSNYGFANSAMERICEQRHHDGLPGLAVQWGAIGDVGILKAMGNREVVIGGTVLQQISSCLEVLDMFLNQPHPVMSSFVLAEKVSVKSEGGSQRDLVEAVAHILGVRDVSSLNAESSLADLGLDSLMGVEVRQTLERDYDIVMTMREIRLLTINKLRELSSKTGTAEELKPSQVLKTGPGEPPKLDLNNLLVNPEGPTITRLNEVQSTERPLFLVHPIEGSIAVFYTLASKLHMPCYGLQCTKAAPLDSIQSLASYYIDCMKQIQPEGPYRIAGYSFGACVAFEMCSQLQAQQNASHALNSLFLFDGSHSFVAAYTQSYRAKLTQGNEAALETEALCAFVQQFTGIEYNKLLEILLPLEDLEARVNAAADLITQIHKNINREALSFAAASFYHKLKAADKYIPESKYHGNVTLMRAKTHNEYEEGLGGDYRLSEVCDGKVSVHIIEGDHRTLLEGDGVESIIGIIHGSLAEPRVSVREG

SEQ ID NO: 15 - protein, 2509 aa, Nestor notabilis
MEDVVIAGIAGKLPESENLQEFWENLLNGVDMVTEDDRRWKPGIYGLPKRNGKLKDISKFDASFFGVHPKQAHTMDPQLRLLLEVSYEAILDGGINPATLRGTDTGVWIGASGSEAAEALSQDPEKLLGYSMTGCQRAMLANRISYFYDFTGPSIAIDTACSSSLIALENAFKAIRHGQCSAALVGGVNLLLKPNTSVQFMKLGMLSSDGACKAFDASGSGYCRSEAVVVVLLTKRSMAKRIYATIVNAGSNTDGFKEQGVTFPSGEMQQRLVSSLYRECGIKLEEVEYVEAHGTGTKVGDPQEINGIVKMFHQCERAPLLIGSTKSNMGHPEPASGLAALAKVMGGLRRRIEGGREHNNIPALQDGTLEVVCKPTPVKGGLVGINSFGFGGANAHVILRPHKNKCQPLETCNTPRLVQICGRTQEAVETLIQESREHGGCSPFLSLLTDISAVPVSSMPYRGYTLVGTESDIKEVQHVQASGRPLWYICSGMGSQWKGMGLSLMKLDMFRQSILRSDEALKNTGLKVSDLLLRADENTFDETINAFVGLAAIQIAQIDLLKAAGLQPDGILGHSVGELACGYADNCLSQEEAILGAYWRGRCVKEAKLPPGAMAAVGLTWEECKQRCPPNVVPACHNSEDTVTVSGPLESVTEFVAKLKKDGVFAKEVRSAGVAYHSHYMASIAPVLLNALKKVIPHPKPRSARWISTSIPESQWQSDLARSCSAEYLVNNLVNPVLFHDGLKHVPENAVVVEIAPHALLQAILRRTLKPTCTILPLMKKDQKNNLEFFLTQTGKIHLTGINVLGNNLFPLVEYPVPVGTPLISPYIKWDHSQDWDVPKAEDFPAGSKGSASASVYSIDLSPDSPDHYLVGHCIDGRVLYPATGYLVLAWRTLARSLGMAMEQMAVTFEEVTIHQATILPKNGSVQLEVRLMPASHYFEVSGNGNLTVSGKIFLLENTALKNFHNQLVDFQTQADTSSKSGLLKEDIYQELHLRGYNYGPTFQGVLECNSEASTGKVLWNGNWVTFLDTLLHMMVLAKSGRSLRLPTRIRSVCIDPVLHQEKVCQYQDNVEALDVVVDPCLGSLKAGGVQIDGLHASVAPRRQQERIPPTLEKFCFVPYTESNCLSSSVHLRAYLEHCKDLIRNVQAKVAVHGVKLVIPGLKTAVAAAGSSPIQKGLQHILAEICRLELNGNLSSELEQIVTQEKMHFQDDPLLNGLLDSSELKTCLGVALENMTSHRMKIVEALAGSGCLFSRIKSILNAQPLLQVDYIATDRILKTLSDSETELQDAGVSISQWDPSCLPSGDLANADLVVYNCLTVLGNTTEIVSNLAAAVKEGGFFLLHTLLKGETFGEIVSFLTSPDLQQKHSFLSEAQWEGLFSKASLNVVAMKKSFFGSVIFLCRRQAPAKTPIFLPVDETHFAWVESLKEVLADPSEQPVWLTATSCGNSGILGMVNCLRLEAEGHRIRCVFVSNLNPSSAVPPTSLSSLEMQKIVQRDLVMNVYRDGKWGSFRHLPLQQAQSQELTEYAYVNVLTRGDLSSLHWIVSPLRHFHTTNPNVQLCKVYYASLNFRDIMLATGKLPPDAIPGNWVLQQCMLGMEFSGRDLAGRRVMGLLPAKGLATVVDCDKRFLWEVPKNWTLEEAASVPVVYATAYYALVVRGGMKKGESILIHSGSGGVGQAAIAIALSMGCRVFTTVGSTEKREYLQARFPQLDANSFASSRNTTFEQHILRLTNGKGVNLVLNSLAEEKLQASLRCLAQHGRFLEIGKFDLSNNSQLGMALFLKNVAFHGILLDAIFEENQAWEVVSELLKKGIKDGVVKPLRSTIFNKDEVEAAFRFMAQGKHIGKVMIKVQEEELESPLRRSDPVKISAISRTSCPPTKSYIITGGLGGFGLELAQWLVERGAQKLILTSRSGIRTGYQADRVRQWKALGVQVLVSTSDIATLEGTQLLIEEALQLGPVGGIFNLAVVLRDGMIENQTPELFCEVNKPKYSGTLHLDWVTRKKCPDLDYFVVFSSVSCGRGNAGQSNYGFANSTMERICEQRHHDGLPGLAIQWGAIGDVGILLKTMGDREIVIGGTLPQQISSCLEVLDIFLNQPHPVMSSFVLAEKVSVKTEGGSQQDLVAAVAHILGVRDVSSLNAESTLADLGLDSLMGVEVRQTLERDYDIVMTMREIRLLTVNKLRELSSKSRTAEGIVPARAQLMKTGPGKSPKLDLNNLLVNPEGPTITRLNDVQSTERPLFLVHPIEGSVAVFYTLSSRLHMPCYGLQCTKAAPLDSIQSLAAYYIDCMKQIQPEGPYRIAGYSFGACVAFEMCSQLQDQQNASHALNSLFLFDGSHSFVAAYTQSYRAKLAQGNEAALETEALCAFVQQFTGIEYNKLLEVLLPLKDLEARVNAAADLITQIHANINREALSFAAASFYHKLKAADKYIPESKYRGNVTLMRAKSHSEYEEGLGGDYRLSEVCDGKVSVHIIEGDHRTLLEGDGVESIIGIIHSSLAEPRVSVREG

SEQ ID NO: 16 - protein, 2516 aa, Podiceps cristatus
MEDVVIAGIAGKLPESENLQEFWENLLNGVDMVTEDDRRWKPGIYGLPKRNGKLKDISKFDASFFGVHPKQANTMDPQLRLLLEVSYEAILDAGINPTTLRGTNTGVWVGASGSEAAEAFSRDPEELLGYSMTGCQRAMLANRISYFYDLKGPSLVIDTACSSSLVALESAYKAIRNGRCSAALVGGANLLLKPNTSVQFMKLGLLSPDGTCKAFDASGNGYCRSEAVVVILLTKRSMAKRIYATIVNAGINTDGFKEQGVTFPSGEMQQQLISSLYKECNIKPEELEYIETHGTGTKVGDPQEINGIADLFCQLERPPLLIGSTKSNMGHPEPASGLAALAKVTGGLRRKIGGEGEHNGAWVFVNIPALQDGSLEVICKPTPVKGGLVGINSFGFGGANAHVILRPNEKKSQPLETCNMPRLVQFCGRTKEAVETLIQASRNHGACSPFVSLLSDISTLPVSSMPYRGYALVGTDDSDIKEVQQVQGSGRPLWYICSGMGTQWKGMGVDLMKLDLFRQSILRSDEALKSTGLKVSDLLLQADENTFDDTVHAFVGLAAIQIAQIDMLKAAGLQPDGILGHSVGELACGYADNSLSREEAILAAYWRGRCVKEAKLPPGGMAAVGLTWEECKQCCPPNVVPACHNSEDTVTISGPLDSVHEFVAKLKKDGVFAKEVRSAGVAFHSYYMASIAPVLLSALKKVIPHPKPRSARWISTSIPESQWQSDLARNSSAEYHVNNLVNPVLFHEGLKHVPENAVVVEIAPHALLQAILRRTLKPTCTILPLMKKDHKNNLEFFLTQTGKIHLTGINVLGNNLLPLVEYPVPVGTPLISPYIKWDHSQDWDVPKAEDFPSGSKGSASASVYNIDVSPDSPDHYLVGHCVDGRVLYPATGYLVLAWRTLARSLGMAMEQMAVMFEEVTIHQATILPKKGSIQLEVRLMPASHCFEVSGNGNLAVSGKISLLENTALKDFHNQIVDFQTRVDRSSKSGLLKEDIYQELHLRGYNYGPTFQGVLECNSEASMGKVLWNRNWVTFLDTLLHMIVLTETGRSLRLPTRIRSVCIDPVLHQEYVCQYQDNVEAFDVVVDRCLDSLRAGGVQINGLHASVAPRRQQERTPPTLEKFCFVPYTESNCLSSSVHLNAYLEHCKGLIRNLQAKVAVHGVKLVIPGLETSVAAAKSSPIQKGLQHILAEICHLELNGNLHSELEQIVTQEKMHLQDDPLLNGLLDSSELNTCLDVALENMTSHRIKIVEALAGSGHLFSRVKSILNTRPLLQVDYIATDCILETFSANETELQDAGVSFSQWDPSSLPSGNLTNADLVVYNYSRSVLGNITEILSNLVAAVKEGGFVLLHTLLKGGTLGDIVSFLTSPDLQQKHSFLSEEQWEGLFSKASLNLVAMKKSFFGSVIFLCRRQAPAKTPIFLPVDETHYKWVESLKEILANPSEQPVWLTATSCGNSGILGMVNCLRLEAEGHRIRCVFVTNLNPSSAVPPTSLSSLEMQKIVQRDLVMNVYRDGKWGSFRHLPLQQAQPQELTEYAYVNVLTRGDLSSLHWIVSPLQHFHATNPNVQLCKVYYASLNFRDIMLATGKLSPDAIPGNWALQQCMLGMEFSGRDLAGRRVMGLLPAKGLATVVDCDKKFLWEVPKNWTLEEAASVPVVYATAYYALVVRGGMKKGESILIHSGSGGVGQAAIAIALSMGCRVFATVGSTEKREYLQARFPQLDANSFASSRNTTFEQHILRVTNGKGVNLVLNSLAEEKLQASLRCLARHGRFLEIGKFDLSNNSQLGMALFLKNVSFHGILLDAVFEDGNEEWEVVSELLKKGIKDGVVKPLRSTVFNKEEVEAAFRFMAQGKHIGKVMIKVQEEEKEYLLRKSEPVKVSAISRTSCPPTKVYIITGGLGGFGLELAQWLVERGAQKLILTSRSGIRTGYQAKCVGDWKALGIQVLVSTSDIATLEGTQLLIEEALQLGPVGGIFNLAVVLRDSMIENQTPESFWEVNKPKYSGTLHLDWVTRKKCPDLDYFVVFSSVSCGKGNAGQSNYGFANSTMERICEQRHHDGLPGLAIQWGAIGDVGILLKTIGNKDVVIGGTVPQQISSCLEVLDIFLNQPHPVMSSFVLAEKVSVKPQEGSQRDLVEAVAHILGVRDVSTLNAESSLADLGLDSLMGVEVRQTLERDYDIVMTMREIRNLTINKLRELSSKSGTAEELKPSQLTKTGPGEPPKLDLNNLLVNPEGPTITRLNDVQSTERPLFLVHPIEGSIAVFSTLASRLHLPCYGLQCTKAAPLDSIQSLAAYYIDCMKQIQPEGPYRIAGYSFGACVAFEMCSQLQAQQNASHALNSLFLFDGSHSFVTAYTRSYRAKLTQGNEAALETEALCAFVQQFIGIEYNKLLEVLLPLKDLDARVNAAADLITRIHTNINHEALSFAAASFYHKLKAADKYIPESMYHGNVTLMRAKSYNEYEEGLGGDYRLSEVCDGKVSVHVIEGDHRTLLEGDGVESIIGIIHSSLAEPRVSVREG

SEQ ID NO: 17 - protein, 2518 aa, Balearica regulorum gibbericeps
MEDVVIAGIAGKLPESENLQEFWENLLNGVDMVTEDDRRWKPGIYGLPKRNGKLKDISKFDASFFGVHPKQAHTMDPQLRLLLEVSYEAILDGGINPATLRGTDTGVWIGASGSEAGEALSQDPEELLGYSMTGCQRAMFANRISYIYDLTGPSITIDTACSSSLVALENAYKAIRHGRCSAALVGGVNLLLKPNTSVQFMKLGMLSPDGACKAFDASGNGYCRSEAVVVILLTKRSMAKRIYATIVNAGSNTDGFKEQGVTFPSGEMQQQLVSSLYRECGIKPGEVEYVEAHGTGTKAGDPQEVNGIVSVFCQCEREPLLIGSTKSNMGHPEPASGLAALAKVTGGLKKKIGEGTHAHPNVYVFLNVDIPALQDGSLEVVCKPTPVKGGIVSINSFGFGGANAHVILRPNENKRQPLETCNMPRLVQICGRTQEAVEILIQESRKHGGCSPFVSLLSDISAVPVSSMPYRGYTLVGTESDIKEVQQVQASGRPLWYICSGMGTQWKGMGLSLMKLDLFRQSILRSDEALKNTGLKVSDLLLQADENTFDDTVHAFVGLAAIQIAQIDMLKAAGLQPDGILGHSVGELACGYADNSLSHEEAILAAYWRGRCVKEAKLPPGGMAAVGLTWEECKQCCPPNVVPACHNSEDTVTVSGPLDSVNEFVAKLKKDGVFAKEVRSAGVAFHSYYMASIAPVLLSALKKVIPHPKPRSARWISTSIPESQWQSDLARNSSAEYHVNNLVNPVLFHEGLKHVPENAVVVEIAPHALLQAILRRTLKPTCTILPLMKKEHKNNLEFFLTQTGKIHLTGINVLGNNLFPLVEYPVPVGTPLISPYIKWDHSQDWDVPKAEDFPSGSKGSASASVYNIDVSPDSPDHYLLGHCIDGRVLYPAAGYLVLAWRTLARSLGMAMEQMAVTFEEVTIHQATILPKKGSVQLEVRLMPASHCFEVSGNGNLAVSGKISLLENTALKNFHNQAVDFQTQVDTSSKSGLLKEDVYQELHLRGYNYGPTFQGVLECNNEASTGKVVWNGNWVTFLDSLLHVIILAETGRSLRLPTRIRSVIIDPVLHQEQVYQYQDNVEAFNVTVDHCLNSLKAGGVQINGLHASAAPRRQQERNPPTLEKFCFVPYTESNCLSSSVHLHAYLGHCKDLIQNLQAKVAVHGVKLVIPGLETAVAAAESSPIQKGLQHILAAICHLELNGNLHSELEQIVTQEKMHFQDDPLLNGLLDSSELKTCLDVALENMTSHRMKIIEALAGSGHLFSRVKSVLNTQPLLQVDYIATDCSLEALSANETELQDAGVSLSQWDPSSLPSGNLTNADLVVYNYSTSVLGNTTEILSNLAAAVKEGGFVLLHTLLKGETLGEIVSFLTSPDLQQKHSFLSEAQWEGLFSKASLNLVAMKKSFFGSVIFLCRRQAPAKTPVFLPIDETHFKWVESLKEVLADPSEQPVWLTATSCGNSGILGMVNCLRLEAEGHRIRCVFVSNLNRSSAVPPMTLSSLEMQKIVQRDLVVNVYRDGKWGSFRHLPLQQAQPQELTEYAYVNVLTRGDLSSLRWIVSPLRHFHATNPNVQLCKVYYASLNFRDIMLATGKLSPDAIPGNWALQQCMLGMEFSGRDLAGRRVMGLLPAKGLATVVDCDKMFLWEVPKNWTLEEAASVPVVYATAYYALVVRGGMRKGESILIHSGSGGVGQAAIAIALSMGCRVFTTVGSTEKREYLQARFPQLDANSFASSRNTTFEQHILRVTNGKGVNLVLNSLAEEKLQASLRCLAQHGRFLEIGKFDLSNNSRLGMALFLKNVAFHGILLDAIFEDGNKEWEVVSELLKKGIKDGVVKPLRSTVFNKEEVEAAFRFMAQGKHIGKVMIKVQEEEKENPLRRSEPVKISAISRTLCPPTKSYIITGGLGGFGLELAQWLVERGAQKLILTSRSGIRTGYQAKRVREWKALGIQVLVSTSDIGTLEGAQLLIEEALQLGPVGGIFNLAVVLRDGMIENQTPELFWEVNKPKYSGTLHLDWVTRKKCSDLDYFVVFSSVSCGRGNAGQSNYGFANSTMERICEQRHHDGLPGLAIQWGAIGDVGILLKTMGNKEIVVGGTVPQQISSCLEVLDIFLNQPHPVMSSFVLAEKISLKTEGGSQRDLVEAVAHILGVRDVNSLNAESSLADLGLDSLMGVEVRQTLERDYDIVMTMREIRLLTINKLRELSSKSGTAEELKPSQLMKTGPGEPPKLDLNNLLVNPEGPTLTRLNDVQSTERPLFLVHPIEGSIAVFYTLASRLHVPCYGLQCTKAAPLDSIQSLATYYIDCMKQIQPEGPYRIAGYSFGACVAFEMCSQLQAQQNASHALNSLFLFDGSHSFVAAYTQSYRAKLTQGNEAALETEALCAFVQQFTGIEYNKLLEVLLPLEDLEARVNAAADLITQIHTNINREALSFAAASFYHKLKAADKYIPESKYHGNVTLMRAKSHNEYEEGLGGDYRLSEVCDGKVSVHIIEGDHRTLLEGDGVESIIGIIHSSLAEPRVSVREG

SEQ ID NO: 18 - protein, 2515 aa, Phaethon lepturus
MEDVVIAGIAGKLPESENLQEFWENLFNGVDMVTEDDRRWKPGIYGLPKRNGKLKDISKFDASFFGVHPKQAHTMDPQLRLLLEVSYEAILDGGINPATLRGTDTGVWVGASGSEAGEALSQDPEQLLGYSMTGCQRAMFANRISYFYDLTGPSITIDTACSSSLVALENAYKAIRHGQCCAALVGGVNLLLKPSTSVQFMKLGMLSPDGACKAFDVSGNGYCRSEAVVVVLLTKRSMAKRIYATIVNAGSNTDGFKEQGVTFPSGEMQQRLVSSLYRECGIRPGEVEYIETHGTGTKVGDPQEVNGIANVFCQCEREPLLIGSTKSNMGHPEPASGLAALAKVTGGLRRKILGGSTTVMRCSLRDIPALQDGSLEVVCKPTPVKGGLVSINSFGFGGANAHVILRPNEKKRQPLETCNTPRLVQICGRTQEAVEILIQESRRHGGCSPFVSLLSDISTVPVSFMPYRGYTLVGTESDIKEVQQVQASDRPLWYICSGMGTQWKGMGLSLMKLDLFRQSILRSDEALKNTGLKVSDLLLQADENTFDDTVHAFVGLAAIQIAQIDMLKAAGLQPDGILGHSVGELACGYADNSLSHEEAILAAYWRGRCVKEAKLPPGGMAAVGLTWEECKQCCPPNVVPACHNSEDTVTVSGPLDSVNEFVAKLKKDGVFAKEVRSAGVAFHSYYMASIAPVLLSALKKVIPHPKPRSARWISTSIPESQWQSDLARNSSAEYHVNNLVNPVLFHEGLKHIPENAVVVEIAPHALLQAILRRTLKPTCTILPLMKKEHKNNLEFFLTQTGKIHLTGINVLGNNLFPLVEYPVPVGTPLISPYIKWDHSQDWDVPKAEDFPAGSKGSASASVYNIDVSPDSPDHYLVGHCIDGRVLYPATGYLVLAWRTLARSLGTAMEQTAVMFEEVTIHQATILPKKGSVQLEVRLMPASHCFEVSGNGNLAVSGKISLLEHTAPKNFHNQPVDFQTQADMSSKSGLLKDDIYQELHLRGYNYGSTFQGVLECNSEASTGKVLWNGNWVTFLDTLLHVIILAETGRSLRLPTRIRSVCIDPVLHQEQVCQYRDNVEAFDVVVDRCLDSLKAGGVQINGLHASVAPRRQQERIPPTLEKFCFVPYNEHNCLSSSVHLHAYLERCKDLIQNLKAKVAVHGVKLVIPGLETTVAAAESSPIQNGLQHILAEICRLELNGNLHSELEQIVTQEKMHFQDDPLLNGLLDSSELKTCLDVALENMTSHRMKIVEALAGSGHLFSRVKSILNTQPLLQVDYIATDHILETLSANETELQDAGVLFSQWDPSSLPSGNLTNADLVVYNCSTSVSGNTIEILSNLAAAVKEGGFVLLHTLLKGETLGEIVSFLTSPDLQQKHSFLNEAQWEGLFSKASLNLVAMKKSFFGSVIFLCRRQAPAKTPVFLPIDETHYKWVESLKEVLADPSEQPVWLTATSCGNSGILGMVNCLRLEAEGHRIRCVFISNLNPSSAVPPTSLSSLEMQKIVQRDLVMNVYRDGKWGSFRHLPLQQEQPQELTEYAYVNVLTRGDLSSLRWIVSPLRHFHATNPNVQLCKVYYASLNFRDIMLATGKLSPDAIPGNWALQQCMLGMEFSGRDLAGRRVMGLLPAKGLATVVDCDKMFLWEVPKNWTLEEAASVPVVYATAYYALVVRGGMKKGESVLIHSGSGGVGQAAIAIALSMGCRVFATVGSTEKREYLQARFPQLDADSFASSRNTTFEQHILRVTNGKGVNLVLNSLAEEKLQASLRCLARHGRFLEIGKFDLSNNSQLGMSLFLKNVAFHGILLDAIFEQGNQEWEVVSELLKKGIKDGVVKPLRSTVFNKEEVEAAFRFMAQGKHIGKVMIKVQEEEKEYSLRRFETVKISAISRTSCPPTKSYIITGGLGGFGLELAQWLVERGAQKLILTSRSGIRTGYQAKRVREWKALGIQVLVSTSDIGTLEGTQLLIEEALQLGPVGGIFNLAVVLRDGMIENQTPEFFWEVNKPKYSGTLHLDWVTRKKCPDLDYFVVFSSVSCGRGNAGQSNYGFANSTMERICEQRHHDGLPGLAIQWGAIGDVGILLKTMGNREVVVGGTIPQQISSCLEVLDIFLNQPHPVMSSFVLAEKVSVKTEGGSQRDLVEAVAHILGVRDVSSLNAESSLADLGLDSLMGVEVRQTLERDYDIVMTMREIRLLTINKLRELSSKSGTAEDLKLSQLMKTGPGEPPKLDLNNLLVNPEGPTITRLNDVQSTERPLFLVHPIEGSIAVFYTLASRLHIPCYGLQCTKAAPLDSIQSLAAYYIDCMKQIQPEGPYRIAGYSFGACVAFEMCSQLQAQQNASHAFNSLFLFDGSHSFVAAYTQSYRAKLTQGNEAALETEALCAFVQQFTGIEYNKLVEVLLPLKDLEARVNAAADLITQIHTNINREALSFAAASFYHKLKAADKYIPESKYHGNVTLMRAKSHNEYEEGLGGDYRLSEVCDGKVSVHIIEGDHRTLLEGDGVESIIGIIHSSLAEPRVSVREG

SEQ ID NO: 19 - protein, 2140 aa, Phoenicopterus ruber
EVVCKPTPVKGGLVGINSFGFGGANAHVILRPNDNKSQPLKTCNMPRLVQICGRTQEAVEVLIQESRKHGGCSPFLSLLSDISTVPVSSMPYRGYTLVGTESDIKEVQQVQASGRPLWYICSGMGTQWKGMGLSLMKLDLFRQSILRSDEALKNTGLKVSDLLLQADENTFDDTVHAFVGLAAIQIAQIDLLKAAGLQPDGILGHSVGELACGYADNSLSHEEAILAAYWRGRCVKEAKLPPGGMAAVGLTWEECKQCCPPNVVPACHNSEDTVTVSGPLDSVREFVAKLKKDGVFAKEVRSAGVAFHSYYMASIAPVLLSALKKVIPHPKPRSARWISTSIPESQWQSDLARNSSAEYHVNNLVNPVLFQEGLKHIPENAVVVEIAPHALLQAILRRALKPTCTILPLMKKEHKNNLEFFLTQTGKIHLTGINVLGNNLFPLVEYPVPVGTPLISPYIKWDHSQDWDVPKAEDFPAGSQGSASASVYNIDVSPDSPDHYLVGHCIDGRVLYPATGYLVLAWRTLARSRGMAMEQMAVMFEEVTIHQATILPKKGSVQLEVRLMPASHCFEVSGNGNLAVSGKISLLEDTALKNFHNQPVDFQTQVDMSSKSGLLKEDIYQELHLRGYNYGPTFQGVLECNSEASTGKVLWNGNWVTFLDTLLHMIILTETGRSLRLPTRIRSVCIDPVLHQEHVCQYQDNIEAFDVVVDRCLDSLKAGGVQINGLHASVAPRRQQERIPPTLEKFCFVPYTESNCLSSSVHLNAYLEHCKDLIQNLQAKVAVHGVKLVIPGLETAVAAAESSPIQKGLQHILAEICRLELNGNLHSELEQIVTQEKMHLQDDPLLNGLLDSSELKTCLDVALENTTSHRIKIVEALAGSGHLFSRIKSILNTQPLLQVDYIATDRILETLSANETELQDAGVSFSQWDPSSLPSENLTNADLVVYNYSTSVLGNTTEILSNLAAAVKEGGFVLLHTLLKGETLGDIVSFLTSPDLQQKHSFLSEEQWEGLFRKASLNLVAMKKSFFGSVIFLCRRQAPAKTPIFLPIDETHYKWVESLKEILADPSEQPVWLTATSCGNSGILGMVNCLRLEAEGHRIRCVFVSNLNPSSAVPPTSLSSLEMQKIVQRDLVMNVYRDGKWGSFRHLPLQQAQPQELTEYAYVNALTRGDLSSLRWIVSPLRHFHATNPNVQLCKVYYASLNFRDIMLATGKLSPDAIPGNWALQQCMLGMEFSGRDLAGRRVMGLLPAKGLATVVDCDKKFLWEVPKNWTLEEAASVPVVYATAYYALVVRGGMKKGESILIHSGSGGVGQAAIAIALSMGCRVFATVGSTEKREYLQARFPQLDASSFASSRNTTFEQHILRVTNGKGVNLVLNSLAEEKLQASLRCLARHGRFLEIGKFDLSNNSQLGMALFLKNVAFHGILLDAIFEDGNEEWEVVSELLKKGIKDGVVKPLRSTVFNKEEVEAAFRFMAQGKHIGKVMIKVQEEEKEYLLRKSEPVTISAISQTSCPPSKSYIITGGLGGFGLELAQWLVERGAQKLILTSRSGIRTGYQAKCVRQWKALGIQVLVSTSDIGTLEGTQLLIEEALQLGPVGGIFNLAVVLRDGMIENQTPELFWEVNKPKYSGTLHLDWVTRKKCPDLDYFVVFSSVSCGRGNAGQSNYGFANSTMERICEQRHHDGLPGLAIQWGAIGDVGILLKTIGNKEVVIGGTVPQQISSCLEVLDIFLNQPHPVVSSFVRAEKVSVKTEGGGQQDLVEAVAHILGVRDTSSLNPESSLADLGLDSLMGVEVRQTLERDYDIVMTMREIRNLTIKKLRELSSKSGTAEELKPSQLMKTGPGEPPKLDLNNLLVNPEGPTITRLNDVQSTERPLFLVHPIEGSIAVFNTLASRLHMPCYGLQCTKAAPLDSIQSLAAYYIDCMKQIQPEGPYRIAGYSFGACVAFEMCSQLQAQQNASHALNSLFLFDGSHSFVAAYTQSYRAKLTQGNEAALETEALCAFVQQFTGIEYNKLLEVLLPLKDFEARVNAAADLITQIHTNINREALSFAAASFYHKLKAADKYIPESKYHGNVTLMRAKSYNEYEEGLGGDYRLSEVCDGKVSVHIIEGDHHTLLEGDGVESIIGIIHSSLAEPRVSVREG

SEQ ID NO: 20 - protein, 2419 aa, Ooceraea biroi
MPAQFESINNPMTRESMARNGVPYSIDSDIVITGISGRLPESSNIEEFKENLMKEMDMVTDDERRWPAGIYGLPLRTAKLKDLDNFDASFFGVHAKQAHVMDPQLRMMLEITYEAIVDAGINPSTIKGSRTGVFVGVSTSESDEYWTKDTEKVNGYGLIGCCRAMFANRVSFAFDFHGPSFVLDTACSSSMVAMHEAVTAMRAGECDAAIVGGMNLLLKPANSLQFHKLGMLSSDGKCKAFDATGKGYVRAEALVAIYLQKAKDARRVYATVVHTKTNMDGYKFQGITYPNGEMQNQLMREVYSETGINPADIVYVEAHGTGTKVGDPEEINSVDQLFCKDRKTPLLIGSVKSNMGHSEPCSGLCSIAKVLIAMESGMIPANLHFSTPNPDIPALMEGRIRVITKATPWNGGLVGINSFGFGGANAHVILRSNSKPKLSPVLDTAKLLPKLVAVSGRTEDAVYTLLDKAKEHRQDDEFLSLLHAMHNNDIPGHGFRGYEILGIDHTRELTEVASYNEKRPIWFVFSGMGTQWSGMGRELLGIEVFRRTLQRCADTLLPHGVDLMNIILNNTNETLENVIDTFVAIAAMQVALIDVLAAIDIYPDGIAGHSVGELGCAYADGAFTAEQTVLAAYWRGKSIVDSTLEPGAMAAVGLSWEDAQKMCPPNVSPACHNSMDSVTISGPTKDVLKFVEELKSKNIFAKLVRSSGIAFHSKYIASAGPKLRASLDKIIPNPKQRSAKWISSSIPEAAWGSPLAQVSSSAYHVNNLLSPVLFQEAIAHIPDNAITIEIAPHCLLQAILRRSLPSTVTNVSLHMRDHTNNLAFLLSNIGKLYMAGAQPNISKLYPPVSFPVGRGTPMIGPLVKWDHSQKWNVASFKKTSGQSGECIVQVDLSKETDAYIAGHQIDGRILFPATGYMLLVWKTLAKLRGTDFELLPVVFENLRFQRATIMPKEGAIKFSINIFEGTGEFEISEAGTVVVRGNIRVSEAIEKDQLKLPPPAVPPVKEEILPLNTKDVYKELKLRGYEYHGIFQGINSCDNYATAGELRWSNEWVSYMDTMLQFSILARKHKLMYIPSRLQYCAINPVLHKQFVEGLPQDGGLPVYYYKNVNIVKSGGIEFRGLNASVVARRQQTQAEPRHERYIFVPYENPHSLVEDPTRGKLHALTILTQIMYENMTALKLKIVEIADERAAEALLTPLVTEIVNNELSSVTVEVQVAAVSPGNYAEAFNHVDVNVSIVAQDANTAPPAQDVHLGVAVDVLSNKSYTILKNLSASLKPSGFILLEETAAHLDLETALKDTDLTLVSRQTDSIGKNYLLLKKLKKSGEPIVIQITEKNLSWVETLKAALKITYTGEQEVLLMSQGEELIGLAGLITCIRKETGGANVRYVFIQDKNSPKFGLSVPYYVNQLDKGLMANVLKGGQWGSYRHLQLDRQNNVSSLQVEHAYVNTLTRGDLGSLRWIEGPLSYYQPDNSSNTMLCSVYYAPLNFKDIMMATGKLPADALPGKMAAEECVLGIEYSGRDENGRRVMGIVEAKGLATTVLTDLDFLWEVPDKWTLEEAATIPVAYATSYYALFVRGQLKAGESVLIHAGSGGVGQAAIAIALRTGCTVFTTVGTLEKRKYLKKRFPQLIDSHIGNSRDTSFEQMILTETQGRGVDLVLNSLAEEKLQAGIRCLAMNGRFLEIGKYDLSNDNNVGMSMFLKNTTFHGVLVDALFYASSLEKKELMRLVSEGIKNGAVQPLPSTVFTEQQVEQGFRYMASGKHIGKVLLKIREEEPKKCVSPAPKTVAAVPRTYMNPEKSYVLIGGLGGFGLELANWMIARGAKFIVLVSRFGITTGYQSLCVRRWRENGVKVVISTMDITTLSGAERLIAQSNQLAPIGGIFNLAAVLRDALIDNQKEADFKAVMLPKVDGTRNLDVVSRKLCPSLDYFVVFSSISSGRGNIGQTNYGFANSAMERMMEERQANGLPGLAIQWGAIGDVGLIIEKMGNSSEIGSTLPQHISSCLATMDIFLQQPHAVLTSVISAEKHKPNTDSNRISLVEAIANILGIKDIKLVNLNNSLADLGMDSLMGTEIKQTLERNYDIALSPQDIRSLTFSKLQELSVTSTTTMKEQQPVAANASTATNSLANAIENNAADNMLLMQWPSNEVLPKEVLVRMKTKSANGPALFIVHAIEGSVNALETLASEFERPVWGLQCVEQAPHDSILELAEFYVKAIRKVQKKGPYHVAGYSFGSCVAIEMAMQLEFAGEKVILSLIDGSPAYIRQQTEMIGKVDTTQEDYIPSDACMKALAYFSIQFNKQLNFFQAYSILKESKSETDMFNKMLQVIGDIPFAQDDLKIAGYLLFKKLTAAMRYSPDKKFKGPVTLIKATDNFLHLTKDYDLSQICVQPARIDEVSGNHRSILLGESAKRIASLLRM

SEQ ID NO: 21 - protein, 2453 aa, Anopheles funestus
MPARFEEVTATDTRRGVPIDLAGGHYDVDAGVGGHAGHRPNIVDDICITGFSGRLPESSDIGEFTRNLLEGVDMVNDDDRRWPAGLYDLPTRIGKIKDEDLQHLDAEFFKIHQKQAECMDPQLRMLLECTHEAIIDAGINPQEIRGSRTGVYIGCSNSETEQHWCADPDLVNGYGLTGCARAMFANRISYTFDFKGPSYAVDTACSSSLFALSQAFADMKAGHCDAAIVAGCGLILKPTMSLQFKRLNMLSKDGMCKAFDESGNGYVRSDGCVVTFLQRASNSRRIYASVLNVRTNTDGFKEQGITYPIGEMQKRLIRETYEEIGLNPADVVYVEAHGTGTKVGDPQEVNAITDFFCKDRKTPLLIGSVKSNMGHSEPASGVCSIAKILIAMEQGVIPGNLHYKNPNPDLYGLLDGRLKVVDRNLPWNGGIIGLNSFGFGGANAHVIMKSNPKPKPISPKDDGFPKLMVASGRTTEAVEAFLDQATVSKDDEEFVGIVNEIHSRNIPLHNYRGYTVVAGDGQSQTVREVLEVTADDKRPVWFIYSGMGSQWASMAKDLMQLEVFHNSIYRCAEALRPEGVDLIDVLTKSDDTKFDNILNSFISIAAVQVALTDVLTHVGITPDGMVGHSVGELGCAYADGCFTPEQTVLAAYWRGRSILDTDLIAGQMAAVGLSWEECKQKLPKDVIPACHNSADSVTISGPVNSVGKVIADLNAQGIFAKGVKSSGIAFHSRYIADAAPKLRKSLDKIIPNPKNRTPRWISTSIPEESWPTPLAQQSSSAYHVNNLLSPVLFSEGLKHVPANAICIEIAPHGLLQAILKRALGKDATNLSLMKRDHANNMIFLLSNLGKLYAAGVQPQVQKLYRPITYPVGRGTPMLNSLVKWDHSINWFLARIGVENKSGETIIDVNLGKDEDAYLAGHTIDGRVLFPATGYLTLAWRTYAKMQGADIEKTPVVIENAVFHRATILPKDGSVKFGINFFDGTGAFEICEGGTLAVSGKLTIPEKIELEELPLNKLEADKSGLALNMSDVYKELRLRGYDYANMFRGVTRSDPRALTGELQWRDNWVSFMDTMLQFSILGKDLRELYLPTRIEKIVINPARHMELVNNLTQTGDDRTLPVYMYRDINVIKSGGVEMRGLRATLAPRRQGTQAPPTLEKYVFVPNNNEKELAEDNSEKARLRSITAAVHLVIENSSGALKIKVAEASFERSPENTMAGTVQAIIEGEPTLASDVAVVTNHQPDTLVQHYGESGVRVINKDAAAGPIEQNCHLAIGYDTFGRADPEAILCNLRDSIKSDGFVLLEESRSTFDARCRATVVKTGFTIISTQVCDKKVFVLLRPIVAELAQRKSIIITISERSFSWVEELKAALAKAEETATYVYIVCQGEELCGAQGLMNCVKNELGGKFARLFFIQDRKADKFSLTSTLYKEQLAKDLICNVLRPANGTPTAAWGCFRHLRLDNQSNAPSLPVEHAYINALTKGDLASLKWIESSLSRDRPDAAARNDRTELCTVYYAPINFRDVMLSSGKLGADALPGDLATQDCILGLEFAGRDSNGRRIMAMVQAKSLATTCVAQRNMIWEIPDNWTMEQASTVPCVYSTVYYALVMRGRMKRGESILIHAGSGGVGQAAISVALAAGVTVYTTVGSKEKREFLKRTFPQLTDRNIGNSRDCSFEQLVMRETQGRGVDLVLNSLAEEKLQASIRCLGLNGRFLEIGKFDLNNNSPLGMSVFLKNTSFHGILLDSVMEGDDDTIAEVVKLVADGIKSGAVRPLPTSVFTEQQVEQAFRFMASGKHIGKVVVRVREEEKAKIVKPSPKLINAIPRTYMHAEKVYILIGGLGGFGLELSNWLVSRGAKIIVLTSRSGVRTGYQSLMIRRWTERGVKVVIDTNDVTTLKGAQKLLTDAARHGPVGGVFNLAAVLRDGLLENSSEADFRAVCVPKVDGTKNLDVATRELCPDLDYFICFSSVSCGRGNQGQVNYGLANSAMERICEARHAAGLPATAIQWGAIGDTGLVLENLGDNDTVVGGTLPQRMPSCLQTMDLFMQQPSPVLASMVIAEKRKTDTGGVSLVGCIANILGLKDTKNVSDGATLADLGMDSLMGAEIKQTLERSFDLVLSAAEIRLLTFGKLRSFEKGGSGGDAGAASGAPAAAAAGAGGKRTDEHAIGDGTQVKFSADLMPKECLVRLESAVPAGSKARPVFAVHAIEGVITALIPLAQTLPVPVYGLQCVEAAPLDSLETLAAYYIKQIRTIQARGPYTIIGYSFGASIAYEMVVQLEKAGDACHLLLLDGSPRYVSWYTEAQKQRNANGEVVQAVDEAYALAYFAMVCGSLDYGRTAKELVEAKSWDDRVAKCAEMVHAKIPQYSRQLLATTARSFVGKIVASHMYKPASKIKATVKLVKPTENYAKLQGDYGLSDLCQQKVEIFTVQGDHRSMLIGDSMKQIASVLQQLF

SEQ ID NO: 22 - protein, 2469 aa, Anopheles darlingi
MPARFEEVTATDTRRGVPIDLAGHYDDHHHDTGSNIGNNHHQQQQHGRRPAIRDDICITGFSGRLPESSNIDEFRRNLFEGVDMVNDDDRRWPSGLYDLPTRIGKIKDEDLQHLDAEFFKIHQKQAECMDPQLRMLLECTHEAIVDAGINPQEIRGSRTGVYIGCSNSETEQHWCADPDLVNGYGLTGCARAMFANRLSFTFDFKGPSYAVDTACSSSLFALSQAFADMKAGHCDAAIVAGCGLILKPTMSLQFKRLNMLSKDGMCKAFDESGNGYVRSDGCVVTFLQRASDSRRVYASVLNVRTNTDGFKNQGITYPIGEMQKRLIRETYEEIGLNAADVVYVEAHGTGTKVGDPQEVNAITDYFCKDRKTPLLIGSVKSNMGHSEPASGVCSIAKILIAMEAGVLPGNLHYRNPNPDLYGLLDGRLKVVDRNMPWNGGIIGLNSFGFGGANAHVILKSNPKPKPISPRDDAFPKLVLASGRTTEAVEAFLDQTAISKDDEEFVGLVNEINSRNTPLHYHRGYTVVSGDGKPPVREVLEVSDEKRPLWFIYSGMGSQWASMARDLMQLEVFHSTIARCAEALRPEGIDLIDVLTKSDESRFDNILNSFISIAAVQVALTDVLTHVGIVPEGMVGHSVGELGCAYADGCFTPEQTVLAAYWRGRSILDTDLIAGQMAAVGLSWEDCKQKLPKDVIPACHNSSDSVTISGPVASVGKVIADLNAQGIFAKGVKSSGIAFHSRYIADAAPKLRKSLDKIIPNPKPRTQRWISTSIPEESWGTALAQQSSSAYHVNNLLSPVLFAEGLKHVPANAICIEIAPHGLLQAILKRALGKEATNLSLMKRDHDNNLIFLLSNLGKLYAAGAQPQVQKLYPPITYPVGRGTPMLNSLVKWDHSDKWFLARIGVENKSGETIIDVNLGKDEDAYLAGHTIDGRVLFPATGYLTLAWRTFAKMRGADLEKTPVVIENAVFHRATILPRDGSVKFGINFFDGTGAFEICEGGTLAVSGKLTIPEKIELEELPLAKLEADRSALPLNTSDIYKELRLRGYDYGGMFRGVTRSDSKALTGELQWRDNWVSFMDTMLQFSILGKDLRELYLPTRIEKIVINPARHLEIVSGLPVAKDGTDRTLPVYMYRDINVIKSGGVEMRGLRATLAPRRQGTQAAPTLEKYVFVPNSNEKELAENADKARLRSITSAVHLVIENSAGALKIKVVEASAERSPENTMAGTVQGIIEGEPTLASDVAIATTHQPDSLVQHYGESGVRVLNKDIAAGAIEQGCHLAIAYDVFGSGATADVLRNLRDTIKTEGFVLLEESRTGIDLSAKGAVRNALSKAGFLLVSEQVCDKKVFLLVRPILAEIAQRKSTIVTITEKNFSWLDSLKTALAKAEESSTYVYVVCQGEELCGAQGLLNCIKNEAGGKFARLFFIQDRSAEKFSLTSALYREQAAKDLICNVLRPANGSPACWGTFRHLRLDSQSNAPSLPVEHAYINALTKGDLASLKWIESSLSRDRPAGDDRTELCTVYYAPINFRDVMLSSGKLGADALPGDLATHDCVLGLEFAGRDSSGRRIMAMVQAKSLATTCVAQRNMIWSIPDSWTMEQASTVPCVYSTVYYALVMRGRMKRGESILIHAGSGGVGQAAISVALAAGVTVYTTVGSAEKRAFLKRTFPQLTDRHIGNSRDCSFEQLVMRETQGRGVDLVLNSLAEEKLQASVRCLGLNGRFLEIGKFDLNNNSPLGMSVFLKNTQFHGILLDSVMEGDDETIAEVVRLVADGIANGAVRPLPTSVFSETQVEQAFRFMASGKHIGKVVIRVRDEEKQKVLKPAPKLINAIPRTYMHAEKAYILIGGLGGFGLELSNWLVSRGAKILVLTSRSGIRSGYQALMVRRWTERGVKVVIDTNDVTTLKGAQKLLTEAARHGPVGGVFNLAAVLRDGLLENSSEADFKAVCVPKVDGSKNLDQATRELCPDLDYFVCFSSVSCGRGNIGQVNYGLANSAMERICEARHAAGLPATAIQWGAIGDTGLVLENLGDNDTVVGGTLPQRMPSCLQTMDLFMQQPCPVLASMVIAEKRKTETGGVSLVSCIANILGLKDTKNVSDASTLADLGMDSLMGAEIKQTLERSFDLVLSAAEIRLLTFGKLRSFEKGGITSDGAAGGDGAAADGGSGAGGAAAKSAADQQTAIGDGTQVMFSAELMPKECLVKLESAAPPSKSPARPVFVVHAIEGVITALIPLAKTLPVPVYGLQCVEAAPLESLVVLAGYYIQQIKTVQPRGPYTIVGYSFGASIAYEMVAQLEAAGEKCSLLLLDGSPRYVSWYTEAQKQRNANGEVVQAEDEAYALAYFAMVCGKLDYGKTAHELVSAKSWNERVAKCAEMVHAKAPQYSKQLLETTARSFVGKIVASHMYKPSSKINANVKLVKPTENYAKLQGDYGLSDLCKQKVEILTVKGDHRSMLTGESMKQIAAALHQLC

SEQ ID NO: 23 - protein, 2540 aa, Glossina austeni
MYISVDFKSNDQIFILLHGAKANKINPSQVNHNRQHTNNNSNNENKNDSQKSSNKGKSANRRRKRRQKNSQNSNFSENPQQNHQDDVAQIVVKDNPSTSFPFHFSSSNSNYDSSSFPLVNGRLHKDSIMPARFVENSEPSVPMNLENRYDHPSSNGVNSDIVITGISGRLPESTNIEEFRKNLFEGVDMVNDEPRRWSKGLYGLPERNGKIKEEDLENFDQTFFGIHQKQADGMDPQMRMLLECTYEAIIDAGLNPAEIRGTRTGVYVGASSADSENYQLSDPDRVDGYGLIGCARAMFPNRISFSFDLKGPSYCVDTACSSSLYALSQAFADMNSGKCDAAIVAGSNLCLRPTMSLQFKRLSMLSAEGKCKAFDESGSGYVRSDAVVVILLQRVSVAKRVYATILNARTNVDGHKEQGITFPNGQMQNQLMRETYGEINLDPAEVNYVEAHGTGTKVGDPQEVNSITDFFCKNRKSPLLVGSVKSNMGHSEPSSGLCSIAKVLLAMEQNVLPPNLHYKNPNPDLYGLLDGRLKVVDKPTPWEGGIVGINSFGFGGANAHVILKSNPKPKVITPTVGPPKLILCSGRTSDAVQEFLEDAEQHKDDDEYLTLINDIHSRPISGHYYRGFSVMDSKGALQKDVAEINPESRPIWFVYSGMGSQWASMAKDLMVFDTFKKTIHRCCEILRPEGLDLMEVLTRSTEKTFENILNSFVGIAAMQVALTDLLTSLNIVPDGIVGHSVGEVACAYADGCLSMEQTILAAYWRGKSILDTKLTKGKMAAVGLSWEEAHKRLPADCFPACHNSAENCTISGPEESIDAVCQKLTAEGVFARAVKSSGYAFHSKYIADAGPKLRKSLEKVIPNAKNRSPRWISSSIPEVAWNTAIAQQASAAYHVNNLLSPVLFHQALQHVPKNAICIEVAPTGLLQAILKRSLGNETTNLSLIKRDYENNPEFFLASIGKLYAAGAQPQIMTLSKPISYPVGRGTPMLGCKVGWDHSQKWHVPKFDKMTSSGETIIEVDLSKEEDAFLAGHTIDGRILFPATGYMTLAWMTYAKMRGHEFQKTPVVMENVVFHRATILNKEGVVKFGINFFDGTGAFEICEGGSLAVSGKISIPENVDNEQLPLDPLPVSTVAKELSTSDVYKELRLRGYDYAGIFRGITASDSLSSTGKLQWVDNWISFMDTMLQFSILSKNLRELYLPTRIEKAIINPDHHLKEIAKLTPEQQTKEGVPVYMYDDINVIKSGGIELRGMKASLAQKRPSNQNPPTLERYAFIPNENGVDLNENHEKAHFHALSVALRLLNENSSGALKIKGVELADGRNPDSLLAAKIVQVLEGEPSLTAEIAVATSNSNEEAISAALGPDAGVRVISKNILKEPVDQNNHFVFGVDVLSRPDTAVLVNSLASIKDNGFLIFEESAYGYRNTGRNLLTEFGLVVASEQSCGNSRVLVMARRPVDLKQRKSVVINVTEKNFDWLEELKAALAKAAENEQYVYIVCQGEEAFGAVGLMTCIRRENGGNFARLVFVQDGNAKPFSFNDAFYTKQLAKDLISNVLKNGLWGTYRHMKLETNAATLQVEHAYVNALVKGDLASLKWIESPRLTPNISNDFELCTVYYAPINFRDVMLSSGKLSADALPGDLAQQDCVLGLEFSGRDSKGRRIMAMVPAKSLATTCVAAKIMTWQIPDKWSMEEASTVPCVYSTVYYALMVRGQMKKGEKILIHAGSGGVGQAAISVALHHGLTVFTTVGSKEKREFLKKRFPQLKDNHIGNSRDTSFEQMIMRETQGRGVDLVLNSLAEEKLQASVRCLGLNGRFLEIGKFDLSNNSPLGMSVFLKNTSFHGILLDSVMEGEEAMQKQVVDLVAEGIKNGAVRPLPTSVFNDQQVEAAFRFMASGKHIGKVVVKIRDEEPGSKAIKPPTHLVNAIPRTYMHPEKSYVLIGGLGGFGLELTNWLVFRGAKHIVLNSRSGLRTGYQALMVRRWQEKGVKVLVDTSDVTNASGCKQLLTNANKLATVGGIFSLAAVLRDDILENQTAKDFKTVCDPKVTATKLLDQCSRSLCTSLDHFVCFSSVSCGRGNIGQSNYGLANSAMERICEARQASGFPGLAIQWGAIGDTGLVIETLGDNDTVIGGTLPQRMNSCLQTIDLFLQQPHPVLASMVVAEKRKSDQSGGVSLIASVANILGIRNIKNIPEKSSLADLGMDSLMGAEIKQTLERNFDIVLSAQEIRQLTFGALTQMDSGPARAESATSPQATSPSAFGDGTQDVFSSELMPTETIVRLKSKAPADSNKRPLFIASPIEGFADPLKNLAELLDCPVYGLQCTANADLDTIQSLASFYLKEVRKIQAKGPYVIAGYSFGAAVAFEMVINLQSHDIVSNYIALDGAPKYVSWNTSSFKDRRSMDDGDNYDYGLAYFAMVVANMDYAFVVKMLLDKPTWQEKLAKCAEMVAQEIKKPIDLIKQAGEIFYKKLSAGHNYKATTKITCPVTLVKPSENYVQLEEDYGFNEICQKPVKVFTVEGNHRTFLVEEASLKTIESELNRLTA

SEQ ID NO: 24 - protein, 2540 aa, Drosophila melanogaster
MPLQLNLLQAVDQPHPVAFKPNNCSTHQPQHSPSTQNNGKSARANRRRRRRRNKQQQNSQQPDAFRDTDAQLTPSTSSSTPHSAPNDRQDHLNSQFNPESINMPARFAEEVITAEPAQRAAPQLDLGGGHYVPRQQHLNDEIAITGFSGRLPESSTIEEFKQNLFDGVDMVNDDPRRWERGLYGLPDRIGKLKDSDLENFDQQFFGVHQKQAECMDPLLRMLLELTHEAIIDAGLNPSDLRGSRTGVYIGVSNSETEQHWCSDADRVNGYGLTGCARAMFANRISFTFDFKGPSYSIDTACSSSLYALEQAFSDMREGKVDNALVAGAGLILKPTMSLQFKRLNMLSPDGSCKAFDESGNGYVRSDGCVVLLLQRTSAARRVYASILNVRTNTDGFKEQGITYPIGKMQNRLIRETYEEIGLNPADVVYVEAHGTGTKVGDPQEVNSITDFFCKDRTTPLLIGSVKSNMGHSEPASGVCSVAKILIAMEEGVIPGNLHYNKPNPDLYGLVDGRLKVVDRNLPWNGGIIGLNSFGFGGANAHVILKSNPKPKALTPKDGALKVVLASGRTFEAVEQLLESASTNADDDEYLQLINEIHSKAIPNHFFRGYGVVSSKGTHQREVIESNDDKRPIWYIYSGMGSQWASMAKDLMKIEAFAKTIQRCADVLKPEGVDLIDVLTRSTDKSFENILNSFISIAAMQVALTDLLSSLGIHPDGIVGHSVGELGCAYADGCFTPEQTVLAAYWRGKSILDTQLAKGKMAAVGLSWEDAHSRVPSDCFPVCHNSEDNCTISGPEASIEALVAKLNAEGVFAKAVNSSGYAFHSKYIAEAGPKLRKSLEKIIPNAKNRTARWISTSIPESAWNTPVAKQSSAAYHVNNLLSPVLFHEALQHVPKNAISVEIAPHGLLQAILKRALGPDATNLSLVKRGHENNVEFFLTNVGKLFAAGAQPQVLTLVRPISYPVGRGTPMLNSKVGWDHTQKWLVAKFGKETSSGETIVEVDLSKEDDAFLAGHTIDGRILFPATGYMTLAWQTFAKMQGSEFHKTPVVMENLVFHRATILNKNAVVKFGINFFDGTGAFEICESGSLAVSGKITIPESIDNEELPLEEQTPSAVAKELGTNDVYKELRLRGYDYGGIFRGIVRSDTVASTGKLQWVDNWISFMDTMLQFSILSKNLRELYLPTRIERAVINPAKHFELLSALTKEEQVETGLPVQWYSDINVIKSAGVELRGLKANLAQRRPGTQAPPTLERYQFVPNINTTDLNENSEKARLHALDVAIQVIIENSSGAVKLKGVELANGRNPDVLVANRLLQIIEGEPVLTGDVAVVTSNNNEETITAALGDSGVRVVSKDVLKEPVEQNCHFVFGIDVLSRPDTKTLENSIASIRENGFLILEETLPTYTKTGRALLTKFGFVAVQEQSLGATRVLVLARKAVDLKTRKSVVVVATEQNFNWVDDLKAALATAATEEQYVYVVCQGEELFGAVGLMTCIKNENGGKLARLVFVQDAKAEKFSLTSTLYRQQLEKDLISNVLKNGAWGTFRHLKLETQQATLQVEHAYVNALVKGDLASLKWIEAAQADTAATVDKNLETCTVYYAPINFRDVMLTSGKLAADALPGDLAEQDCVLGLEFAGRDTQGRRVMAMVPAKSLATTCVASKRMMWQIPEKWTMEEASTVPCVYSTVYYALVVRGQMKKGEKILIHAGSGGVGQAAISVALAHGLTVFTTVGSKEKREFLLKRFPKLQERNIGNSRDTSFEQLVLRETKGRGVDLVLNSLSEEKLQASIRCLGLNGRFLEIGKFDLSNNSPLGMSVFLKNTSFHGILLDSVMEGEEEMQNQVVSLVAEGIKTGAVVPLPTSVFNDQQVEQAFRFMASGKHIGKVVIKVRDEEAGKKALQPKPRLINAIPRTYMHPEKSYILVGGLGGFGLELTNWLVTRGARYIVLTSRSGVKTGYQGLMIRRWQERGVKVVIDTSDVTTAAGAKKLLENSNKLALVGGIFNLAAVLRDALIEDQTAKDFKTVADPKVTATKYLDQFSRDICTELDYFICFSSVSCGRGNIGQTNYGLANSAMERICEQRQVSGFPGTAIQWGAIGDTGLVLENLGDNDTVIGGTLPQRMPSCLQTIDLFLQQPHPVVASMVVAEKRKSDQSAGVSLIATIANILGLRDTKNIQDGASLADLGMDSLMSAEIKQTLERNFDIVLSAQEIRQLTFGALKAMDGGADVKPAAAAPAAAAGVPEANITSGGSSRTASPMGDGTQVVFTTSLIPTEAIVQLDTKAPANSKQSPIFFISPIEGFASALEPLAKRLEVPAYGLQYTEAVPSDSLESAAKFFIKQLRTVQPKGPYKLAGYSFGCLLTYVMAGILEETNEVANVIMLDGAPSYVNWYTSSFKQRYTDGTNADNDNQSYGLAYFGIVLANIDYKALVRLLIVIPTWEEKLERFAELMSNEITQPVETIKKSATLFYKKLELADGYQPTLKLKTNVTLVKPTDNSAKLDEDYRLKEVCTKPVEVHTVEGNHRTFLIEDQSLKTIQSILKRLFN

SEQ ID NO: 25 - protein, 2574 aa, Brugia malayi
MNSSGEVPFWRDQEEIVITGISGRFPRCENVQEFGDLLLAGEDLVTEDSLRWPPGVFDLPKRHGKLKDLKKFDAQYFGVTPKQANYLDPQVRKLLEVTLEAIIDAGLNPTELRGSRTGVFVGCSASETGGVLTQDPETVTGYTLTGCVRSMFSNRLSFTFDLRGPSFSVDTACSSSLCALQLAVDAIRQEQCDAAIVAGAHLTLTPTAALQFLRLGMLSDKGSCRSFDASGDGYCRTEAIAAILLQRQSAARRIYATVVHAKSNTDGYKEQGITFPSGERQAALLEEVYREAGVDPNTVTYVESHGTGTKVGDPQEANAICQVFCQNRNSALLIGSVKSNMGHAEPASGLCSIAKVLIAMERGFIPPNLHYNEPNPYIPGLTDGRLQVVTEKTPFQRGLVGINSFGFGGSNTHIILRPANHSERKPAPTTFMKIIPYSGRTAEAVNNILDCVLAHPENAYLQQLLANQANLPAKDTPYRGYVIINQLPPLRDVQKIMITEPKQIYFIYSGMGSQWAGMVRQLMSIPAFDESLRSSSDAIVDFGVNVYEMLQSDDPSFYKNNTLNCMLAITAIQIALTDVLFLLGVMPDGIIGHSTGEMCCGYADGGLTREQTMQLAYHRGHTIMNANIKGGMAAVGLSWEEAGKRCPEGVIPACHNAADSVTISGDAEKIKEFVEELKKEDIFGKLVDSSGIPFHSPAMLKVKDKMLKAMRTSVPNPKPRSSRWISTSIPESNWENELAQMCSADYHTNNAVSPVLFYEALQKIPANAVTIEIAPHCLMHSILRRSLQKTCTNVGLINMKEKDRELESFLQALGKIYQTGITIHIEALYPAIQYPVPIGTPMISPMWRWDHSQDWPVVDGKTLSAAGGRQLPASYCYTVDPFASDSKETFLLDHIIDGRVLYPFTGHMVLAWKTIAKLNGVDFLKTPVILEEIRVYSATIVTKPIRLDVIVTPGNGYFEILDGDQLAASGYIRIVDEDVPFYYKSIQEIQTSEIAERIELDTEDAYKEFLLRGYEYGQAFRGIYRACNSGERGMLYWTGNWVTFLDSLLQTALLAERADSLRLPTRVRYLRIDPVKHMEHIQERDGIQVIELRNDVATNGCIAGGVECCDLTAHTVARRLQSSGQLYYEKIYFTKHFDMKAFDEFPQIREELNAYRDFLRSLLANGLAKWEVNGCLKELTNGALLSGAVRKFTKSPVATVFDEIFAIEIGNNPKDFENKVAEKMQSMLKIFNVDRLWSAAIVHDRILKTIQDTCIENSTGHNCKACALEFNSTEQLKFCVDAVNSHPLLEVEWLCVGPKVDDMDESTLVQLGVKKVTTVLDEKQFVPSAEIKNCDIIILDKILSQKKDVVRYLSRCKEMLRDDGFIILVETTSDYEIALAIQGLNAETISISDSGRIYGAYFTHDQLLKLFEECDFRLCNYQSDPSMMTTMYAIRKIPSQPREPIVIDVDDIKEFTWIEPLQKAIEERLNEPDYKTIWLTSTTVRNNGLLGLALCFNEENLKSNRFRTLIDMSVKKENRTGPAQIGMEHESVKQLVKLDLHANNYRDGVWGSMRHLVVKDDEMHLYKDVEHAFINTLIRGDVSSLTWFESPNQFFEDTCQKNPSLELCNVYYSAINFRDVMLAYGRLPPDAIPGQFADRECLLGMEFSGRLKDGTRLMGILPAQALATSVIVNREYAWTVPDNWSLTDAATVPVVYTTAYYALVMRGRIRRGDKVLIHGGSGGVGQAAISVALSRGCEVFTTVGNAEKKAFLQKRFPQLKDRHFANSRNSDFELHIRHQTRGRGVDVVLNSLAQHMLQASIRCLAQNGRFLEIGKVDLSQNSPLGMAVFLKNITFHGILLDAVMDPSVGKKEDWQEVARLVQDGIKSGIVQPLSYTTFSSEKAEEAFRFMSSGKHIGKVLMEIRREEPERVCVPSPIKVRAICRTLCHPNHVYLITGGLGGFGLELSQWLINRGAKKLVLTSRMGIRTGYQARCVHFWRRTGISVLVSTLNIAHLSDAHELISQCKALGPVGGVFHLAMVLRDCLFENQNVQNFKDAAEAKYWGTLNLDAATRDACGKELRWFVAFSSITSGRGNAGQTNYGWSNCTMERIIEHRREDGFPGIAIQWGAIGDVGVILENMGDNNTVVGGTLPQRMPSCLAALDLFLSWNHPIVASYIKADIGAKKVGSSGNLWQTMAHILGVNDAAQLNPDAYLGDLGLDSLMGVEIKQALERDYDIVLSMKDIRTLTLNKLQQLVDSGGTTSTVLQTTELELKKESEKEAEQNTVEQLERQMNQLFKMRVDVNDLEPMDLIIKCNKVEAGPPTFFVHSIEGIATPLKKVMSKCNFPAYCFQSTREVPQDSIEKVAQKYILEMKKIQPEGPYRIIGYSYGACIGFEMATMLQESDGANSVERLILLDGSHLYMQTYRNVYRMAFGVTGDTLVNNPLFESEIMCAMTLRFANVDYKKFRVELLQQPGFKARVQKVVDTVMTTGLFKSADTIDFACCAMRSKFVMADKYKPERKFKGLITLIRAEQGAAREEDVGSDYGISQVSDENKVYIVEGDHDSFVQGKTSAKTVNIINDLIAEANKKAKNV

SEQ ID NO: 26 - protein, 2613 aa, Caenorhabditis elegans
MDNTGEGSSDSSGTWERISDNSQSSDNMDPTQWWQKQDDIVISGVSGRFPRCDNVKMFGDMLLAGEDLVTEDSLRWTPGFCDLPKRHGKLKVLNKFDAGFFQVTPKQANFMDPQVRLLLEASWEAMVDAGINPTDLRGSKTGVFVGCSASETSGMLTQDPDTVTGYTLTGCVRSMFSNRISYTFDLQGPSFSVDTACSSSLLALQLAVDSIRQGQCDAAIVAGAHLTLTPTAALQFLRLGMLTDKGSCRSFDESGDGYCRTEGVAAIFIQRKKKAQRLYATVVHAKSNTDGHKEHGITFPSGERQAQLLQEVYSEAGIDPNSVYYVEAHGTGTKVGDPQEANAICEVFCSKRTDSLLIGSVKSNMGHAEPASGVCSLTKILLSIERQLIPPNLHYNTPNQYIPGLTDGRLKVVTEPTALPGGLIGINSFGFGGSNTHVILKAADHIAPPITPHPFTKLVTYCGRTQEAVENIFTEIESNKDDLYLQALLANQANMPANLLPFRGYMLLDRENNVETLKSITKVPITEARPIYFIYSGMGSQWPGMAIKLMKIPMFDDSLRASSKTLEEFGLDVYGMLCNPDPEQYSNNTMNCMLAITAIQIALTDVLTALGVSPDGIIGHSTGEMGCGYADGGITREQTMRLAYHRGTTIMKHTEIKGAMAAVGLTWEQVKEQAPPGVVAACHNGADSVTISGDAEGVATFCAQLKEKDIFAKVVDTSGIPFHSPAMLAVQDEMIECMRTAVPEPKPRSSKWISTSIPEDDWESDLAATCSAEYHVHNACSPVLFYEAIQKIPANAVTIEMAPHSLMQAILRRSLQKTVTNVGLMNRPKSENDDELESFLGSLGKIYQAGVNIQITELYPGGQYKGVVPKGTPMIGPMWKWDHTQDWLTIDGRQVLAGGSGSVASSATYNIDPFATDSKETYLLDHVIDGRVLYPFTGHMVLAWRTLCKLKGLDYTKTPVVFENINVFSATILTKPIKLDVVLSPGNGYFEIISDDQVAASGRIYIPEDNQPFYYGKLEDIRTSEIADRIELDTEDAYKEFLLRGYEYGQAFRGIYKTCNSGERGFLYWTGNWVTFLDSLLQTALLAERSDTLRLPTRVRHLRIDPNKHLEHVVEKDGIQVIELRNDHSTNGCIAGGVECCDLNAHSVARRIQVSGQLYHEKIFFVPHFDHNCLSGHKKTSTILKDYSAVIKQQLYTGFSKWQSAGLLKKLKNGAQIVKALAVLKASQSDVVLDDTVTRFTHDGKCTVLHHIADMFKIEDCEDFEDRVAAKLKSVRGIFELDRLWAGAVLNDRIVKSLQDICIENSAGHHATMAAVDLVSTDQIRHCIEANSSHPLLETDYTCIGANVDHLDESTLEIIGGKKQKIDLENNFTGHGEVKNLDYVLLDKVISKKADPIAFIEACKHLIRETGFLLVVEVTSQYEIALAIEGLLGNEMVGDASRKYNQFFTHEQLLDMFKSTGFLICNFQSDPALMTTTYAVRRVSPIPRDPVFIDVDDVKEFNWIEPLQKVSEERLNEPDSKTIWLVSNKCRNNGIVGLGLCFVEENLKINRFRSAFDMSANKEIRDGPPVWNIGDEETKKIVELDLHANDYMDGQWGSMRHIVVKDEDVHVYKDCEHAFINTLTRGDVSSLTWFESPNQYFDSMVKSKATQELCSVYYAPINFRDIMLAYGRLPPDAIPGNFADRECLLGMEFSGRLKDGTRLMGILPAQALATTVMVDRDYAWEVPRDWTLAEASTVPVVYTTAYYALVRRGLMKKGDKILIHGGAGGVGQAAIAIALAAGCEVFTTVGSAEKREFLKNLFPQLQEHHFANSRSADFELHIRQHTKGRGVNIVLNSLANEMLQASLRCLARHGRFLEIGKVDLSQNSSLGMAKLLDNVSVHGILLDSIMDPTVGDLDEWKEIARLLEQGIKSGVVKPLHSHSFPADKAEEAFRFMSAGKHIGKVIMEIRPDEGTKVCPPSKISVRAICRTLCHPQHTYLITGGLGGFGLELAQWLINRGARKLVLTSRTGIRTGYQARCVHFWRRTGVSVLVSTLNIAKKSDAVELINQCTAMGPIGGIFHLAMVLRDCLFENQNVQNFKDAAEAKYYGTINLDYASREHCDKNILKWFVVFSSITSGRGNAGQTNYGWSNSCMERMIDQRRADGFPGIAIQWGAIGDVGVILENMGDNNTVVGGTLPQRMPSCLSSLDNFLSWNHPIVSSFIKAELGSKKNVGGGDLMATIAHILGVNDISQLNADANLSDLGLDSLMGVEIKQALERDHDIVLSMKEIRTLTLNKLQQLADQGGTGRTALQVNELEMKKDGERDAELNTAEMLEQQMNQLFKMRVDVNDLDPQDIIVKANKVEEGPITFFVHSIEGIATPLKKVMNKCEFPAYCFQSTKNVPQTSIEDVAKCYIREMKKIQPSGPYRLVGYSYGACIGFEMANMLQESDGRDAVERLILLDGSHLYMQTYRNVYRMAFGVTGDSLVNNPLFESEIMCAMTLRFANVDYKKFRFELLQQPGFKARVQKVVDQVMLTGLFKSPETVAFACEAMHSKFLMADKYKPRRNFGGHITLIRAEQGAAREEDVGEDYGVAAVSEDCEVLKVKGDHDTFVQGKSSSVTVEHINRIILQ

SEQ ID NO: 27 - protein, 2731 aa, Caenorhabditis briggsae
MDNTGEGSSDSSGTWERISDNSQVSLLPEFRLSVSPNLSTVLLRSGRGHHHLRFSSLLLFYLLPSLPRARIRIVFASLLLLFLNVFVRSADAFLFFFSFFVYLFPLSFFRSSDNMESTNWWQKQDDIVISGVSGRFPRCDNVKEFGDLLLAGEDLVTEDDLRWPPGFYDLPKRHGKLKELKKFDAGFFSVTPKQANFMDPQVRILLEASWEAMVDAGMFLSISHFIPLFGTETEIGKLCLSPDVPGSINPIDLRGSKTGVFVGCSASETSGALTQDPESVTGYTLTGCVRSMFSNRISYTFDLQGPSFSVDTACSSSLLALQLAIDSIRQGQCDAAIVAGAHLTLTPTAALQFLRLGMLTDKGSCRSFDDSGDGYCRTEGVAAIFIQRKKKAQRIYATVLHAKSNTDGYKEQGITFPSGERQAQLLQEVYSEAGVDPNSVYYVESHGTGTKVGDPQEANAICQVFCSSRSDSLLIGSVKSNMGHAEPASGVMSLTKILLSIERQMIPPNLHYNTPNQYIPGLVDGRLKVVTEPTPLPGGIIGVNSFGFGGSNTHVILKAADHVAPAITQHPFTKIVTYCGRTQESVEKIFGEIEANKDDLYLQSLLANQANMPANLLPFRGFMLLDRENNQAALKNITKVPITEPRPIYFIYSGMGSQWPGMAIELMKIPMYDESLRASSKTLEEFGLDVYGMLCNPDPEQYSNNTMNCMLAITAIQIALTDTLTALGVSPDGIIGHSTGEMGCGYADGGITREQTMRLAYHRGTTIMKHTEIKGAMAAVGLTWEEVKAQAPPGVVAACHNGADSVTISGDAEGVASFCAQLKEKEIFAKVVDTSGIPFHSPAMLAVKDEMIESMRTAVPEPKPRSSKWISTSIPEEDWESDLAATCSAEYHVHNACSPVLFYEALQKIPANAVTIEMAPHSLMQAILRRSLQKTVTNVGLMNKPKSENDNELEGFLGSLGKIYQAGVNIQISELYPGGQYKGVVPKGTPMIGPMWQWDHSQDWQTIDGRHMVAGGGGSIPASATYNIDPFAADSKEAYLLDHVIDGRVLYPFTGHMVLAWKTLCKLKSLDFQKTPVVFENINVYSATIVTKPIKLDVVLTPGNGYFEIISDEQVAASGRIYVPEDNQPFYYGKLEDIRTSEIADRIELDTEDAYKEFLLRGYEYGQAFRGIYKTCNSGERGYLYWTGNWVTFLDSLLQTALLAERSDTLRLPTRVRHLRIDPNKHLEHVVERDGIQVVELRNDHSTNGCIAGGVECCDLNAHSVARRIQVSGQLYHEKVFFVPHFDTNCLKQHNETAATLKDYTSVIKQTLFNGFSAWKSAGLLKKLKNGALIEKALPALKSSLSDVVLDDTVTRFMHDGKCTVLPHFTEMFKIQDSEDFEDQVIGKLKSVRGIFELDRLWAGAVLNDRIVKSLQDICIENSAGHHAKMAAVDLVSTDQIRHCIEANSSHPLLEVDYTCVGATVDHLDESTLEIVGAKKQKIVLDEAFTGHGELKNMDYVLLDKVLNKKADPIAFIEACKNLIRDDGFLLVVEVTAQYEIALAIEALLGTDLAGDANRQYGQFFTHEQLLKMFETTGFKICNYQSDPALMTTTYAVRRIASVPRDPAFIDVDDIKEFSWIEPLQKTVEERLNEPDAKTIWLVSNKCRNNGIVGLALCFVEENLKSNRFRSAFDMSATKAIRDGPPVWNIGDEETKKIIDLDMHANDYMDGQWGSMRHIVVKDEDAHVYKDCEHAFINTLTRGDVSSLTWFESPNQYFDSMAKTKSSQELCSVYYAPINFRDIMLAYGRLPPDAIPGNFADRECLLGMEFSGRLKDGTRLMGILPAQALATTVMVDRDYAWEVPSDWTLAEASTVPVVYTTAYYALVRRGMMKKGDKVLIHGGAGGVGQAAIAIALAAGCEVFTTVGSTEKREFLKKLFPQLKEHHFANSRSADFELHIRQHTKGRGVNIVLNSLANEMLQASLRCLARHGRFLEIGKVDLSQNSSLGMAKLLDNVSVHGILLDSIMDPTVGDLEEWKEIARLLEQGIKSGVVKPLHSHSFPADKAEEAFRFMSAGKHIGKVIMEIRQEETTKVCPPSRISVRAICRTLCHPQHTYLITGGLGGFGLELAQWLINRGARKLVLTSRTGIRTGYQARCVHFWRRTGVSILVSTLNIAKKSDAVELVKQCTAMGPVGGVFHLAMVLRDCLFENQNIQNFKDAAEAKYYGTINLDYATREDTVKEHLKWFVVFSSITSGRGNAGQTNYGWSNSCMERMIDQRRADGFPGIAIQWGAIGDVGVILENMGDNNTVVGGTLPQRMPSCLSSLDNFLSWNHPIVSSYIKADMGAKKSAGGGNLMQTIAHILGVNDISQLNPDANLGDLGLDSLMGVEIKQALERDYDIVLSMKDIRTLTLNKLQQLAEQGGTGGTALQVNELEMKKDGERDAELNTVEMLEKQMNQLFKMRVDVNDLDPQDVIVKANKAEEGPITFFVHSIEGIATPLKKVMSKCEFPVYCFQATKNVPQTSIEDVAKYYIREMKKVQPTGPYRLVGYSYGACIGFEMACMLQQSDGQDAVEKLVLLDGSHLYMQTYRNVYRMAFGVTGDTLVNNPLFESEIMCAMTLRFANVDYKKFRVELLQQPGFKARVQKVVDTVMTTGLFKSPETVAFACMAMHSKFLMADKYKPERKFRGHITLIRAEQGAAREEDVGRDYGISQVSDDSDVHVVEGDHDTFVQGKSSAKTVSIINSLILNN

SEQ ID NO: 28 - protein, 2587 aa, Caenorhabditis remanei
MESNSWWQKQDDIVISGVSGRFPRCDNVKEFGDLLLAGEDLVTEDDLRWPPGFYDLPKRHGKLKELKKFDAGFFQVTPKQANFMDPQVRILLEASWEAMVDAGINPIDLRGSKTGVFVGCSASETSGALTQDPESVTGYTLTGCVRSMFSNRISYTFDLQGPSFSVDTACSSSLLALQLAIDSIRQGQCDAALVAGAHLTLTPTAALQFLRLGMLTDKGSCRSFDDSGDGYCRTEGVAAIFIQRKKKAQRIYATVLHAKSNTDGYKEQGITFPSGERQAQLLQEVYSEAGVDPNSVYYVESHGTGTKVGDPQEANAICQVFCSNRSDSLLIGSVKSNMGHAEPASGVCSLTKILLAIERQMIPPNLHYNTPNQYIPGLVDGRLKVVTEPTPLPGGVIGVNSFGFGGSNTHVILRAADHVAPAIHQHPFTKIVTYCGRTQESVEKMFAEIEANKENLYLQALLANQANMPANLLPFRGYMLLDRENAQSPMKNITKVPITEPRPIYFIYSGMGSQWPGMAIKLMKIPMFDESLRASSKTLDEYGLDVYGMLCNPDPEQYSNNTMNCMLAITAIQIALTDTLTALGVSPDGIIGHSTGEMGCGYADGGITREQTMRLAYYRGTTIMNHTEIKGAMAAVGLTWEEVKAQAPKGVVAACHNGADSVTISGDAEGVATFCAQLKEKDIFAKVVDTSGIPFHSPAMLAVKDEMIESMRTAVPEPKPRSSKWISTSIPEEDWESDLAATCSAEYHVHNACSPVLFYEALQKIPANAVTIEMAPHSLMQAILRRSLMKTVTNVGLMNKPKSENDDELESFLGSLGKIYQAGVNIQISELYPGGQYKGVVPKGTPMIGPMWQWDHSQDWQTIDGRHMVAGGGGSIPASATYNIDPFAADSKEAYLLDHCIDGRVLYPFTGHMVLAWKTLCKLKSLDFQKTPVVFENINVYSATIVTKPIKLDVVLSPGNGYFEIISDEQVAASGRIYVPEDNQPFYYGKLEDIRTSEIADRIELDTEDAYKEFLLRGYEYGQAFRGIYKTCNSGERGYLYWTGNWVTFLDSLLQTALLAERSDTLRLPTRVRHLRIDPNKHLEHVVERDGIQVVELRNDHSTNGCIAGGVECCDLNAHSVARRIQVSGQLYHEKVYFVPHFDQNCLKEQPETSTILKDYAAVIKQTLYNGFSKWQKAGLLKKLTNGPLIEKALPVLKSSLNEVVLDDTVTRFMHDGKCTILPHFTELFKIPDSDDFAEMVIGKLKSVRGIFELDRLWAGAVINDRIVKSLQDICIENSAGHHAKMAAVDLVSTDQIRHCIEANSSHPLLEVDYMCVGANVDHLDESTLEIVGGKKQKIVLDENFTGHGEVKNMDYVLLDKVLNKKANPIAFIEACKHLIRDDGFLLVVEVTSQFEIALALESLLGNEMAGDADRKYTQFFTHEQLLEIFKATGFKICNFQSDPALMTTTYAVRRVAPVPRDPAFIDVDDIKEFSWIEPLQKTVEERLNEPDSKTIWLVSNKCRNNGIVGLALCFVEENLKSNRFRSAFDMSATKAIRDGPPVWTIDDEETKKIIDLDLHANDYMDGQWGSMRHIVVKDEDAHVYKDCEHAFINTLTRGDVSSLTWFESPNQYFDSMAKTKSSQELCSVYYAPINFRDIMLAYGRLPPDAIPGNFADRECLLGMEFSGRLKDGTRLMGILPAQALATTVMVDRDYAWEVPSDWTLAEASTVPVVYTTAYYALVRRGMMKKGDKVLIHGGAGGVGQAAIAIALAAGCEVFTTVGSAEKRQFLKNLFPQLQEHHFANSRSADFELHIRQHTKGRGVNIVLNSLANEMLQASLRCLARHGRFLEIGKVDLSQNSSLGMAKLLDNVSIHGILLDSIMDPTVGDLEEWKEIARLLEQGIKSGVVKPLHSHSFPANKAEEAFRFMSAGKHIGKVIMEIRTEESTKICPPSRISVRAICRTLCHPQHVYLITGGLGGFGLELAQWLINRGARKLVLTSRTGIRTGYQARCVHFWRRTGVSVLVSTLNISKKSDAIELVKQCTQMGPLGGVFHLAMVLRDCLFENQNIQNFKDAAEAKYYGTINLDYATRDHSDKETLKWFVVFSSITSGRGNAGQTNYGWSNSTMERMIDQRRADGFPGIAIQWGAIGDVGVILENMGDNNTVVGGTLPQRMPSCLSSLDNFLSWNHPIVSSFIKADMGAKKSAGGGNLMQTIAHILGVNDISQLNPDANLGDLGLDSLMGVEIKQALERDYDIVLSMKDIRTLTLNKLQQLAEQGGTGGTALQVNELEMKKDGERDAELNTVEMLEKQMNQLFKMRVDVNDLDPQDIIVKANKVEEGPITFFVHSIEGIATPLKKVMSKCEFPVYCFQSTKNVPQTSIEDVAKCYIREMKKIQPTGPYRLIGYSYGACIGFEMACMLQQSDGQDAVEKLVLLDGSHLYMQTYRNVYRMAFGVTGDTLVNNPLFESEIMCAMTLRFANVDYKKFRVELLQQSGFKARVQKVVDTVMTTGLFKSDETVAFACMAMHSKFLMADKYKPERKFRGHITLIRAEQGAAREEDVGRDYGISQVSDDSDVHVVEGDHDTFVQGKSSAKTVSIINSIILNK

SEQ ID NO: 29 - protein, 319 aa, Mus musculus
NKRPLWFICSGMGTQWRGMGLSLMRLDSFRESILRSDEAVKPLGVKVSDLLLSTDERTFDDIVHAFVSLTAIQIALIDLLTSVGLKPDGIIGHSLGEVACGYADGCLSQREAVLAAYWRGQCIKDAHLPPGSMAAVGLSWEECKQRCPAGVVPACHNSEDTVTISGPQAAVNEFVEQLKQEGVFAKEVRTGGLAFHSYFMEGIAPTLLQALKKVIREPRPRSARWLSTSIPEAQWQSSLARTSSAEYNVNNLVSPVLFQEALWHIPEHAVVLEIAPHALLQAVLKRGVKSSCTIIPLMKRDHKDNLEFFLTNLGKVHLT

SEQ ID NO: 30 - protein, 319 aa, Rattus norvegicus
SQRPLWFICSGMGTQWRGMGLSLMRLDSFRESILRSDEALKPLGVKVSDLLLSTDEHTFDDIVHSFVSLTAIQIALIDLLTSMGLKPDGIIGHSLGEVACGYADGCLSQREAVLAAYWRGQCIKDANLPAGSMAAVGLSWEECKQRCPPGVVPACHNSEDTVTISGPQAAVNEFVEQLKQEGVFAKEVRTGGLAFHSYFMEGIAPTLLQALKKVIREPRPRSARWLSTSIPEAQWQSSLARTSSAEYNVNNLVSPVLFQEALWHVPEHAVVLEIAPHALLQAVLKRGVKPSCTIIPLMKRDHKDNLEFFLTNLGKVHLT

SEQ ID NO: 31 - protein, 319 aa, Cricetulus griseus
SKRPLWFICSGMGTQWRGMGLSLMRLDSFRESILRSDEAVKPLGIKVSDLLLSTDESTFDDIVHAFVGLTAIQIALIDLLTSVGLKPDGIIGHSLGEVACGYADGCLSQREAVLAAYWRGQCIKDAHLPPGSMAAVGLSWEECKQRCPSGVVPACHNSEDTVTISGPQAAVSEFVEQLKQEGVFAKEVRTGGLAFHSYFMEGIAPMLLQALKKVIREPRPRSARWLSTSIPEAQWQSSLARTSSAEYNVNNLVSPVLFQEALWHVPEHAVLLEIAPHALLQAVLKRGVKSSCTIIPLMKRDHKDNLEFFLTNLGKVHLT

SEQ ID NO: 32 - protein, 319 aa, Homo sapiens
GERPLWFICSGMGTQWRGMGLSLMRLDRFRDSILRSDEAVKPFGLKVSQLLLSTDESTFDDIVHSFVSLTAIQIGLIDLLSCMGLRPDGIVGHSLGEVACGYADGCLSQEEAVLAAYWRGQCIKEAHLPPGAMAAVGLSWEECKQRCPPGVVPACHNSKDTVTISGPQAPVFEFVEQLRKEGVFAKEVRTGGMAFHSYFMEAIAPPLLQELKKVIREPKPRSARWLSTSIPEAQWHSSLARTSSAEYNVNNLVSPVLFQEALWHVPEHAVVLEIAPHALLQAVLKRGLKPSCTIIPLMKKDHRDNLEFFLAGIGRLHLS

SEQ ID NO: 33 - protein, 319 aa, Macaca mulatta
GERPLWFICSGMGTQWRGMGLSLMRLDRFRDSILRSDEAVKPFGLKVSQLLLSMDESTFDDIVHAFVSLTAIQIGLIDLLSCMGLRPDGIIGHSLGEVACGYADGCLSQEEAVLAAYWRGQCIKEAHLPPGAMAAVGLSWEECKQRCPPGVVPACHNSKDTVTISGPQASVFEFMEQLRKEGVFAKEVRTGGMAFHSYFMEAIAPPLLQALKKVIREPKPRSARWLSTSIPEAQWHSSLARTSSAEYNVNNLVSPVLFQEALCHVPEHAVVLEVAPHALLQAVLKRGLKPGCTIIPLMKKDHRDNLEFFLTGIGRLHLS

SEQ ID NO: 34 - protein, 319 aa, Bos taurus
GKRPLWFICSGMGTQWRGMGLSLMRLSRFRDSILRSDEAVKPLGLQVSQLLLSTDEAIFDDMVISFVSLTAIQIALIDLLTSMGLQPDGIIGHSLGEVACGYADGCISQEEAILSAYWRGQCIKEANIPPGAMAAVGLTWEECKQRCPPGIVPACHNCIDTVTISGPQASMLEFVQQLKQEGVFAKEVRTGGMAFHSYFMDAIAPMLLQQLKKVIREPQPRSPRWLSTSIPETQWQESLARTFSAEYNVNNLVSPVLFQEALWRVPEDAVVLEIAPHALLQAVLKRGLKSSCTIIPLMKKDHRDNLEFFLSNVGQLYLT

SEQ ID NO: 35 - protein, 318 aa, Capra hircus
SKRPLWFICSGMGTQWRGMGLSLMRLSSFRDSILRSDEAVKPLGLRVSQLLLSADDIFDDIIVSFVSLTAFQIALIDLLTSMGLRPDGIIGHSLGEVACAYADGCISQEEAILSAYWRGQCIKEANIPPGAMAAVGLTWEECKQRCPPGIVPACHNSIDTVTISGPQASMLEFVKQLKQEGVFAKEVQTGGMAFHSYFMDAIAPTLLQQLKKVIREPQLRSPRWLSTSIPESQWHESLARTFSAEYNVNNLVSPVLFQEALWHVPENAVVLEIAPHALLQAILKRGLQPSCTIIPLMKKDHRDNLEFFLSNVGQLYLT

SEQ ID NO: 36 - protein, 319 aa, Equus caballus
GQRPLWFICSGMGAQWRGMGLSLMRLGTFRDSILRSDKAVKPLGLQVSDLLLSADEATFDDTVPGFVSLTAIQIALIDLLTSMGLRPDGIIGHSLGEVACGYADGCVSQEEAILAAYWRGQCIKEANIPPGAMAAVGLSWEECKQRCPPGVVPACHNSKDTVTISGPQAAVSEFVEQLKQEGVFAKEVRTGGLAFHSYFMDSISHTLLQALKKVIREPRPRSVRWLSTSIPEAQWQSSLARTFSAEYNVNNLVSPVLFQEALCHVPEHAVVLEIAPHALLQAVLKRGLKPSCTIVPLMKKDHRDNLEFFLSNVGRLHLM

SEQ ID NO: 37 - protein, 319 aa, Felis catus
GKRPLWFICSGMGAQWCGMGLSLMRLGSFRDSILRSDEAVKPLGLQVSELLLSTDEATFDDIIHAFVSLTAIQIALIDLLNSMGLRPDGIIGHSLGEVACGYADGCLSQEEAILAAYWRGQCIKETNIPPGTMAAVGLSWEECKQRCPPGVVPACHNSEDTVTISGPQAEVAAFVAELKREGVFAKEVRTGGMAFHSYFMDSIAPTLLQALKKVIREPRPRSARWLSTSIPEAQWQGSLARTFSAEYNVNNLVSPVLFQEALWHVPGDAVVLEIAPHALLQAVLKRGLKSSCTIVPLMKKDQRDNLEFFLSNVGKLHLL

SEQ ID NO: 38 - protein, 319 aa, Sus scrofa
SKRPVWFICSGMGAQWQGMGLSLMRLDRFRDSILRSDQALKPLGLRVSDLLLSTDEAVLDDIVSSFVSLTSIQIALIDLLTSLGLQPDGIIGHSLGEVACGYADGCLTQEEAVLSSYWRGYCIKEANVLPGAMAAVGLSWEECKQRCPPGIVPACHNSKDTVTISGPQAAMSEFLQQLKREDVFVKEVRTGGIAFHSYFMESIAPTLLRQLRKVILDPKPRSKRWLSTSIPEAQWQGSLARTFSAEYSVNNLVSPVLFQEALQHVPAHAVVVEIAPHALLQAVLKRSLESSCTIIPLMKKDHRDNLEFFLSNVGRLHLA

SEQ ID NO: 39 - protein, 319 aa, Cuculus canorus
TGRPLWYICSGMGTQWKGMGLSLMKLDLFRQSVLRSDEALKHTGLKVSELLLNEDENTFDDTVHAFVGLAAIQIAQIDILKAAGLEPDGIVGHSVGELACGYADNSLSHEEAILAAYWRGRCVKDAKLPPGGMAAVGLSWEECKQICPPNVVPACHNSEDTVTVSGPLGAVSEFVAKLKKDGVFAKEVRTSGVAFHSHYMASIAPVLLSALKKVIPHPKPRSPRWISTSIPESQWQSDLARYSSAEYHVNNLVNPVLFHEGLSHVPGNALVVEIAPHALLQAILKRSLKPTCIILPLMKKEHKNNLEFFLTQLGKFHMS

SEQ ID NO: 40 - protein, 319 aa, Calypte anna
SGRPLWYICSGMGTQWKGMGLSLMKLDLFRQSILRSDQALKNTGLKVSDLLLQADDNTFDETVHAFVGLAAIQIAQIDMLKAAGLQPDGILGHSVGELACGYADNCLSHEEAILAAYWRGRCVKEAKLPPGGMAAVGLTWEECKQQCPPNVVPACHNSEDTVTISGPLATVSEFVAKLKKAGVFAKEVRSAGVAFHSHYMASIAPVLLSALKKVIPHPKPRSARWISTSIPESQWQSDLAKYSSAEYHVNNLVSPVLFHEGLKHIPENAVVVEIAPHALLQAILKRTLKPTCTILPLMKKDHKNNLEFFLTQAGKIHLT

SEQ ID NO: 41 - protein, 319 aa, Anas platyrhynchos
SGRPLWYICSGMGTQWKGMGLSLMKLDVFRQSIMRSDEALKNTGLKVSDLLLQADDNTFDETVNAFVGVAAVQIAQIDMLKAAGLQPDGILGHSVGEVACGYADNSLSHEEAILAAYWRGRCVKEAKLPPGGMAAVGLTWEECKQRCPPNVVPACHNSEDTVTISGPLDSVNEFVAKLKKDGVFAKEVRSAGVAFHSYYMASIAPALLSALRKVIPHPKPRSARWISTSIPESQWQSDLARNSSAEYYVNNLVSPVLFHEGLKHIPENAVVVEIAPHALLQAILRRSLKPSCTILPLMKKDQKNNLEFFLTQAGKIHLT

SEQ ID NO: 42 - protein, 319 aa, Gallus gallus
SGRPLWYICSGMGTQWKGMGLSLMKLDLFRQSILRSDEALKSTGLKVSDLLLNADENTFDDTVHAFVGLAAIQIAQIDVLKAAGLQPDGILGHSVGELACGYADNSLSHEEAVLAAYWRGRCVKEAKLPPGGMAAVGLTWEECKQRCPPNVVPACHNSEDTVTVSGPLDSVSEFVTKLKKDGVFAKEVRRAGVAFHSYYMASIAPALLSALKKVIPHPKPRSARWISTSIPESQWQSDLARNSSAEYHVNNLVNPVLFHEGLKHIPENAVVVEIAPHALLQAILRRTLKPTCTILPLMKKDHKNNLEFFLTQTGKIHLT

SEQ ID NO: 43 - protein, 319 aa, Nestor notabilis
SGRPLWYICSGMGSQWKGMGLSLMKLDMFRQSILRSDEALKNTGLKVSDLLLRADENTFDETINAFVGLAAIQIAQIDLLKAAGLQPDGILGHSVGELACGYADNCLSQEEAILGAYWRGRCVKEAKLPPGAMAAVGLTWEECKQRCPPNVVPACHNSEDTVTVSGPLESVTEFVAKLKKDGVFAKEVRSAGVAYHSHYMASIAPVLLNALKKVIPHPKPRSARWISTSIPESQWQSDLARSCSAEYLVNNLVNPVLFHDGLKHVPENAVVVEIAPHALLQAILRRTLKPTCTILPLMKKDQKNNLEFFLTQTGKIHLT

SEQ ID NO: 44 - protein, 319 aa, Podiceps cristatus
SGRPLWYICSGMGTQWKGMGVDLMKLDLFRQSILRSDEALKSTGLKVSDLLLQADENTFDDTVHAFVGLAAIQIAQIDMLKAAGLQPDGILGHSVGELACGYADNSLSREEAILAAYWRGRCVKEAKLPPGGMAAVGLTWEECKQCCPPNVVPACHNSEDTVTISGPLDSVHEFVAKLKKDGVFAKEVRSAGVAFHSYYMASIAPVLLSALKKVIPHPKPRSARWISTSIPESQWQSDLARNSSAEYHVNNLVNPVLFHEGLKHVPENAVVVEIAPHALLQAILRRTLKPTCTILPLMKKDHKNNLEFFLTQTGKIHLT

SEQ ID NO: 45 - protein, 319 aa, Balearica regulorum gibbericeps
SGRPLWYICSGMGTQWKGMGLSLMKLDLFRQSILRSDEALKNTGLKVSDLLLQADENTFDDTVHAFVGLAAIQIAQIDMLKAAGLQPDGILGHSVGELACGYADNSLSHEEAILAAYWRGRCVKEAKLPPGGMAAVGLTWEECKQCCPPNVVPACHNSEDTVTVSGPLDSVNEFVAKLKKDGVFAKEVRSAGVAFHSYYMASIAPVLLSALKKVIPHPKPRSARWISTSIPESQWQSDLARNSSAEYHVNNLVNPVLFHEGLKHVPENAVVVEIAPHALLQAILRRTLKPTCTILPLMKKEHKNNLEFFLTQTGKIHLT

SEQ ID NO: 46 - protein, 319 aa, Phaethon lepturus
SDRPLWYICSGMGTQWKGMGLSLMKLDLFRQSILRSDEALKNTGLKVSDLLLQADENTFDDTVHAFVGLAAIQIAQIDMLKAAGLQPDGILGHSVGELACGYADNSLSHEEAILAAYWRGRCVKEAKLPPGGMAAVGLTWEECKQCCPPNVVPACHNSEDTVTVSGPLDSVNEFVAKLKKDGVFAKEVRSAGVAFHSYYMASIAPVLLSALKKVIPHPKPRSARWISTSIPESQWQSDLARNSSAEYHVNNLVNPVLFHEGLKHIPENAVVVEIAPHALLQAILRRTLKPTCTILPLMKKEHKNNLEFFLTQTGKIHLT

SEQ ID NO: 47 - protein, 319 aa, Phoenicopterus ruber
SGRPLWYICSGMGTQWKGMGLSLMKLDLFRQSILRSDEALKNTGLKVSDLLLQADENTFDDTVHAFVGLAAIQIAQIDLLKAAGLQPDGILGHSVGELACGYADNSLSHEEAILAAYWRGRCVKEAKLPPGGMAAVGLTWEECKQCCPPNVVPACHNSEDTVTVSGPLDSVREFVAKLKKDGVFAKEVRSAGVAFHSYYMASIAPVLLSALKKVIPHPKPRSARWISTSIPESQWQSDLARNSSAEYHVNNLVNPVLFQEGLKHIPENAVVVEIAPHALLQAILRRALKPTCTILPLMKKEHKNNLEFFLTQTGKIHLT

SEQ ID NO: 48 - protein, 319 aa, Ooceraea biroi
EKRPIWFVFSGMGTQWSGMGRELLGIEVFRRTLQRCADTLLPHGVDLMNIILNNTNETLENVIDTFVAIAAMQVALIDVLAAIDIYPDGIAGHSVGELGCAYADGAFTAEQTVLAAYWRGKSIVDSTLEPGAMAAVGLSWEDAQKMCPPNVSPACHNSMDSVTISGPTKDVLKFVEELKSKNIFAKLVRSSGIAFHSKYIASAGPKLRASLDKIIPNPKQRSAKWISSSIPEAAWGSPLAQVSSSAYHVNNLLSPVLFQEAIAHIPDNAITIEIAPHCLLQAILRRSLPSTVTNVSLHMRDHTNNLAFLLSNIGKLYMA

SEQ ID NO: 49 - protein, 319 aa, Anopheles funestus
DKRPVWFIYSGMGSQWASMAKDLMQLEVFHNSIYRCAEALRPEGVDLIDVLTKSDDTKFDNILNSFISIAAVQVALTDVLTHVGITPDGMVGHSVGELGCAYADGCFTPEQTVLAAYWRGRSILDTDLIAGQMAAVGLSWEECKQKLPKDVIPACHNSADSVTISGPVNSVGKVIADLNAQGIFAKGVKSSGIAFHSRYIADAAPKLRKSLDKIIPNPKNRTPRWISTSIPEESWPTPLAQQSSSAYHVNNLLSPVLFSEGLKHVPANAICIEIAPHGLLQAILKRALGKDATNLSLMKRDHANNMIFLLSNLGKLYAA

SEQ ID NO: 50 - protein, 319 aa, Anopheles darlingi
EKRPLWFIYSGMGSQWASMARDLMQLEVFHSTIARCAEALRPEGIDLIDVLTKSDESRFDNILNSFISIAAVQVALTDVLTHVGIVPEGMVGHSVGELGCAYADGCFTPEQTVLAAYWRGRSILDTDLIAGQMAAVGLSWEDCKQKLPKDVIPACHNSSDSVTISGPVASVGKVIADLNAQGIFAKGVKSSGIAFHSRYIADAAPKLRKSLDKIIPNPKPRTQRWISTSIPEESWGTALAQQSSSAYHVNNLLSPVLFAEGLKHVPANAICIEIAPHGLLQAILKRALGKEATNLSLMKRDHDNNLIFLLSNLGKLYAA

SEQ ID NO: 51 - protein, 319 aa, Glossina austeni
ESRPIWFVYSGMGSQWASMAKDLMVFDTFKKTIHRCCEILRPEGLDLMEVLTRSTEKTFENILNSFVGIAAMQVALTDLLTSLNIVPDGIVGHSVGEVACAYADGCLSMEQTILAAYWRGKSILDTKLTKGKMAAVGLSWEEAHKRLPADCFPACHNSAENCTISGPEESIDAVCQKLTAEGVFARAVKSSGYAFHSKYIADAGPKLRKSLEKVIPNAKNRSPRWISSSIPEVAWNTAIAQQASAAYHVNNLLSPVLFHQALQHVPKNAICIEVAPTGLLQAILKRSLGNETTNLSLIKRDYENNPEFFLASIGKLYAA

SEQ ID NO: 52 - protein, 319 aa, Drosophila melanogaster
DKRPIWYIYSGMGSQWASMAKDLMKIEAFAKTIQRCADVLKPEGVDLIDVLTRSTDKSFENILNSFISIAAMQVALTDLLSSLGIHPDGIVGHSVGELGCAYADGCFTPEQTVLAAYWRGKSILDTQLAKGKMAAVGLSWEDAHSRVPSDCFPVCHNSEDNCTISGPEASIEALVAKLNAEGVFAKAVNSSGYAFHSKYIAEAGPKLRKSLEKIIPNAKNRTARWISTSIPESAWNTPVAKQSSAAYHVNNLLSPVLFHEALQHVPKNAISVEIAPHGLLQAILKRALGPDATNLSLVKRGHENNVEFFLTNVGKLFAA

SEQ ID NO: 53 - protein, 320 aa, Brugia malayi
EPKQIYFIYSGMGSQWAGMVRQLMSIPAFDESLRSSSDAIVDFGVNVYEMLQSDDPSFYKNNTLNCMLAITAIQIALTDVLFLLGVMPDGIIGHSTGEMCCGYADGGLTREQTMQLAYHRGHTIMNANIKGGMAAVGLSWEEAGKRCPEGVIPACHNAADSVTISGDAEKIKEFVEELKKEDIFGKLVDSSGIPFHSPAMLKVKDKMLKAMRTSVPNPKPRSSRWISTSIPESNWENELAQMCSADYHTNNAVSPVLFYEALQKIPANAVTIEIAPHCLMHSILRRSLQKTCTNVGLINMKEKDRELESFLQALGKIYQT

SEQ ID NO: 54 - protein, 323 aa, Caenorhabditis elegans
EARPIYFIYSGMGSQWPGMAIKLMKIPMFDDSLRASSKTLEEFGLDVYGMLCNPDPEQYSNNTMNCMLAITAIQIALTDVLTALGVSPDGIIGHSTGEMGCGYADGGITREQTMRLAYHRGTTIMKHTEIKGAMAAVGLTWEQVKEQAPPGVVAACHNGADSVTISGDAEGVATFCAQLKEKDIFAKVVDTSGIPFHSPAMLAVQDEMIECMRTAVPEPKPRSSKWISTSIPEDDWESDLAATCSAEYHVHNACSPVLFYEAIQKIPANAVTIEMAPHSLMQAILRRSLQKTVTNVGLMNRPKSENDDELESFLGSLGKIYQA

SEQ ID NO: 55 - protein, 323 aa, Caenorhabditis briggsae
EPRPIYFIYSGMGSQWPGMAIELMKIPMYDESLRASSKTLEEFGLDVYGMLCNPDPEQYSNNTMNCMLAITAIQIALTDTLTALGVSPDGIIGHSTGEMGCGYADGGITREQTMRLAYHRGTTIMKHTEIKGAMAAVGLTWEEVKAQAPPGVVAACHNGADSVTISGDAEGVASFCAQLKEKEIFAKVVDTSGIPFHSPAMLAVKDEMIESMRTAVPEPKPRSSKWISTSIPEEDWESDLAATCSAEYHVHNACSPVLFYEALQKIPANAVTIEMAPHSLMQAILRRSLQKTVTNVGLMNKPKSENDNELEGFLGSLGKIYQA

SEQ ID NO: 56 - protein, 323 aa, Caenorhabditis remanei
EPRPIYFIYSGMGSQWPGMAIKLMKIPMFDESLRASSKTLDEYGLDVYGMLCNPDPEQYSNNTMNCMLAITAIQIALTDTLTALGVSPDGIIGHSTGEMGCGYADGGITREQTMRLAYYRGTTIMNHTEIKGAMAAVGLTWEEVKAQAPKGVVAACHNGADSVTISGDAEGVATFCAQLKEKDIFAKVVDTSGIPFHSPAMLAVKDEMIESMRTAVPEPKPRSSKWISTSIPEEDWESDLAATCSAEYHVHNACSPVLFYEALQKIPANAVTIEMAPHSLMQAILRRSLMKTVTNVGLMNKPKSENDDELESFLGSLGKIYQA

SEQ ID NO: 57 - protein, 319 aa, synthetic construct
NKRPLWFICSGMGTQWRGMGLSLMRLDSFRESILRSDEAVKPLGVKVSDLLLSTDERTFDDIVHAFVSLTAIQIALIDLLTSVGLKPDGIIGHSLGEVACGYADGCLSQREAVLAAYWRGQCIKDAHLPPGSMAAVGLSWEECKQRCPAGVVPACHNSEDAVTISGPQAAVNEFVEQLKQEGVFAKEVRTGGLAFHSYFMEGIAPTLLQALKKVIREPRPRSARWLSTSIPEAQWQSSLARTSSAEYNVNNLVSPVLFQEALWHIPEHAVVLEIAPHALLQAVLKRGVKSSCTIIPLMKRDHKDNLEFFLTNLGKVHLT

SEQ ID NO: 58 - protein, 319 aa, synthetic construct
NKRPLWFICSGMGTQWRGMGLSLMRLDSFRESILRSDEAVKPLGVKVSDLLLSTDERTFDDIVHAFVSLTAIQIALIDLLTSVGLKPDGIIGHSLGEVACGYADGCLSQREAVLAAYWRGQCIKDAHLPPGSMAAVGLSWEECKQRCPAGVVPACHNSEDYVTISGPQAAVNEFVEQLKQEGVFAKEVRTGGLAFHSYFMEGIAPTLLQALKKVIREPRPRSARWLSTSIPEAQWQSSLARTSSAEYNVNNLVSPVLFQEALWHIPEHAVVLEIAPHALLQAVLKRGVKSSCTIIPLMKRDHKDNLEFFLTNLGKVHLT

SEQ ID NO: 59 - protein, 319 aa, synthetic construct
NKRPLWFICSGMGTQWRGMGLSLMRLDSFRESILRSDEAVKPLGVKVSDLLLSTDERTFDDIVHAFVSLTAIQIALIDLLTSVGLKPDGIIGHSLGEVACGYADGCLSQREAVLAAYWRGQCIKDAHLPPGSMAAVGLSWEECKQRCPAGVVPACHNSEDAVTISGPQAAVNEFVEQLKQEGVAAKEVRTGGLAFHSYFMEGIAPTLLQALKKVIREPRPRSARWLSTSIPEAQWQSSLARTSSAEYNVNNLVSPVLFQEALWHIPEHAVVLEIAPHALLQAVLKAGVKSSCTIIPLMKRDHKDNLEFFLTNLGKVHLT

SEQ ID NO: 60 - protein, 319 aa, synthetic construct
NKRPLWFICSGMGTQWRGMGLSLMRLDSFRESILRSDEAVKPLGVKVSDLLLSTDERTFDDIVHAFVSLTAIQIALIDLLTSVGLKPDGIIGHSLGEVACGYADGCLSQREAVLAAYWRGQCIKDAHLPPGSMAAVGLSWEECKQRCPAGVVPACHNSEDAVTISGPQAAVNEFVEQLKQEGVAAAEVRTGGLAFHSYFMEGIAPTLLQALKKVIREPRPRSARWLSTSIPEAQWQSSLARTSSAEYNVNNLVSPVLFQEALWHIPEHAVVLEIAPHALLQAVLKAGVKSSCTIIPLMKRDHKDNLEFFLTNLGKVHLT

SEQ ID NO: 61 - protein, 319 aa, synthetic construct
NKRPLWFICSGMGTQWRGMGLSLMRLDSFRESILRSDEAVKPLGVKVSDLLLSTDERTFDDIVHAFVSLTAIQIALIDLLTSVGLKPDGIIGHSLGEVACGYADGCLSQREAVLAAYWRGQCIKDAHLPPGSMAAVGLSWEECKQRCPAGVVPACHNSEDTVTISGPQAAVNEFVEQLKQEGVFAEEVRTGGLAFHSYFMEGIAPTLLQALKKVIREPRPRSARWLSTSIPEAQWQSSLARTSSAEYNVNNLVSPVLFQEALWHIPEHAVVLEIAPHALLQAVLKRGVKSSCTIIPLMKRDHKDNLEFFLTNLGKVHLT

SEQ ID NO: 62 - protein, 319 aa, synthetic construct
NKRPLWFICSGMGTQWRGMGLSLMRLDSFRESILRSDEAVKPLGVKVSDLLLSTDERTFDDIVHAFVSLTAIQIALIDLLTSVGLKPDGIIGHSLGEVACGYADGCLSQREAVLAAYWRGQCIKDAHLPPGSMAAVGLSWEECKQRCPAGVVPACHNSEDTVTISGPQAAVNEFVEQLKQEGVFADEVRTGGLAFHSYFMEGIAPTLLQALKKVIREPRPRSARWLSTSIPEAQWQSSLARTSSAEYNVNNLVSPVLFQEALWHIPEHAVVLEIAPHALLQAVLKRGVKSSCTIIPLMKRDHKDNLEFFLTNLGKVHLT

SEQ ID NO: 63 - protein, 319 aa, synthetic construct
NKRPLWFICSGMGTQWRGMGLSLMRLDSFRESILRSDEAVKPLGVKVSDLLLSTDERTFDDIVHAFVSLTAIQIALIDLLTSVGLKPDGIIGHSLGEVACGYADGCLSQREAVLAAYWRGQCIKDAHLPPGSMAAVGLSWEECKQRCPAGVVPACHNSEDTVTISGPQAAVNEFVEQLKQEGVFAKEVRTGGLAFHSYFMEGIAPTLLQALKKVIREPRPRSARWLSTSIPEAQWQSSLARTSSAEYNVNNLVSPVLFQEALWHIPEHAVVLEIAPHALLQAVLDRGVKSSCTIIPLMKRDHKDNLEFFLTNLGKVHLT

SEQ ID NO: 64 - protein, 319 aa, synthetic construct
NKRPLWFICSGMGTQWRGMGLSLMRLDSFRESILRSDEAVKPLGVKVSDLLLSTDERTFDDIVHAFVSLTAIQIALIDLLTSVGLKPDGIIGHSLGEVACGYADGCLSQREAVLAAYWRGQCIKDAHLPPGSMAAVGLSWEECKQRCPAGVVPACHNSEDTVTISGPQAAVNEFVEQLKQEGVFAKEVRTGGLAFHSYFMEGIAPTLLQALKKVIREPRPRSARWLSTSIPEAQWQSSLARTSSAEYNVNNLVSPVLFQEALWHIPEHAVVLEIAPHALLQAVLERGVKSSCTIIPLMKRDHKDNLEFFLTNLGKVHLT

SEQ ID NO: 65 - protein, 319 aa, synthetic construct
NKRPLWFICSGMGTQWRGMGLSLMRLDSFRESILRSDEAVKPLGVKVSDLLLSTDERTFDDIVHAFVSLTAIQIALIDLLTSVGLKPDGIIGHSLGEVACGYADGCLSQREAVLAAYWRGQCIKDAHLPPGSMAAVGLSWEECKQRCPAGVVPACHNSEDTVTISGPQAAVNEFVEQLKQEGVFAKEVRTGGLAFHSYFMEGIAPTLLQALKKVIREPRPRSARWLSTSIPEAQWQSSLARTSSAEYNVNNLVSPVLFQEALWHIPEHAVVLEIAPHALLQAVLKRGVKSSCTIIPLMKDDHKDNLEFFLTNLGKVHLT

SEQ ID NO: 66 - protein, 319 aa, synthetic construct
NKRPLWFICSGMGTQWRGMGLSLMRLDSFRESILRSDEAVKPLGVKVSDLLLSTDERTFDDIVHAFVSLTAIQIALIDLLTSVGLKPDGIIGHSLGEVACGYADGCLSQREAVLAAYWRGQCIKDAHLPPGSMAAVGLSWEECKQRCPAGVVPACHNSEDTVTISGPQAAVNEFVEQLKQEGVFAKEVRTGGLAFHSYFMEGIAPTLLQALKKVIREPRPRSARWLSTSIPEAQWQSSLARTSSAEYNVNNLVSPVLFQEALWHIPEHAVVLEIAPHALLQAVLKRGVKSSCTIIPLMKEDHKDNLEFFLTNLGKVHLT

SEQ ID NO: 67 - protein, 319 aa, synthetic construct
NKRPLWFICSGMGTQWRGMGLSLMRLDSFRESILRSDEAVKPLGVKVSDLLLSTDERTFDDIVHAFVSLTAIQIALIDLLTSVGLKPDGIIGHSLGEVACGYADGCLSQREAVLAAYWRGQCIKDAHLPPGSMAAVGLSWEECKQRCPAGVVPACHNSEDTVTISGPQAAVNEFVEQLKQEGVFADEVRTGGLAFHSYFMEGIAPTLLQALKKVIREPRPRSARWLSTSIPEAQWQSSLARTSSAEYNVNNLVSPVLFQEALWHIPEHAVVLEIAPHALLQAVLKRGVKSSCTIIPLMKDDHKDNLEFFLTNLGKVHLT

SEQ ID NO: 68 - protein, 319 aa, synthetic construct
NKRPLWFICSGMGTQWRGMGLSLMRLDSFRESILRSDEAVKPLGVKVSDLLLSTDERTFDDIVHAFVSLTAIQIALIDLLTSVGLKPDGIIGHSLGEVACGYADGCLSQREAVLAAYWRGQCIKDAHLPPGSMAAVGLSWEECKQRCPAGVVPACHNSEDTVTISGPQAAVNEFVEQLKQEGVFADEVRTGGLAFHSYFMEGIAPTLLQALKKVIREPRPRSARWLSTSIPEAQWQSSLARTSSAEYNVNNLVSPVLFQEALWHIPEHAVVLEIAPHALLQAVLKRGVKSSCTIIPLMKEDHKDNLEFFLTNLGKVHLT

SEQ ID NO: 69 - protein, 319 aa, synthetic construct
NKRPLWFICSGMGTQWRGMGLSLMRLDSFRESILRSDEAVKPLGVKVSDLLLSTDERTFDDIVHAFVSLTAIQIALIDLLTSVGLKPDGIIGHSLGEVACGYADGCLSQREAVLAAYWRGQCIKDAHLPPGSMAAVGLSWEECKQRCPAGVVPACHNSEDTVTISGPQAAVNEFVEQLKQEGVFAEEVRTGGLAFHSYFMEGIAPTLLQALKKVIREPRPRSARWLSTSIPEAQWQSSLARTSSAEYNVNNLVSPVLFQEALWHIPEHAVVLEIAPHALLQAVLKRGVKSSCTIIPLMKDDHKDNLEFFLTNLGKVHLT

SEQ ID NO: 70 - protein, 319 aa, synthetic construct
NKRPLWFICSGMGTQWRGMGLSLMRLDSFRESILRSDEAVKPLGVKVSDLLLSTDERTFDDIVHAFVSLTAIQIALIDLLTSVGLKPDGIIGHSLGEVACGYADGCLSQREAVLAAYWRGQCIKDAHLPPGSMAAVGLSWEECKQRCPAGVVPACHNSEDTVTISGPQAAVNEFVEQLKQEGVFAEEVRTGGLAFHSYFMEGIAPTLLQALKKVIREPRPRSARWLSTSIPEAQWQSSLARTSSAEYNVNNLVSPVLFQEALWHIPEHAVVLEIAPHALLQAVLKRGVKSSCTIIPLMKEDHKDNLEFFLTNLGKVHLT

SEQ ID NO: 71 - protein, 319 aa, synthetic construct
NKRPLWFICSGMGTQWRGMGLSLMRLDSFRESILRSDEAVKPLGVKVSDLLLSTDERTFDDIVHAFVSLTAIQIALIDLLTSVGLKPDGIIGHSLGEVACGYADGCLSQREAVLAAYWRGQCIKDAHLPPGSMAAVGLSWEECKQRCPAGVVPACHNSEDTVTISGPQAAVNEFVEQLKQEGVFAKEVRTGGLAFHSYFMEGIAPTLLQALKKVIREPRPRSARWLSTSIPEAQWQSSLARTSSAEYNVNNLVSPVLFQEALWHIPEHAVVLEIAPHALLQVVLKRGVKSSCTIIPLMKRDHKDNLEFFLTNLGKVHLT

SEQ ID NO: 72 - protein, 319 aa, synthetic construct
NKRPLWFICSGMGTQWRGMGLSLMRLDSFRESILRSDEAVKPLGVKVSDLLLSTDERTFDDIVHAFVSLTAIQIALIDLLTSVGLKPDGIIGHSLGEVACGYADGCLSQREAVLAAYWRGQCIKDAHLPPGSMAAVGLSWEECKQRCPAGVVPACHNSEDTVTISGPQAAVNEFVEQLKQEGVFAKEVRTGGLAFHSYFMEGIAPTLLQALKKVIREPRPRSARWLSTSIPEAQWQSSLARTSSAEYNVNNLVSPVLFQEALWHIPEHAVVLEIAPHALLQLVLKRGVKSSCTIIPLMKRDHKDNLEFFLTNLGKVHLT

SEQ ID NO: 73 - protein, 319 aa, synthetic construct
NKRPLWFICSGMGTQWRGMGLSLMRLDSFRESILRSDEAVKPLGVKVSDLLLSTDERTFDDIVHAFVSLTAIQIALIDLLTSVGLKPDGIIGHSLGEVACGYADGCLSQREAVLAAYWRGQCIKDAHLPPGSMAAVVLSWEECKQRCPAGVVPACHNSEDTVTISGPQAAVNEFVEQLKQEGVFAKEVRTGGLAFHSYFMEGIAPTLLQALKKVIREPRPRSARWLSTSIPEAQWQSSLARTSSAEYNVNNLVSPVLFQEALWHIPEHAVVLEIAPHALLQAVLKRGVKSSCTIIPLMKRDHKDNLEFFLTNLGKVHLT

SEQ ID NO: 74 - protein, 319 aa, synthetic construct
NKRPLWFICSGMGTQWRGMGLSLMRLDSFRESILRSDEAVKPLGVKVSDLLLSTDERTFDDIVHAFVSLTAIQIALIDLLTSVGLKPDGIIGHSLGEVACGYADGCLSQREAVLAAYWRGQCIKDAHLPPGSMAAVLLSWEECKQRCPAGVVPACHNSEDTVTISGPQAAVNEFVEQLKQEGVFAKEVRTGGLAFHSYFMEGIAPTLLQALKKVIREPRPRSARWLSTSIPEAQWQSSLARTSSAEYNVNNLVSPVLFQEALWHIPEHAVVLEIAPHALLQAVLKRGVKSSCTIIPLMKRDHKDNLEFFLTNLGKVHLT

SEQ ID NO: 75 - protein, 319 aa, synthetic construct
NKRPLWFICSGMGTQWRGMGLSLMRLDSFRESILRSDEAVKPLGVKVSDLLLSTDERTFDDIVHAFVSLTAIQIALIDLLTSVGLKPDGIIGHSLGEVACGYADGCLSQREAVLAAYWRGQCIKDAHLPPGSMAAVGLSWEECKQRCPAGVVPACHNSEDVVTISGPQAAVNEFVEQLKQEGVFAKEVRTGGLAFHSYFMEGIAPTLLQALKKVIREPRPRSARWLSTSIPEAQWQSSLARTSSAEYNVNNLVSPVLFQEALWHIPEHAVVLEIAPHALLQAVLKRGVKSSCTIIPLMKRDHKDNLEFFLTNLGKVHLT

SEQ ID NO: 76 - protein, 319 aa, synthetic construct
NKRPLWFICSGMGTQWRGMGLSLMRLDSFRESILRSDEAVKPLGVKVSDLLLSTDERTFDDIVHAFVSLTAIQIALIDLLTSVGLKPDGIIGHSLGEVACGYADGCLSQREAVLAAYWRGQCIKDAHLPPGSMAAVGLSWEECKQRCPAGVVPACHNSEDLVTISGPQAAVNEFVEQLKQEGVFAKEVRTGGLAFHSYFMEGIAPTLLQALKKVIREPRPRSARWLSTSIPEAQWQSSLARTSSAEYNVNNLVSPVLFQEALWHIPEHAVVLEIAPHALLQAVLKRGVKSSCTIIPLMKRDHKDNLEFFLTNLGKVHLT

SEQ ID NO: 77 - protein, 319 aa, synthetic construct
NKRPLWFICSGMGTQWRGMGLSLMRLDSFRESILRSDEAVKPLGVKVSDLLLSTDERTFDDIVHAFVSLTAIQIALIDLLTSVGLKPDGIIGHSLGEVACGYADGCLSQREAVLAAYWRGQCIKDAHLPPGSMAAVGLSWEECKQRCPAGVVPACHNSEDTVTISGPQAAVNEFVEQLKQEGVLAKEVRTGGLAFHSYFMEGIAPTLLQALKKVIREPRPRSARWLSTSIPEAQWQSSLARTSSAEYNVNNLVSPVLFQEALWHIPEHAVVLEIAPHALLQAVLKLGVKSSCTIIPLMKRDHKDNLEFFLTNLGKVHLT

SEQ ID NO: 78 - protein, 319 aa, synthetic construct
NKRPLWFICSGMGTQWRGMGLSLMRLDSFRESILRSDEAVKPLGVKVSDLLLSTDERTFDDIVHAFVSLTAIQIALIDLLTSVGLKPDGIIGHSLGEVACGYADGCLSQREAVLAAYWRGQCIKDAHLPPGSMAAVGLSWEECKQRCPAGVVPACHNSEDLVTISGPQAAVNEFVEQLKQEGVLAKEVRTGGLAFHSYFMEGIAPTLLQALKKVIREPRPRSARWLSTSIPEAQWQSSLARTSSAEYNVNNLVSPVLFQEALWHIPEHAVVLEIAPHALLQAVLKLGVKSSCTIIPLMKRDHKDNLEFFLTNLGKVHLT

SEQ ID NO: 79 - protein, 319 aa, synthetic construct
NKRPLWFICSGMGTQWRGMGLSLMRLDSFRESILRSDEAVKPLGVKVSDLLLSTDERTFDDIVHAFVSLTAIQIALIDLLTSVGLKPDGIIGHSLGEVACGYADGCLSQREAVLAAYWRGQCIKDAHLPPGSMAAVGLSWEECKQRCPAGVVPACHNSEDAVTISGPQAAVNEFVEQLKQEGVAADEVRTGGLAFHSYFMEGIAPTLLQALKKVIREPRPRSARWLSTSIPEAQWQSSLARTSSAEYNVNNLVSPVLFQEALWHIPEHAVVLEIAPHALLQAVLKAGVKSSCTIIPLMKDDHKDNLEFFLTNLGKVHLT

SEQ ID NO: 80 - protein, 319 aa, synthetic construct
NKRPLWFICSGMGTQWRGMGLSLMRLDSFRESILRSDEAVKPLGVKVSDLLLSTDERTFDDIVHAFVSLTAIQIALIDLLTSVGLKPDGIIGHSLGEVACGYADGCLSQREAVLAAYWRGQCIKDAHLPPGSMAAVGLSWEECKQRCPAGVVPACHNSEDAVTISGPQAAVNEFVEQLKQEGVAADEVRTGGLAFHSYFMEGIAPTLLQALKKVIREPRPRSARWLSTSIPEAQWQSSLARTSSAEYNVNNLVSPVLFQEALWHIPEHAVVLEIAPHALLQAVLKAGVKSSCTIIPLMKEDHKDNLEFFLTNLGKVHLT

SEQ ID NO: 81 - protein, 319 aa, synthetic construct
NKRPLWFICSGMGTQWRGMGLSLMRLDSFRESILRSDEAVKPLGVKVSDLLLSTDERTFDDIVHAFVSLTAIQIALIDLLTSVGLKPDGIIGHSLGEVACGYADGCLSQREAVLAAYWRGQCIKDAHLPPGSMAAVGLSWEECKQRCPAGVVPACHNSEDAVTISGPQAAVNEFVEQLKQEGVAAEEVRTGGLAFHSYFMEGIAPTLLQALKKVIREPRPRSARWLSTSIPEAQWQSSLARTSSAEYNVNNLVSPVLFQEALWHIPEHAVVLEIAPHALLQAVLKAGVKSSCTIIPLMKDDHKDNLEFFLTNLGKVHLT

SEQ ID NO: 82 - protein, 319 aa, synthetic construct
NKRPLWFICSGMGTQWRGMGLSLMRLDSFRESILRSDEAVKPLGVKVSDLLLSTDERTFDDIVHAFVSLTAIQIALIDLLTSVGLKPDGIIGHSLGEVACGYADGCLSQREAVLAAYWRGQCIKDAHLPPGSMAAVGLSWEECKQRCPAGVVPACHNSEDAVTISGPQAAVNEFVEQLKQEGVAAEEVRTGGLAFHSYFMEGIAPTLLQALKKVIREPRPRSARWLSTSIPEAQWQSSLARTSSAEYNVNNLVSPVLFQEALWHIPEHAVVLEIAPHALLQAVLKAGVKSSCTIIPLMKEDHKDNLEFFLTNLGKVHLT